European Patent Application EP 4 578 949 A1, published July 2, 2025. Title: 超開花性ムギとその生産方法および評価方法. Applicant: 国立大学法人　岡山大学. The sequence listing filed with the application follows.

SEQUENCE LISTING (21 sequences)

SEQ ID NO: 1 - DNA, 10326 bp, Hordeum vulgare
  source 1..10326: mol_type = other DNA
  CDS 1..10326: protein_id = 2; translation = MASSQHVEVEAAKLLQKLILESKDEPAKLATKLYVICQHMKLSGKEQSLPYQVISRAMETVVSQHGIDMDALRSSRVPFSGGTQAVDASGVMSKDKEIIGGQSSMVGSDASQSSGQAALWHLPPGSADMTRPGVYIPGRVPAGNRGDVAGSDIHQGSMSQKSGRSSGVESPASLQMEDTRSMNSHDSLRSDEKTNKKASSSKRKRMDSKAAGDMQSEENSKSDGISSGQNIRKRKQVGKAGAQGQPSRGAEPEQSHKLQGATAQVPPLPGGASFFRAHQEGPPASAGRTIDNTKPSNPFAMSQVSNFAEGLASGSIPTDLQKSILGGTNMFNAGFGWNQSPQGSVIKNTQGSVANLMRPGVNVEGKINIGSQGAFNPTPTSQMDFPKIPPYMSSSFGGGSQFLDKGKDSASGNTGTELHSAAKVGVNTGIAHGSPMQERQNITRAPQRAESSLQEARLSSLPNRNVGPYQTSHISPNTPFKEQQLKQLRAQCLVFLAFRNNMQPRKVHLEIALGGGPTAEGGSVGQGGNESRMADGSARENGNSQENSAIFGSQSDMSRLPSTSAGSIAEADSSLKDSEIKKKINIAEHEKSSMEIENVQQAVVMQGTGSSSEMRSQEIASPAPSGPQQSYFQGDKRRNAPETYRTDAENLNRNLSFGGQGPSSLGGNRQHPNLEAAVLTKDRLQDEASKESYPSSRLHHMPIDGYNSNLPGKDLTPDTDRNEVEHCTQIGEMSDRSADEGDDDLFEHDGFASTPPKHTMTEKWIMDYQKRKYGENEKKVLEQQKAHKRMSASYQKLKESVSSSEDLTAKTKSVIELKKLQLLSLQRRVRSEFLLDFFKPNTADLERVKAVKKHRHGRRVKQLEKIEQKMKEERQKRIRERQKEFFADIESHRERLEDSFKAKRERLKGFNRYIKEFHKRKERIHREKLDRIQREKINLLKNNDVEGYLRMVQDAKSDRVKQLLRETEKYLQKLGAKLRGDSSMDGRSYVSGKGVTANDVEDESYQPQNYLESNEKYYQLAHSVKEIVNDQPTYLNGGKLREYQMNGLRWLVSLYNNNLNGILADEMGLGKTVQVISLLCYLMETKNDRGPFLVVVPSSVLSGWVSELNFWAPSINKIAYFGPPEERRRLFKEMIVQQKFNVLLTTYEYLMNKHDRPKLSKIQWHYIIIDEGHRIKNASCKLNADLKLYRSSHRLLLTGTPLQNNLEELWALLNFLLPNIFNSSEDFSQWFNKPFESNGDNSADEALLSEEENLLIINRLHQVLRPFVLRRLKHKVESELPGKIERLVRCEASAYQKLLMTRVEDNLGGIGAVKVRSVHNSVMELRNICNHPYLSQLHVEEIEGHLPRHYLPSIVRLCGKLEMLDRLLPKLKATGHRVLLFSTMTRLLDVMEDYLVWKKYQYLRLDGHTSGHERGALIDRFNDPDSPAFIFLLSIRAGGVGVNLQAADTVIIFDTDWNPQVDLQAQARAHRIGQKKEVLVLRLETVRTVEEQVRASAEHKLGVANQSITAGFFDNNTSAEDRREYLESLLRECKKEESAPVLDDDALNNILARSEDEIDIFESIDKQRLDDEMAIWLKVVQDGSVSGLDPSVLPSRLVSDDDLKPFCDAMKIYESSNVKNVKVNVRKKGELGGLDTKHYGRGKRAREVRSYEDQWTEEEFEKLCQAESPDSPPPGGVLKELDISKESKLEVPAESSADPVEAKTVPVLAVPDSSPPVSAVPDSSPPVPSVPDSSPPLPAVPDSSPAKRRRGRPRRSDVSVSPVMSPAKAVQQEAGTTLGSSAPASTIDSAAPTTTIHSTGPDVTIHSTAPVAATKPEIGTEVKATAFVPAVPSATMKPEIGTDVKDRVLEGLIAKKVGPEVESGHDPVAASAAPHPPAPATSRGRKTQAVETPRRRGRKPKSLSSSSAGDVNIYPVVAIGSGPTSVGSPYPQGDMPSSHASAMSRFQKDLVTDRPVTSLPEGVKGISAPEGTTTPVPEDEHTGTVISSDNASSLMPKTIHNENVGFVQASSEQVFSASVPTLTSVSGGILKASHVLLADKPAEKQSASRRRRKKAPGGEDTGVSTRQRAAMKKSYGIPGTTDNVGADMSTAEKLGAVNVKDGSPLKDTPKELPNMNSPPYDKSGYDSQPRTPIAIPISEAAVPGGFGNAHVAYSDITPRISTNPDVQDKPLNLHIGASLAAASQAQVPCKTGNDHVAVCSVVTTTHSETVTEKPLLNPVSEPANVQFEAPSSLLHNSGKNTSIEINSVAPSKASGRRRKGPASEPRTRSKAATAASERRARLAGSKQTGDARKVEILAIPSTAVCVSSVEQQEAAPAEALTASVCEMQKNAESQAHGGMSTPMGIPDAKLEPPKQIATQSITACSSFTTQTPTLPISRESNLSMGDKQGLGVHTIHGQTKMVLAAELASANDENKLHEVHDKTADSNMLQRSAAQDTLHDKTDSIAGLNLASRHRIGDLEMEKDNSNTVMLPNCQSPFDASVKDIKDTLSPTEADVSDLQSEASAINVSSLKQDTTAVEALHTNSGGCANHLPAALQSTDSNQCADRKESSENSDSELFASGKKTEEMEGTLDKNTDYNLTQTNEDSHSIALGRHSPSEDKKEDSCAHVVDGGLLGSKQTLPEIVSAINTDGSEEALNASSTRSNKDASMLEVGAFTNDATSVCEVTKDPESHASVSVLASAAMSTGDGCEEVNNVPSTHSDREDNMVEVDASRNDATSVCEARKDPESNVSGELPMPVGLSEPELELQIQSKSSSQSSSVNADETNASINIRTTSLVESEQKSPRNGAHELKEGMEVAGPKIVCAIQMPSPDGSEAHSLAQLEMVSAAEQASTKDDKEDKTVDVNLPTCPRYPDGEGEKDHSPKTILAGSQSFCEASDKDVAPMKDDHTDPQSEVNVVGMNGANQDSAETEAMLIDGVPKGSSSDLPAALRSTDSNQLAEQEDGLENSASISASPKEHEKLKETSDEIGGGNSSRRRTDDDSHFMNLVGYSEDSDEDDSVQVADVGDVGCKETTPDGISAVAREAEPGDGPCTEPTCETAVHVNECSAEAAISEDGHATTALGSVRASSTELMNLESVSACNVHQNPLNKELSYAVSVTPDSVEHDDTVVPVALQEGAAVATEPEAKKEVDEPTQNENVEPAAIKPEFVEHAGTEADPSKEASIPQEKTTVALVAGPEKNEEADAPTQVEPVALVPDSVEHAGTKVDQIIETSVGLPDETFVVPGTEPEEKKVEASAQEDIAEAVAAEPEPAGTQENAEASTQPSPMEIEGVVAEAGELPSTERGDNDVTIEPEESDASAAAAMKEPEVLSTEPAPDGENAKLGEAEAEQLLQQPSSCEATTVTEELPSTVGAKTDGTSDVGAKTDGTSDVGADESPAVVGEEVLNTEAAPDDKNARPNEPGMAQSPPLPEEGKSVAAGEPANLEGLEAPSADSQPNDGK
atggcttcatcacagcatgttgaagtggaggctgcgaagctacttcaaaaactcattctggaatcaaaggatgagcctgctaaattagcaacaaaactttacgtgatatgtcaacatatgaagttaagtggaaaagagcagtctcttccttatcaggtcatatctagggccatggagactgttgtaagtcaacatggaattgacatggatgcattgcgatcatcacgagttccattttctggcggtacacaagcagtagatgctagtggcgttatgtcgaaggataaggagatcattggtggtcagtcttccatggttggaagtgatgcatcccagagcagcggtcaagctgcattatggcatttgccaccaggttcagcagatatgacaaggcctggggtgtatattccaggcagggttccagcaggaaataggggtgatgtcgcaggatctgatattcatcaaggatccatgtcgcaaaagagtggcaggtcctctggagtcgaaagccctgcaagtctgcaaatggaggacactagatctatgaattcacatgattctttgaggtctgatgaaaaaacaaacaagaaagcttcctcttccaagagaaaaaggatggattcaaaagcagcaggggatatgcaatctgaagaaaattcaaaatcagatggtatctcaagtggacaaaatattagaaaaaggaaacaggttggcaaagctggtgcacaaggtcagccctccaggggagctgagcctgagcaatcacataaactgcaaggtgctactgctcaggtgccacccttacctggtggtgcatcatttttcagggctcaccaggaaggtccaccagcttctgctgggaggactattgacaatactaaaccatcaaacccgtttgcaatgtcacaagtttcaaattttgctgaagggctggcttctggtagtatccccactgacttgcagaaaagtatactgggaggaacaaatatgtttaacgctggttttggctggaatcaaagtccacaaggttcagttattaagaatactcaaggttctgttgccaacttaatgcggccaggagttaatgttgaagggaaaattaatatagggtcacaaggagcttttaaccctactcccacatcgcagatggatttccccaaaatccctccttacatgtcttcttcctttggaggtggctcacagtttctggacaagggcaaggactcggcttctggcaatactggcactgaacttcattctgctgctaaagttggagttaacacggggattgcgcatggcagtccaatgcaagaaaggcaaaatattaccagagcaccacagagggccgaatcatctttgcaagaagccagactgtcttcgctcccgaatagaaatgttgggccgtatcaaacatctcacatctctccaaacacaccattcaaagaacaacagttaaagcagctccgagcacagtgcttagtgtttcttgcattcagaaataacatgcagcccagaaaggtgcaccttgaaattgccttaggtggaggccccactgcagagggtggcagcgtaggtcagggaggtaacgagagcagaatggctgatggttctgcaagggaaaacggaaacagtcaggaaaactctgctattttcggcagccaaagtgatatgtctagactcccatccacatccgcaggcagcattgcagaggctgattcttcactgaaggactcggaaattaagaagaagatcaatatcgctgaacatgagaagtcatcgatggaaatagaaaatgtccagcaagctgttgttatgcagggaactggttcaagttctgaaatgcgttcccaagaaatagcatcccctgcgccatctggaccacagcagtcatactttcagggagataaaagaagaaatgcccctgagacctacaggacggatgcagaaaatttgaacaggaatttaagtttcggaggccagggaccatcttctttgggtggtaatagacaacatccaaatttggaagctgctgttttgaccaaagatcgattacaggatgaagcgtctaaagaatcatacccatcttcgaggcttcatcatatgcctattgatggttataactccaatttaccaggaaaggatctaaccccagatacagatagaaatgaggttgaacattgtacccagattggggagatgtctgatcgatcggccgatgaaggagatgatgatctatttgagcatgatggttttgcatcaactcctccaaaacacacaatgactgaaaaatggatcatggattatcaaaagagaaaatatggagaaaatgaaaagaaggtattagagcagcagaaggcacataaaaggatgtcagcatcttatcagaagttaaaggaaagtgttagttcatctgaagatcttactgcaaagacaaagagtgtcattgaattgaaaaagcttcaacttctctcacttcaacgtcgtgtccgcagtgaattcttgttagactttttcaagcctaatacagctgatttggagcgtgtaaaagcagtaaagaaacaccggcatggacgccgtgtgaaacagcttgaaaaaattgagcagaaaatgaaggaggaaaggcaaaaaagaatacgcgagaggcaaaaagaattctttgctgatatagagtctcacagagagagactggaggatagtttcaaggctaaaagagagcgtctaaagggtttcaatcgatatattaaagagttccacaagaggaaagagcgaattcatcgggagaagctggataggatccagcgggagaaaattaacttgcttaagaacaatgatgtcgaagggtatcttaggatggtccaggatgcaaaatctgaccgtgttaagcaactactacgtgagactgagaaatatctacagaaacttggggccaaattacgaggtgacagctcaatggatggccgttcttatgtttccggtaagggcgtcactgcaaacgatgttgaagacgagagctaccagccacagaattatcttgagagcaacgagaagtactatcagttggcccacagtgtgaaggagattgtaaatgaccagcctacttatcttaatggtggaaaattgcgggagtaccagatgaacggtttgcgttggctggtttcattgtacaataataatttgaatggaattttagctgacgagatgggtcttggtaaaacagttcaagtaatctctttattgtgctatcttatggaaacaaaaaatgaccggggcccatttcttgtggttgtaccatcctctgttctttctggatgggtatctgaactcaacttctgggcacctagtataaataaaattgcttattttggtcctccagaagaaaggcgcagactgttcaaagagatgattgttcaacagaagttcaatgtccttttgacaacatatgagtacttgatgaacaaacatgataggccaaaactaagcaaaatacagtggcactatataataatcgatgaagggcaccgtataaagaacgcgtcttgtaaactcaatgctgatctgaagctttatcggagttctcatcggctattgttgacaggaacacctctgcagaataatcttgaggagctgtgggcacttttgaactttttgttgcccaatatatttaactcatctgaagatttttctcagtggtttaacaaaccatttgaaagcaatggtgataactcagctgatgaggccttactttcagaagaggaaaacttgctgatcataaaccgtcttcaccaagttcttcggccctttgtactccgaagacttaagcataaggttgaaagtgaattgccggggaagattgaaagacttgtaagatgcgaggcatcagcttatcagaaacttctaatgacaagggtggaagacaaccttggtggaattggagcagttaaggtccgctcggtgcacaattctgtcatggaattgaggaacatatgcaaccatccataccttagccaacttcatgttgaggagattgagggtcatctaccgaggcactacctgccatctattgtgaggctgtgtgggaaacttgagatgttggacagattgctacccaaactcaaagctactggccatagggttctacttttttctacaatgacaagattgcttgatgtgatggaggattatttggtatggaaaaagtatcagtatcttcggttagatggacacacttctgggcatgagagaggagcacttattgatagatttaatgatcctgattctccagctttcattttcctgctaagtatccgagcaggaggtgttggtgtcaatcttcaagcagctgatactgtcataatttttgatactgattggaatcctcaggttgacctgcaagcacaggctagagcccacagaattggtcaaaagaaggaggttcttgttttacgtctagaaactgtccgaactgtagaagagcaagtcagggcttcggcagaacataaattaggcgttgctaatcagagtataactgctggatttttcgacaacaacacaagtgctgaagatcggagggagtatcttgagtcacttctacgtgagtgtaaaaaggaagaatcagctccagtgttagatgatgatgctctgaataatattcttgcccgcagcgaagatgagatcgacatatttgaatctattgacaagcaaagactagatgatgaaatggctatatggctaaaggttgttcaggatggttcagttagtgggctagacccctcagtattgccctcccgtcttgtgtctgatgatgatctgaagcccttctgcgatgctatgaagatttatgagtcgtcaaatgtaaaaaatgtgaaggtaaatgtgaggaagaagggtgagcttggcggccttgacacaaagcattatggaaggggaaaacgtgcccgtgaggtccggtcttatgaggatcaatggaccgaagaagaatttgaaaaactttgtcaggctgaatctcctgactcacctccacctggtggtgtattgaaggaattagatatctctaaagagagtaagttggaggtacctgcagaaagttcagcggatccagtcgaagccaaaacggtaccagtcctggctgttccagactcctcaccaccagtctcggctgttccagactcctcaccaccagtcccgtctgttccagactcctcaccaccactcccggctgttccagactcctcaccagctaaacgacgaagaggcagacctagaaggtcagacgtttcagtatctcctgttatgtccccagcaaaggctgtccaacaagaagcaggaactacactcggtagttctgcaccagcaagtaccatcgattctgcagcaccaactactaccatccattctactggtccagatgttaccatccattctactgcaccagttgctgccaccaaaccagagattggtacagaagttaaggctactgcttttgttcctgctgtaccatctgctaccatgaaacccgagattggcactgatgttaaggaccgtgttttggaagggcttatagcaaagaaagttggtccggaggtagagagcggtcatgacccagtagctgctagtgcagcccctcatccaccagctcctgctacatctagaggcagaaagacgcaagcagttgaaacccctcgcagacgaggccgaaaaccaaaatctctttcatcatctagtgctggtgatgttaatatataccctgtggttgcaattggtagtggacctacttctgtgggttctccatatcctcaaggggatatgccctcatcacatgcaagtgccatgtcaagatttcagaaggatttggttacagataggcctgttacatcattgccagagggagttaagggcatctccgcccctgaaggtacgacgacacctgttcccgaagatgaacacactggaactgtaataagctcagacaatgccagctcactgatgccaaagaccattcacaacgaaaatgttggatttgttcaagcgagctctgagcaagttttttctgcatcagtacctactttaacttctgtctcaggtggaatattgaaagcatcacatgttctcttggcagataagcctgctgagaagcaaagtgcttcacgccgtcgcagaaagaaagcgcctggtggtgaggatactggagtaagcactaggcaaagagcagctatgaagaaatcttatggtattcctggtaccaccgacaatgttggtgcggacatgagcacagctgagaagctaggagcagtgaatgtaaaagatggcagtccacttaaagatactcccaaggaattaccaaatatgaattctcctccatatgacaagtctgggtatgactctcaaccaagaacacctatagcaattcccattagtgaagctgcggttcctggtggtttcggtaatgcccatgttgcttattctgatataactcccaggatatctaccaatcctgatgttcaagataaaccattaaatctgcacataggagcatctctagccgcagcctcacaagctcaagtgccatgcaagacagggaatgaccatgttgcagtgtgttctgtggtcactaccactcattctgaaacggttactgaaaaaccattgctaaatcctgttagtgaaccagcaaatgtccagttcgaagcacctagttctttacttcacaattcaggtaaaaacaccagtatagagatcaatagtgtcgctcccagtaaggcatcaggtaggaggaggaaaggtcctgcctccgaaccacgcaccagaagtaaagccgcaacagctgcatctgaacgtcgtgctcgactagctggatcaaaacagacaggtgatgcgagaaaagtagaaatattggcaatcccaagcacggcggtttgtgtttcttcagttgagcaacaggaagcagccccggcagaggctctcactgcttctgtctgcgaaatgcagaagaatgctgagagtcaggcacatggtggaatgtctactccgatggggataccagatgccaagttagagcccccaaagcaaattgctacccagtcaattacagcatgtagcagttttaccactcagactcctacacttcctatatccagagaaagtaatctttccatgggtgacaagcaaggtcttggagttcataccatacatggacaaacaaagatggttttggctgcagagctggcatctgcaaatgatgaaaataagctgcatgaagtacatgataagactgctgatagcaatatgctccaacgtagtgcggcacaggatacactccatgataaaactgatagcattgctggtttgaacctagcctctcgtcatagaattggtgatttggaaatggaaaaggataattctaatacagtgatgttgccaaactgccaatccccttttgatgcctcagttaaggatattaaggatactctttcccccacagaagctgatgtcagtgatctgcaaagtgaggcttctgctattaatgtgtctagtctgaagcaagatactacggcagttgaagcattgcacactaattctggaggttgtgctaatcatctgcctgctgctttacaatcaacggactcaaaccagtgtgcagaccggaaagaaagttcagagaacagtgactctgaactttttgcatccgggaagaaaacagaggaaatggaaggaactttggataagaatacagattacaatcttactcagacaaatgaagattctcacagtatagctttaggaaggcattctccttcagaagacaaaaaagaggacagttgtgcccatgtagttgatggtggcttgttgggaagcaaacaaactcttcccgaaatcgtttctgctataaatactgatggttctgaggaagcacttaatgcttcatctacccgttcgaataaagatgccagcatgttagaagttggtgcgtttacaaatgatgccacctctgtttgtgaagtaacgaaggatcctgagagccatgcatcagtgtcagtactggcctctgctgctatgagcactggtgatggctgtgaggaagttaacaatgttccatccacccattctgacagggaggacaacatggtagaagttgatgcgtctagaaatgatgctacctctgtttgtgaagcacgcaaggatcctgagagtaatgtatctggtgagttgccaatgccagtggggctatcggagcccgagttagaattgcaaatccaatccaaatcttctagtcagtctagctcagtaaatgctgatgaaacaaatgccagtatcaacattcggactacttcactggtagagtcagaacaaaaatcacccagaaatggtgcacatgagttgaaagaagggatggaagtggccgggcctaagattgtgtgcgccatacaaatgccgagtcctgatggttctgaggctcatagtttggcacaactggagatggtttcggctgcagaacaagcatctacgaaagatgataaagaagataagacggttgatgtaaacttgcccacttgtccaagatatccagatggtgagggtgaaaaggaccattcccctaaaactattttggcaggcagccaatctttttgtgaggcctcagataaggacgttgccccaatgaaagatgatcacactgatccgcaaagtgaagttaatgttgttggtatgaatggtgccaaccaagactcagctgaaaccgaagcgatgctgattgatggtgtccccaaaggatcttcaagtgacttgcctgctgctttacgatcgaccgattcaaatcagctggcagaacaagaagatgggttagagaatagtgcctctatatctgcttctccgaaagaacatgagaaattaaaagaaacttctgatgaaattggtggtggcaattccagtcgtaggcggactgatgatgattctcattttatgaatttagttggttattcggaagactcagatgaggacgattctgtccaggtagctgatgttggtgatgtgggatgtaaagaaactactcctgatggcatctcagctgtcgctagagaagcagaaccaggagatggaccctgcacagagcctacttgtgaaactgctgttcatgtgaacgaatgcagtgcggaagctgctatttctgaggatggtcacgccacaacggcccttggcagcgtccgagcgtcttcaacggaactaatgaatttggagagtgtatctgcttgcaatgttcatcaaaaccctctgaacaaagaacttagttatgctgtttcagtaactcctgactctgttgagcatgatgacacagtagtacctgtggctctccaggaaggagctgctgtcgctacagaaccagaagcaaagaaagaggtcgacgaacctacccaaaatgaaaatgttgagccggctgctataaagccagagtttgtggagcatgctggtacagaagctgatccaagtaaagaagcatctatacctcaagagaaaaccactgtagccttggttgcaggaccggaaaaaaatgaagaagcagatgcacctactcaagtcgaaccagttgccttagtgccagattccgtggagcatgctggtaccaaagttgatcaaattatagaaacgtctgtgggtctcccagacgaaacttttgttgtacctggtacggaaccagaagagaagaaggtagaggcatccgctcaagaggatattgctgaagcagttgccgcagagccagaacctgctggaacccaggaaaatgcagaagcttctactcagccgagtcctatggagatagagggcgtggtagcagaggctggtgaacttccaagcacagagagaggggacaacgatgtgaccatagaaccagaagaatctgatgcctcagctgctgctgctatgaaggaaccagaggtgctgagcactgaaccagcacctgatggtgaaaatgctaagcttggagaagccgaagctgaacagctgttgcagcaaccttcatcatgtgaggctacgacagtcacagaagagcttcccagcacagtgggagcgaaaacggatggaacttcagatgtgggagcgaaaacggatggaacttcagacgtgggagctgatgagtctcctgctgtcgtgggagaggaggtgctcaacactgaagctgctcctgatgataagaacgcaaggccgaacgagccaggtatggcgcaatcgccacctttgccggaggagggtaagtccgttgccgctggcgagcctgccaaccttgaggggttggaggctcctagcgccgactcgcagcctaatgatggaaagtag

SEQ ID NO: 2 - protein, 3441 aa, Hordeum vulgare
MASSQHVEVEAAKLLQKLILESKDEPAKLATKLYVICQHMKLSGKEQSLPYQVISRAMETVVSQHGIDMDALRSSRVPFSGGTQAVDASGVMSKDKEIIGGQSSMVGSDASQSSGQAALWHLPPGSADMTRPGVYIPGRVPAGNRGDVAGSDIHQGSMSQKSGRSSGVESPASLQMEDTRSMNSHDSLRSDEKTNKKASSSKRKRMDSKAAGDMQSEENSKSDGISSGQNIRKRKQVGKAGAQGQPSRGAEPEQSHKLQGATAQVPPLPGGASFFRAHQEGPPASAGRTIDNTKPSNPFAMSQVSNFAEGLASGSIPTDLQKSILGGTNMFNAGFGWNQSPQGSVIKNTQGSVANLMRPGVNVEGKINIGSQGAFNPTPTSQMDFPKIPPYMSSSFGGGSQFLDKGKDSASGNTGTELHSAAKVGVNTGIAHGSPMQERQNITRAPQRAESSLQEARLSSLPNRNVGPYQTSHISPNTPFKEQQLKQLRAQCLVFLAFRNNMQPRKVHLEIALGGGPTAEGGSVGQGGNESRMADGSARENGNSQENSAIFGSQSDMSRLPSTSAGSIAEADSSLKDSEIKKKINIAEHEKSSMEIENVQQAVVMQGTGSSSEMRSQEIASPAPSGPQQSYFQGDKRRNAPETYRTDAENLNRNLSFGGQGPSSLGGNRQHPNLEAAVLTKDRLQDEASKESYPSSRLHHMPIDGYNSNLPGKDLTPDTDRNEVEHCTQIGEMSDRSADEGDDDLFEHDGFASTPPKHTMTEKWIMDYQKRKYGENEKKVLEQQKAHKRMSASYQKLKESVSSSEDLTAKTKSVIELKKLQLLSLQRRVRSEFLLDFFKPNTADLERVKAVKKHRHGRRVKQLEKIEQKMKEERQKRIRERQKEFFADIESHRERLEDSFKAKRERLKGFNRYIKEFHKRKERIHREKLDRIQREKINLLKNNDVEGYLRMVQDAKSDRVKQLLRETEKYLQKLGAKLRGDSSMDGRSYVSGKGVTANDVEDESYQPQNYLESNEKYYQLAHSVKEIVNDQPTYLNGGKLREYQMNGLRWLVSLYNNNLNGILADEMGLGKTVQVISLLCYLMETKNDRGPFLVVVPSSVLSGWVSELNFWAPSINKIAYFGPPEERRRLFKEMIVQQKFNVLLTTYEYLMNKHDRPKLSKIQWHYIIIDEGHRIKNASCKLNADLKLYRSSHRLLLTGTPLQNNLEELWALLNFLLPNIFNSSEDFSQWFNKPFESNGDNSADEALLSEEENLLIINRLHQVLRPFVLRRLKHKVESELPGKIERLVRCEASAYQKLLMTRVEDNLGGIGAVKVRSVHNSVMELRNICNHPYLSQLHVEEIEGHLPRHYLPSIVRLCGKLEMLDRLLPKLKATGHRVLLFSTMTRLLDVMEDYLVWKKYQYLRLDGHTSGHERGALIDRFNDPDSPAFIFLLSIRAGGVGVNLQAADTVIIFDTDWNPQVDLQAQARAHRIGQKKEVLVLRLETVRTVEEQVRASAEHKLGVANQSITAGFFDNNTSAEDRREYLESLLRECKKEESAPVLDDDALNNILARSEDEIDIFESIDKQRLDDEMAIWLKVVQDGSVSGLDPSVLPSRLVSDDDLKPFCDAMKIYESSNVKNVKVNVRKKGELGGLDTKHYGRGKRAREVRSYEDQWTEEEFEKLCQAESPDSPPPGGVLKELDISKESKLEVPAESSADPVEAKTVPVLAVPDSSPPVSAVPDSSPPVPSVPDSSPPLPAVPDSSPAKRRRGRPRRSDVSVSPVMSPAKAVQQEAGTTLGSSAPASTIDSAAPTTTIHSTGPDVTIHSTAPVAATKPEIGTEVKATAFVPAVPSATMKPEIGTDVKDRVLEGLIAKKVGPEVESGHDPVAASAAPHPPAPATSRGRKTQAVETPRRRGRKPKSLSSSSAGDVNIYPVVAIGSGPTSVGSPYPQGDMPSSHASAMSRFQKDLVTDRPVTSLPEGVKGISAPEGTTTPVPEDEHTGTVISSDNASSLMPKTIHNENVGFVQASSEQVFSASVPTLTSVSGGILKASHVLLADKPAEKQSASRRRRKKAPGGEDTGVSTRQRAAMKKSYGIPGTTDNVGADMSTAEKLGAVNVKDGSPLKDTPKELPNMNSPPYDKSGYDSQPRTPIAIPISEAAVPGGFGNAHVAYSDITPRISTNPDVQDKPLNLHIGASLAAASQAQVPCKTGNDHVAVCSVVTTTHSETVTEKPLLNPVSEPANVQFEAPSSLLHNSGKNTSIEINSVAPSKASGRRRKGPASEPRTRSKAATAASERRARLAGSKQTGDARKVEILAIPSTAVCVSSVEQQEAAPAEALTASVCEMQKNAESQAHGGMSTPMGIPDAKLEPPKQIATQSITACSSFTTQTPTLPISRESNLSMGDKQGLGVHTIHGQTKMVLAAELASANDENKLHEVHDKTADSNMLQRSAAQDTLHDKTDSIAGLNLASRHRIGDLEMEKDNSNTVMLPNCQSPFDASVKDIKDTLSPTEADVSDLQSEASAINVSSLKQDTTAVEALHTNSGGCANHLPAALQSTDSNQCADRKESSENSDSELFASGKKTEEMEGTLDKNTDYNLTQTNEDSHSIALGRHSPSEDKKEDSCAHVVDGGLLGSKQTLPEIVSAINTDGSEEALNASSTRSNKDASMLEVGAFTNDATSVCEVTKDPESHASVSVLASAAMSTGDGCEEVNNVPSTHSDREDNMVEVDASRNDATSVCEARKDPESNVSGELPMPVGLSEPELELQIQSKSSSQSSSVNADETNASINIRTTSLVESEQKSPRNGAHELKEGMEVAGPKIVCAIQMPSPDGSEAHSLAQLEMVSAAEQASTKDDKEDKTVDVNLPTCPRYPDGEGEKDHSPKTILAGSQSFCEASDKDVAPMKDDHTDPQSEVNVVGMNGANQDSAETEAMLIDGVPKGSSSDLPAALRSTDSNQLAEQEDGLENSASISASPKEHEKLKETSDEIGGGNSSRRRTDDDSHFMNLVGYSEDSDEDDSVQVADVGDVGCKETTPDGISAVAREAEPGDGPCTEPTCETAVHVNECSAEAAISEDGHATTALGSVRASSTELMNLESVSACNVHQNPLNKELSYAVSVTPDSVEHDDTVVPVALQEGAAVATEPEAKKEVDEPTQNENVEPAAIKPEFVEHAGTEADPSKEASIPQEKTTVALVAGPEKNEEADAPTQVEPVALVPDSVEHAGTKVDQIIETSVGLPDETFVVPGTEPEEKKVEASAQEDIAEAVAAEPEPAGTQENAEASTQPSPMEIEGVVAEAGELPSTERGDNDVTIEPEESDASAAAAMKEPEVLSTEPAPDGENAKLGEAEAEQLLQQPSSCEATTVTEELPSTVGAKTDGTSDVGAKTDGTSDVGADESPAVVGEEVLNTEAAPDDKNARPNEPGMAQSPPLPEEGKSVAAGEPANLEGLEAPSADSQPNDGK

SEQ ID NO: 3 - DNA, 20720 bp, Hordeum vulgare
  source 1..20720: mol_type = genomic DNA
  exon 1..105
  exon 184..245
  exon 2747..2952
  exon 3027..3746
  exon 3835..4037
  exon 4455..4654
  exon 4735..4799
  exon 4879..5711
  exon 5921..6018
  exon 6127..6312
  exon 6835..7015
  exon 7160..7324
  exon 7403..7446
  exon 7685..7741
  exon 7882..7978
  exon 8086..8258
  exon 8334..8547
  exon 8679..8804
  exon 8888..8977
  exon 11818..11934
  exon 12033..12113
  exon 12199..12306
  exon 12448..12617
  exon 12758..12836
  exon 12926..13000
  exon 14004..14101
  exon 14184..14291
  exon 14399..14456
  exon 14627..14848
  exon 14932..17155
  exon 17270..18475
  exon 18604..18672
  exon 18755..18820
  exon 18901..20720
atggcttcatcacagcatgttgaagtggaggctgcgaagctacttcaaaaactcattctggaatcaaaggatgagcctgctaaattagcaacaaaactttacgtggtatgcagcgcaaccaatatataggacatgaaaagctttaactcaaccataaccttgtttctttgttcaatgttctagatatgtcaacatatgaagttaagtggaaaagagcagtctcttccttatcaggtcatatctaggtaaatatttcttttgtccttggctatctttttggaagtttttctttgccatcaattttactgtaaatattagtaaatttctgttcgaaaaatactactcctgccgatccatattaaattgacacttgtttagtacaaagtagtacacatgttgtcttcttgttattctttacttgataattgttgatgtgttgttcttatgttcagaagttctacttattggtatatgatgccatcatcaaactagatttcacacatcagttagtactcattgtcaattgtggaatagtatacaaggaggggccctaaccttctaaatgctgttatagcgaggttgtaacttggtactttccctaggtactaaatgttgcaccaactagtttaggcgggaaaataggaataagcagaaaaaccagagtctcctggacacaggctcaatgagggaggggggagaatattgaagctcaccgatggacacttccctcatctatgtagtgaactgttaatacacacttacacagtagtatgatatccacaacccgaaaatgcatgggcaaattggagttcaacatccttcctctgagcagcctttctcatggagatggagattgaggaaggagaaaagtcgttggaggatggcaagagggagtggcacggaagtgcaagtaggagtaagatgggagtaacgagttgtcatttggaggcttaccctgataatatttttcttttggttgacatgttagcctgtagtaatagatctcgattcttgaaatcctctttccttgatgggagtagcgaactttgtaagactatttgattgtgtttggctaggctgtgtattttctgaaagcagatgcaagagatgttccgtgggaaagctgctatggactgtgtgctgtgagaaagctgtgaggccatctggcaaactagctgtctgaaatgcggctgcggggatagatgtctgaaatacccctaaaagccgagacattggatacatactgtttaatgataaaaacatcattacaggttaacctagttcataagtatagctattcaaccaattacctagttaattatttcatggagtttttgagttaatgcatattaacgaaaatgtatatagctttacatatcacaaaatagacgcactagtgacatacaaattttacatatcaatacacacattaatctggggccagtctgaccataggctactattgtcatacaacataaacatatcaccaaaaaaatgcagcggtcgtacacatagttcaaaaaacgccaggctttaattgtgcgttttgccaccgccttgcgcttttctgaccaaagtgcatgcttatgcgcaattatgcgcagattaagtgcagttatgcgctaggcgttttgttatcgcctagagcctaagcgcacttaagcgcttgcttaggcatgccttttttaactatggtcgtacatctcgagtggggcaaatctggagaaaggaacaacatgtacatgggcgagggaagcggcagtggtacaccttgaatgggggatatagcacaagaggtcgggcagccatggtcggcggcggccttgcttgtctgagtagccttggacactggtggaggtagatgagggggtgggggcggagcggagaagaggaggctgattgactgaggtggatgaaggatggaagcatccgacggcggtcttgcggcggcgtgccgtcagcgacataggagtcagttggtgaccagcagctggccggtggcgctaatgaaccctagaatcgccagaggtgtgggacgagaaaagggcctcgctctatgggcttggtagagatgtctctcgtggacatactggctggattatttcggcggcaaaggtgagtaatttcatctcaagtggatgcaggtttgggatcaatgcaggcaaagccagaaaagcacctcttcgaccacttacactcgtatgtgttttttgcgatggctttcaagggaatcgcgttcgctcgttttaccatttggttgcgatttcagctgtgaaggagagaaatctgcagtgaaagccaaaccaattgcagcctttgccttagacaatttacgagtgtagaaccttgagcgcaccttttgtctggaatcaatcatcagtattgtcaactgaagctatcgttttccataaatttggggttgtttttgcaccaaaataattaagtatcttttgtttggtagagattatactccattatggtatcgagtgcgttatggtttatactctatagtaggtggtgtcagatgatttaccaaatgtactgttttcaacgtgcagtatatgtttaataatatacaaataatccagtttggttaggtctactttacctgaatgtttgtaattttaaaggacagaattctgcgtatgtcagaaagttctatcaaacttccaaattttctgtagcttgacttctctcctctttccagttactaagatgcccgtaacatccataattttgcctgcagggccatggagactgttgtaagtcaacatggaattgacatggatgcattgcgatcatcacgagttccattttctggcggtacacaagcagtagatgctagtggcgttatgtcgaaggataaggagatcattggtggtcagtcttccatggttggaagtgatgcatcccagagcagcggtcaagctgcattatggcatttgccaccaggtaaccaaccaacttgaaaaggaaactgcagtcactgttttggggatgtgatatgattttccatatattattaggttcagcagatatgacaaggcctggggtgtatattccaggcagggttccagcaggaaataggggtgatgtcgcaggatctgatattcatcaaggatccatgtcgcaaaagagtggcaggtcctctggagtcgaaagccctgcaagtctgcaaatggaggacactagatctatgaattcacatgattctttgaggtctgatgaaaaaacaaacaagaaagcttcctcttccaagagaaaaaggatggattcaaaagcagcaggggatatgcaatctgaagaaaattcaaaatcagatggtatctcaagtggacaaaatattagaaaaaggaaacaggttggcaaagctggtgcacaaggtcagccctccaggggagctgagcctgagcaatcacataaactgcaaggtgctactgctcaggtgccacccttacctggtggtgcatcatttttcagggctcaccaggaaggtccaccagcttctgctgggaggactattgacaatactaaaccatcaaacccgtttgcaatgtcacaagtttcaaattttgctgaagggctggcttctggtagtatccccactgacttgcagaaaagtatactgggaggaacaaatatgtttaacgctggttttggctggaatcaaagtccacaaggttcagttattaagaatactcaaggttctgttgccaacttaatgcggccaggagttaatgttgaaggtacttccataaaaaaataatgacataacagcattgtggaagacttgaattacaaatatttaccttaatgagcttgcttacactgcagggaaaattaatatagggtcacaaggagcttttaaccctactcccacatcgcagatggatttccccaaaatccctccttacatgtcttcttcctttggaggtggctcacagtttctggacaagggcaaggactcggcttctggcaatactggcactgaacttcattctgctgctaaagttggagttaacacggggattgcgcatgtaaggcctgtagtttaatccttaaagacccagggtgttaacattctatttcggatacagtttggcccttctaaaaaaccttttaattgaaaagctaaaatttgttgctgtgttcgccagagttaggtagcttgttacagaagtgcctagtagtaatggtatagtgcagggtatttgattgcataagattgtaattgagcttcgaacacagtgtattgcattctggtttcgtgtatgtctatttgcatgccttgatagactttctgccaggtataggttgatcaaccaataaataagctgtttctgcctgcaagattaagaatattcttgtctggccatttagtgatatgttaattgatttctttatctcaagtagcggtgctttatttgatgcatccatgtactatgactttgcagggcagtccaatgcaagaaaggcaaaatattaccagagcaccacagagggccgaatcatctttgcaagaagccagactgtcttcgctcccgaatagaaatgttgggccgtatcaaacatctcacatctctccaaacacaccattcaaagaacaacagttaaagcagctccgagcacagtgcttagtgtttcttgcattcaggtacatgcttagagcaatgtaggatgattggtatccgaagttcatctctgtagcactaatgtagctacactttcttgtagaaataacatgcagcccagaaaggtgcaccttgaaattgccttaggtggaggccccactgcagagggtaagacctaagaacagaaaacattgtgtgagttagcagggtttctgtactgatgatgagcttataattaaataaacaggtggcagcgtaggtcagggaggtaacgagagcagaatggctgatggttctgcaagggaaaacggaaacagtcaggaaaactctgctattttcggcagccaaagtgatatgtctagactcccatccacatccgcaggcagcattgcagaggctgattcttcactgaaggactcggaaattaagaagaagatcaatatcgctgaacatgagaagtcatcgatggaaatagaaaatgtccagcaagctgttgttatgcagggaactggttcaagttctgaaatgcgttcccaagaaatagcatcccctgcgccatctggaccacagcagtcatactttcagggagataaaagaagaaatgcccctgagacctacaggacggatgcagaaaatttgaacaggaatttaagtttcggaggccagggaccatcttctttgggtggtaatagacaacatccaaatttggaagctgctgttttgaccaaagatcgattacaggatgaagcgtctaaagaatcatacccatcttcgaggcttcatcatatgcctattgatggttataactccaatttaccaggaaaggatctaaccccagatacagatagaaatgaggttgaacattgtacccagattggggagatgtctgatcgatcggccgatgaaggagatgatgatctatttgagcatgatggttttgcatcaactcctccaaaacacacaatgactgaaaaatggatcatggattatcaaaagagaaaatatggagaaaatgaaaagaaggtattagagcagcagaaggcacataaaaggatgtcagcatcttatcagaagttaaaggtctctctctgccttcctcacatttattctggagatggggaagtgtgctttagaaataccgtgtactccctccgtaaagaagtataagagtgtttagagggagtacatatttatgagtttttgcgagttcctgtttcatatgttcagtttttcctcactgtagcagctgtaattgttgattgcaaaattttaagttgtttatcctacaggaaagtgttagttcatctgaagatcttactgcaaagacaaagagtgtcattgaattgaaaaagcttcaacttctctcacttcaacgtcgtgtccgcaggtttgcttgccaatggagatcatcagtcttcagtttctctcccttgcgcttactgtatgtttctatggctgtaacttcctactctaatttcttgcttatattgggcagtgaattcttgttagactttttcaagcctaatacagctgatttggagcgtgtaaaagcagtaaagaaacaccggcatggacgccgtgtgaaacagcttgaaaaaattgagcagaaaatgaaggaggaaaggcaaaaaagaatacgcgagaggcaaaaagaattctttgctgatatagagtctcacaggttggataactatatttgattcttcattctgatccctttagtatagagacgttatttgaaaatattcttacgctatattctcaagtatttgtggcatctatattatgatttattttctcactgagcaactgatggatctccacttgtacagtactgatgatttggggtctatttgccaatgcagtggctatcaagctttactttcgttttggtattgtgtataggctaatatcatctgcattagagccacaacaaaagcagtttacattattcttgcagctaaataaagtccatggtggagcacagcaaaaacaagctggcccattaaataatcaaacataagtaagctaatctgaaataagtaaatggtgtcttcttaagtaaacatgttgctaaaagaactggatcgggataactgattcaacctagtcacctttgtaaacgctgtctgtctgtgtttacaccccctcaacattttgcccatgtcatttggtaataatgccttgcctttgtaacttgcagagagagactggaggatagtttcaaggctaaaagagagcgtctaaagggtttcaatcgatatattaaagagttccacaagaggaaagagcgaattcatcgggagaagctggataggatccagcgggagaaaattaacttgcttaagaacaatgatgtcgaagggtatcttaggatggtccaggtgagtcttatttgctttgtttctcatcatgttcttctatattattaacccttcacacgtcaaaaattaaagcttaacccttcattttagtttctcaatatttattggacgaagtcacatctgctaagtattgctgctttgcaggatgcaaaatctgaccgtgttaagcaactactacgtgagactgagaaatatctacagaaacttggggccaaattacgaggtgacagctcaatggatggccgttcttatgtttccggtaagggcgtcactgcaaacgatgttgaagacgagagctaccagccacaggttttattatctctttgttttagtcaacgtctaggtgcatttttgttgaatatttacttaattctgttcttcttccagaattatcttgagagcaacgagaagtactatcagttggcccacaggtactacatggattgaatagactttaatgcttccttttttgaatccttatctgtgtctgcctagcgtaaattatttactacctaactttctaatcatccatcttattcatacttttttttgaacttttccatctcattcttacttctttgctattgaacttcctaattcttttcttttgagattactgaactttctaattccgctttgtattcatacatatttgtttattttttctagtgtgaaggagattgtaaatgaccagcctacttatcttaatggtggaaaattgcgggagtaagttgtgctgctattttccctttttattacctccttttcatttaagtttgacattattgttaccgacttgtttcctgctacaacctgtttaaccatccagtacacatttccttgagccatcacttgctgcattacaggtaccagatgaacggtttgcgttggctggtttcattgtacaataataatttgaatggaattttagctgacgagatgggtcttggtaaaacagttcaagtaagatccagtacagcgccgtctcagcatttattgtttggcttgtatgttatctgatctaaacaagtgtctgaattctgcttacgctgcccttgctactttgtcaggtaatctctttattgtgctatcttatggaaacaaaaaatgaccggggcccatttcttgtggttgtaccatcctctgttctttctggatgggtatctgaactcaacttctgggcacctagtataaataaaattgcttattttggtcctccagaagaaaggcgcagactgttcaagtaattctgaatttacagttctatcctttgtcacagttcatgtgaacattttattaaccaagctaattttttcagagagatgattgttcaacagaagttcaatgtccttttgacaacatatgagtacttgatgaacaaacatgataggccaaaactaagcaaaatacagtggcactatataataatcgatgaagggcaccgtataaagaacgcgtcttgtaaactcaatgctgatctgaagctttatcggagttctcatcggctattgttgacaggaacacctctgcaggttctaaagcttgcacttaatactttcacacttgatcctgtatttgttacttttcaaggagggtctctgtatgaagtattctattatgcatatatgtcaatttgctaacttcttgtaacttcttcttgaagaataatcttgaggagctgtgggcacttttgaactttttgttgcccaatatatttaactcatctgaagatttttctcagtggtttaacaaaccatttgaaagcaatggtgataactcagctgatgaggtaaagctgctgtttttcacgatacagcattgttttcttggaaggaaactgtgtttgactccaatcatcttctttcttaaaaggccttactttcagaagaggaaaacttgctgatcataaaccgtcttcaccaagttcttcggccctttgtactccgaagacttaagcataaggtattgattttatttgctatctttatgcttgtgttgagatcactgacactgtagcaattcaccatgcaatttatttgaaattccaagtcccaataggagatctatgctatgcttagctattcaaccttattacctcaaacagagggagttccaaccttccagaattccatcaactgatgacattggcagaacccttctaaccgaaacctagtaataatagggagagagataagagaataattgcttgatgtctttattgatgcgagggcctagccttatatagctggctacatagatatatggaaacaaactaacaatcttggaagcttatctagtattttaaaaaaatctaataaccagtaaccaactagagataaaatttgatacgtactccctccgtcccaaaattcttgtcttagatttgtctagaaatgaaagtatctaaatactaaaatgtgactagatacattcatatctagataaatctaagacaacaattttgggacggagggagtatctgcttaaggcagaccagggggctagactttaggcgttggctgtctgcctgaccccacttgtcacacatattgtttgagtagtacacatgttccttaaatatgtgtgacctatcaggagttgacagatactcacagcatgtaatttggctttcagtatttcagctgattcagtagactttatatgttccatttggtgggatgatcatatttttgtattctacgaatactgagctgggcattgcagttgtgaagagctaaatattgtccataactaggttcaacagcacaagcaacacaatatagcaacgtcaaactggttcttgttagctttgttgctctacatggtctgtaatttaaaaattctatgggcaaggtttctctatgtgcctgtacacatccatctagctgcctgaatgccaaaaatgttgcttatcctgtttctcaatatatgccacttaggcatatcagtacaaacacagtcaggctcaagtttgaccaccaacacatcaaaaacatctagatttttacatcagaacaacacggtagcccttccactagagttgctctataagttgtagatgcttttatgaatgtggattttctcaactagttgctgctgtaacctactctacccatcgcgaaaagttctaaaaagatgtgaatttcgtagatgtacagtttgctataatatgtgcagctgacaaatgaccatttgtgttgtgagagaaatcaagagattagtgtctagtgtagcaactatatgtgcacacatttgtgtttgttcacacatggtcacactcactcttaaagcacatgtgcgagtatgttgtacatctatgacttttttttcttcactttttggcgaaagcattaagtgcttttcatgttctcatttttgtgaaatgcacaacatataattttgccaactactactatacaagcatataatcattaagaccatgaacaggaaagcatcttcattgataaacggtgagtgcctccatatttcttagcttatgattactgtaaaaggtaccacctctgttcctaaatgtagatgtttttagaactgcaaaaacgtgtgacatttatgaacaaagggtgtacgtgcaaggcatgtagagtatacgattcgaaaagataggcgaatcggtcaattaatcggcctataagtcaattaattggctactcggtaatccactgagtagggattaattgggcagttaattgatttatcggccgatattctgacaatacttaattatgataatttcgactgtgaaggacacaaccataaccggtgacatggcttggtgtagacgtgcagaagtgccacaaaagctaaaaggcaagttctatagaactgcggtttgacccgcaatgttgtatggcgttgagtgttgccgactaaaaggcgacatgtgcagcagttaggtgtggtggagatgcgcatgttgagatggatgtgtggccacacaaggaaggaccgagtccggaatgatgatatatgagatagagttggggtagcaccgattgaagagaagcttgtccaactccgtctgagatggtttgggcatattcagcgcaggcctctaaagtgtccgtaaagagagatcagaaggaccggagtatcaccaaacaactagccatggacaggggtgcgtggaagcttgctatccatgtgcgagaagcatgagttggtcgcgagatctgatgggtttcacctctagcctaccccaacttgtttgggactaaaggctttgttgttgtttgtttggttgagcccccccgccgcacacacacgtgcgcggagagtattgactgtacgattgaaggaaacaggaagacctaattcttttgattttctgtccgttcagtttgtagcatccagggtccagctttcttggttttggcaggagtactgtagatggtgtgtaaatcaagttcagaactgctgtttacaagtagtagagattacgattactttaagttgcaacttagttaaaaaaaatgtccatgcccccttttctcttggttttgaattgatttttgtttagactttagaaccgttggtgtcgaataagtttgaaagaagcaccaatcattggagctccaatgatttgtacttctttcaaacttattcaacatcagcggttctaaagtctaaacaaaaagctactattgtgaggctgtgtgggaaactagcttgtcaggttggggatttgatattgtttcccaactggttcctcatctttgtttgtatgattgtatctagatcatttggatggtgcaatagtttcaattgtgttttgccgtcttcaggttgaaagtgaattgccggggaagattgaaagacttgtaagatgcgaggcatcagcttatcagaaacttctaatgacaagggtggaagacaaccttggtggaattggagcagttaaggtgcgtagcgcgtgactgttcctagttgtttactttaattttcacttgtcagatatttcacaggttcttatctgtaatatgtgtcttaaattttttaggtccgctcggtgcacaattctgtcatggaattgaggaacatatgcaaccatccataccttagccaacttcatgttgaggaggtagagcatgattctgcccgtcgctacattctggctatttttgtttcctcttgggcatcaccagccatctggattctctatgcagattgagggtcatctaccgaggcactacctgccatctattgtgaggctgtgtgggaaacttgagatgttggacagattgctacccaaactcaaagctactggccatagggtaagtggattttactggcagtttggtaggtttgtaaagatctcctactcgtatgttacatgaattgtattttctcgaacaagtcacacatcgaacttgcattatctaagttgaagttgtcgttccttccttggcattcaggttctacttttttctacaatgacaagattgcttgatgtgatggaggattatttggtatggaaaaagtatcagtatcttcggttagatggacacacttctgggcatgagagaggagcacttattgatagatttaatgatcctgattctccagctttcattttcctgctaaggtaaatcttggttcagtatattgtggtgtaggaggtattatataaatagaacatagtaaactcatgaatccttattgaccaatttaattaattaattaatattcgatatctaaggcctattccacccctgttttctgtagtatccgagcaggaggtgttggtgtcaatcttcaagcagctgatactgtcataatttttgatactgattggaatcctcaggtagctaaagttccttcagtgttgtcactctatgttgtaaggtttgttttacatacatatatgatatatcttttccttgattattccaggttgacctgcaagcacaggctagagcccacagaattggtcaaaagaaggaggttcttgttttacgtctagaaactgtaagtgttacactgctcgcacgagtttctggaacacgcattaataacctgtaggtccgtagctgactaattttgtcatataactcacatttttcttgaaagcttgtcaatcatatacctggaagtgtcctttgttttatttcattttgtgtatttaggtcttttttggtatttaatattgcttgtttccagatttactccctccgttcctaaatataactcttcttagagattccactacggactacatgcggatgtatatagacatactttagagtgtagattcactcattttgctccgtatgtagcccgtaatggaatctctaaagacttatatttaggaacggaggtatattattcaagaaattagtgaaatatagttacaagaaaagtgcctggtctatctttgttgtattgtagctggggttttcctctctttgcgccaatttgtggttgtgttgctgcgctgctttggaacctagctatagggatctttattgttctcttgtatattttggcgatataactccaaatgaagttactctcaattgctccctccgagaattcacttctgaatatctgtccatggagaatatcacgagtgtagttattgctgtgtttccagtctctgatcttacttaaatgcttggtatctgtcaattagtaggggtacgcatggtcacttctcattaactctctcagatttagtgctctctttgtccatgcgcttggtatgcaaacagatgaagtaactatccatatgtggaaaaaggtgctgcactagctaccagatcgtgactgctctctacggagccttcgtcttcttggctgtttatttttctaagcttggacagaacccactagcgatttatgaaaatgccacaaatatgatagggataaatgctgcctgttatgttctaaccagaacaatgcattgtattacttcaactgaaaatttcaatacgcctgctcctgacttggatgtaccttgttgaattttaaggtccgaactgtagaagagcaagtcagggcttcggcagaacataaattaggcgttgctaatcagagtataactgctggatttttcgacaacaacacaaggtcaattcttctactcggttaagattctagcttttctagctctccttttcctttccttcatgctagatagtaacaattgcagtgctgaagatcggagggagtatcttgagtcacttctacgtgagtgtaaaaaggaagaatcagctccagtgttagatgatgatgctctgaataatattcttgcccgcaggtaagactgagtttgctgttagtattatttaagcattgttttaacaagctctgtcactcctgatactttatctacttgcatgacatattgcttttctctccttgcagcgaagatgagatcgacatatttgaatctattgacaagcaaagactagatgatgaaatggtatagtaaattcctttactttgtattccctccataaagaaatataagagcgtttaagatcactaaagtagtgatctaaacgctctcatgtttctttacagagggagtactacatgtttatttctgctaatattttgtgcatgccaatttgattcttgtatcccttgtaggctatatggctaaaggttgttcaggatggttcagttagtgggctagacccctcagtattgccctcccgtcttgtgtctgatgatgatctgaagcccttctgcgatgctatgaagatttatgagtcgtcaaatgtaaaaaatgtgaaggtaaatgtgaggaagaagggtgagcttggcggccttgacacaaagcattatggaaggggaaaacgtgcccgtgaggtcagttgcattatcatcttttttatgtctctctattattggttgaagtatttgtttgctaattcattatatatcctttgtaggtccggtcttatgaggatcaatggaccgaagaagaatttgaaaaactttgtcaggctgaatctcctgactcacctccacctggtggtgtattgaaggaattagatatctctaaagagagtaagttggaggtacctgcagaaagttcagcggatccagtcgaagccaaaacggtaccagtcctggctgttccagactcctcaccaccagtctcggctgttccagactcctcaccaccagtcccgtctgttccagactcctcaccaccactcccggctgttccagactcctcaccagctaaacgacgaagaggcagacctagaaggtcagacgtttcagtatctcctgttatgtccccagcaaaggctgtccaacaagaagcaggaactacactcggtagttctgcaccagcaagtaccatcgattctgcagcaccaactactaccatccattctactggtccagatgttaccatccattctactgcaccagttgctgccaccaaaccagagattggtacagaagttaaggctactgcttttgttcctgctgtaccatctgctaccatgaaacccgagattggcactgatgttaaggaccgtgttttggaagggcttatagcaaagaaagttggtccggaggtagagagcggtcatgacccagtagctgctagtgcagcccctcatccaccagctcctgctacatctagaggcagaaagacgcaagcagttgaaacccctcgcagacgaggccgaaaaccaaaatctctttcatcatctagtgctggtgatgttaatatataccctgtggttgcaattggtagtggacctacttctgtgggttctccatatcctcaaggggatatgccctcatcacatgcaagtgccatgtcaagatttcagaaggatttggttacagataggcctgttacatcattgccagagggagttaagggcatctccgcccctgaaggtacgacgacacctgttcccgaagatgaacacactggaactgtaataagctcagacaatgccagctcactgatgccaaagaccattcacaacgaaaatgttggatttgttcaagcgagctctgagcaagttttttctgcatcagtacctactttaacttctgtctcaggtggaatattgaaagcatcacatgttctcttggcagataagcctgctgagaagcaaagtgcttcacgccgtcgcagaaagaaagcgcctggtggtgaggatactggagtaagcactaggcaaagagcagctatgaagaaatcttatggtattcctggtaccaccgacaatgttggtgcggacatgagcacagctgagaagctaggagcagtgaatgtaaaagatggcagtccacttaaagatactcccaaggaattaccaaatatgaattctcctccatatgacaagtctgggtatgactctcaaccaagaacacctatagcaattcccattagtgaagctgcggttcctggtggtttcggtaatgcccatgttgcttattctgatataactcccaggatatctaccaatcctgatgttcaagataaaccattaaatctgcacataggagcatctctagccgcagcctcacaagctcaagtgccatgcaagacagggaatgaccatgttgcagtgtgttctgtggtcactaccactcattctgaaacggttactgaaaaaccattgctaaatcctgttagtgaaccagcaaatgtccagttcgaagcacctagttctttacttcacaattcaggtaaaaacaccagtatagagatcaatagtgtcgctcccagtaaggcatcaggtaggaggaggaaaggtcctgcctccgaaccacgcaccagaagtaaagccgcaacagctgcatctgaacgtcgtgctcgactagctggatcaaaacagacaggtgatgcgagaaaagtagaaatattggcaatcccaagcacggcggtttgtgtttcttcagttgagcaacaggaagcagccccggcagaggctctcactgcttctgtctgcgaaatgcagaagaatgctgagagtcaggcacatggtggaatgtctactccgatggggataccagatgccaagttagagcccccaaagcaaattgctacccagtcaattacagcatgtagcagttttaccactcagactcctacacttcctatatccagagaaagtaatctttccatgggtgacaagcaaggttctctccctctctctctctctctctctctctctctctctctctctctactgttattattcattgtttggtagtaacaatggctcatgctgatgcacatgatgcctttttcaggtcttggagttcataccatacatggacaaacaaagatggttttggctgcagagctggcatctgcaaatgatgaaaataagctgcatgaagtacatgataagactgctgatagcaatatgctccaacgtagtgcggcacaggatacactccatgataaaactgatagcattgctggtttgaacctagcctctcgtcatagaattggtgatttggaaatggaaaaggataattctaatacagtgatgttgccaaactgccaatccccttttgatgcctcagttaaggatattaaggatactctttcccccacagaagctgatgtcagtgatctgcaaagtgaggcttctgctattaatgtgtctagtctgaagcaagatactacggcagttgaagcattgcacactaattctggaggttgtgctaatcatctgcctgctgctttacaatcaacggactcaaaccagtgtgcagaccggaaagaaagttcagagaacagtgactctgaactttttgcatccgggaagaaaacagaggaaatggaaggaactttggataagaatacagattacaatcttactcagacaaatgaagattctcacagtatagctttaggaaggcattctccttcagaagacaaaaaagaggacagttgtgcccatgtagttgatggtggcttgttgggaagcaaacaaactcttcccgaaatcgtttctgctataaatactgatggttctgaggaagcacttaatgcttcatctacccgttcgaataaagatgccagcatgttagaagttggtgcgtttacaaatgatgccacctctgtttgtgaagtaacgaaggatcctgagagccatgcatcagtgtcagtactggcctctgctgctatgagcactggtgatggctgtgaggaagttaacaatgttccatccacccattctgacagggaggacaacatggtagaagttgatgcgtctagaaatgatgctacctctgtttgtgaagcacgcaaggatcctgagagtaatgtatctggtgagttgccaatgccagtggggctatcggagcccgagttagaattgcaaatccaatccaaatcttctagtcagtctagctcagtaaatgctgatgaaacaaatgccagtatcaacattcggactacttcactggtagagtcagaacaaaaatcacccagaaatggtgcacatggtactccctatctctatcccctctttccccctttctctcgtacgaaccatgatcctgtgcacattccccacagtgtatgctgattgttattcttatccagatagtgtatattttttatgtttttctagagttgaaagaagggatggaagtggccgggcctaagattgtgtgcgccatacaaatgccgagtcctgatggtaagaatatgctctgttattacgttctgttgtattgtagtagagacaggccagggtctcatgcacgtctgcaccttttcaggttctgaggctcatagtttggcacaactggagatggtttcggctgcagaacaagcatctacgaaaggtataggctggttctaaatttctgaactaactaatgtgcatggtcaatactcataagtagtttatcttacatatgtacagatgataaagaagataagacggttgatgtaaacttgcccacttgtccaagatatccagatggtgagggtgaaaaggaccattcccctaaaactattttggcaggcagccaatctttttgtgaggcctcagataaggacgttgccccaatgaaagatgatcacactgatccgcaaagtgaagttaatgttgttggtatgaatggtgccaaccaagactcagctgaaaccgaagcgatgctgattgatggtgtccccaaaggatcttcaagtgacttgcctgctgctttacgatcgaccgattcaaatcagctggcagaacaagaagatgggttagagaatagtgcctctatatctgcttctccgaaagaacatgagaaattaaaagaaacttctgatgaaattggtggtggcaattccagtcgtaggcggactgatgatgattctcattttatgaatttagttggttattcggaagactcagatgaggacgattctgtccaggtagctgatgttggtgatgtgggatgtaaagaaactactcctgatggcatctcagctgtcgctagagaagcagaaccaggagatggaccctgcacagagcctacttgtgaaactgctgttcatgtgaacgaatgcagtgcggaagctgctatttctgaggatggtcacgccacaacggcccttggcagcgtccgagcgtcttcaacggaactaatgaatttggagagtgtatctgcttgcaatgttcatcaaaaccctctgaacaaagaacttagttatgctgtttcagtaactcctgactctgttgagcatgatgacacagtagtacctgtggctctccaggaaggagctgctgtcgctacagaaccagaagcaaagaaagaggtcgacgaacctacccaaaatgaaaatgttgagccggctgctataaagccagagtttgtggagcatgctggtacagaagctgatccaagtaaagaagcatctatacctcaagagaaaaccactgtagccttggttgcaggaccggaaaaaaatgaagaagcagatgcacctactcaagtcgaaccagttgccttagtgccagattccgtggagcatgctggtaccaaagttgatcaaattatagaaacgtctgtgggtctcccagacgaaacttttgttgtacctggtacggaaccagaagagaagaaggtagaggcatccgctcaagaggatattgctgaagcagttgccgcagagccagaacctgctggaacccaggaaaatgcagaagcttctactcagccgagtcctatggagatagagggcgtggtagcagaggctggtgaacttccaagcacagagagaggggacaacgatgtgaccatagaaccagaagaatctgatgcctcagctgctgctgctatgaaggaaccagaggtgctgagcactgaaccagcacctgatggtgaaaatgctaagcttggagaagccgaagctgaacagctgttgcagcaaccttcatcatgtgaggctacgacagtcacagaagagcttcccagcacagtgggagcgaaaacggatggaacttcagatgtgggagcgaaaacggatggaacttcagacgtgggagctgatgagtctcctgctgtcgtgggagaggaggtgctcaacactgaagctgctcctgatgataagaacgcaaggccgaacgagccaggtatggcgcaatcgccacctttgccggaggagggtaagtccgttgccgctggcgagcctgccaaccttgaggggttggaggctcctagcgccgactcgcagcctaatgatggaaagtag

SEQ ID NO: 4 - DNA, 10173 bp, Triticum aestivum
  source 1..10173: mol_type = other DNA
  CDS 1..10173: protein_id = 5; translation = MASSQHVEVEAAKLLQKLILESKDEPAKLATKLYVICQHMKLSGKEQSLPYQVISRAMETVVSQHGIDMDALRSSRVPFAGGPQAVDSSGVMSKDKEIIGGQSSMVGSDASQSSGQAALWHLPPGSADMARPGVYIPGRVPAGQNRGDVAGSDIHQGSMSQKSGRSSGVESPASLQMEDTRSMNSHDSLKSDEKTSKKASSSKRKRMDSKAAGDMQSEENSKSDGISSGQNIRKRKQVGKAGAQGQPSRGAEPEQSHILQGATAQVPPLPGGASFFRAHQEGPPASAGRTIDNTKPSNPFAMSQVSNFAEGLASGSIPTELQKSILGGTNMFNTGFGWNQSSQGSAIKNTQGSVANLMRPGVKVEGKINVGSQGAFNPTPTSQMDFPKIPPYMSSSFGGGSQFLDKGKDSASGNTGTELHSAAKVGVNMGIVHGSPMQERQNITRAPQRAESSLQEARLSSLPNRNVGPYQTSHISPNTPFKEQQLKQLRAQCLVFLAFRNNMQPRKVHLEIALGGGPTAEGGGAGQGGNESRVADGSVRENGNSQENSAIFGSQSDMSRLPSTSAGSIAEADSSLKDSEIKKKINIAEHEKSSMEMENIQQAVMQGTGSSSEMRSQEIASPVPSGPQQSYFQGDKRRNAPEAYRTDAENLNRNLSFGGQGPSSLGGNRQHPNFEAAVLTKDRLQDEASKESYPPSRLHHMPIDGYNSNLPGKDLTPDTDRNEVEHCTQMGEMSDRSADEGDDDLFEHDDFASTPPKYTMTEKWIVDYQKRKYGENEKKVLEQQSAHKRMSASYQKLKESVSSSEDLTAKTKSVIELKKLQLLSLQRRVRSEFLSDFFKPNTADLERVKAVKKHRHGRRVKQLEKIEQKMKEERQKRIRERQKEFFADIESHRERLEDSFKAKRERLKGFNRYIKEFHKRKERIHREKLDRIQREKINLLKNNDVEGYLRMVQDAKSDRVKQLLRETEKYLQKLGAKLRGDSSMDGRSYVSGKGVTANDVEDESYQPQNYLESNEKYYQLAHSVKEIVNDQPTYLNGGKLREYQMNGLRWLVSLYNNNLNGILADEMGLGKTVQVISLLCYLMETKNDRGPFLVVVPSSVLSGWVSELNFWAPSINKIAYFGPPEERRRLFKEMIVQQKFNVLLTTYEYLMNKHDRPKLSKIQWHYIIIDEGHRIKNASCKLNADLKLYRSSHRLLLTGTPLQNNLEELWALLNFLLPNIFNSSEDFSQWFNKPFESNGDNSADEALLSEEENLLIINRLHQVLRPFVLRRLKHKVESELPGKIERLVRCEPSAYQKLLMTRVEDNLGGIGAVKVRSVHNSVMELRNICNHPYLSQLHVEEIEGHLPRHYLPSIVRLCGKLEMLDRLLPKLKATGHRVLLFSTMTRLLDVMEDYLVWKKYQYLRLDGHTSGHERGALIDRFNDPDSPAFIFLLSIRAGGVGVNLQAADTVIIFDTDWNPQVDLQAQARAHRIGQKKEVLVLRLETVRTVEEQVRASAEHKLGVANQSITAGFFDNNTSAEDRREYLESLLRECKKEESAPVLDDDALNNILARSEDEIDIFESIDKQRLDDEMAVWLKVVQDGSVSGLDPSVLPPRLVSDDDLKPFCHAMKIYESSNVKNVKVNVRKKGELGGLDTKHYGRGKRAREVRSYEDQWTEEEFEKLCQAESPDSPQPGGVLKDIDISKESKLEVPAESSIDPKESSIDPVEAKTVPVLAVPDSSPPVPSVPDSSPAKRRRGRPRRSDVSVSPVMSPAKAVQQEAGTTLGSSAPASTIDSAAPTATIHSTGPDVTTHSAAPVAAIKPDIGAEVKATAFVAAVPTATMKPEIGTEVTDHVVLEGSIAKEVGPAVESGHDPVAASAAPHPPAPATSRGRKTQTVETPRRRGRKPKSLSSSSAGDVNINPVVAIGSGPASVGSPYPQGDMPASLMSRFQKDLVTGRPVTSLPEAVKGISAPEGTTPVAEDKHTGTAISSDNASLLMPKIIHNENVGFVQVSSEQVFSASVPTLTAVSGGILKASHILLADKPAEKQSASRRRRKKAPGGEDTGVSTRQRAAMKKSDGIPGTTDNVGADTSTAEKLGAVNVKDGSSLQDTPKELPNINSPPYDKSGYDSQPRTPIAVPISEAALPSGSGNAHVAYSDITPRIPTNPDVQDKPVNLHIGAPLAAATQPEVPCKTGNDHVAVCSVVTTTHSETVTEKPLLNPVSEVANVQVEAPSSSLHNSGKNISTVPSEVNSVAPSKASGRRRKGPASEPRTRSKAATAACERRARLAGPKQTGDARKLEILASPSTAVCVSSVEQQETALAEPLTASVCEPQKNAESHVRGGMSTPTGILDAPKQIATQSITACTEETNNSLSTQTPALPISRESILSMGDKQGVGVDTIHGQTKMVLAAELTSANDEHKLHEVHDKTADGNILQHSAANDTLQDKTDSIAGLDLASRHRIGDLEMEKGDSKTVMLPDCQTPFDASVKDINDTLAPTEADVSDLQSEAAAIDVTSPKQDTMVVEALYTNPGGSASHLPAALQSTDSNQHAERKGSSDNSGSKIFASGKKTEEMEGTLDKNTDHNLIQANANIALGRYSPSEDKREDSCAHVVDGGLLGSKQTLPEVVSAVNTDGSEEALNASSTHSNKDATLVCEVTKDPESHVSVSVLASAAMNAGDDSEEVHNVPSTHSDRGGSMVEVDASRDDATSICEVRKDPESNVSGELSMPVRLAELELELPNQSKSSSQSSAVNADETKASINIQTTSLVESGEQKSPRNGAHELKEGMELAGPKIECTIQMPSPDDKSSEAHSLAQREMVSGAEQASMKDDKENKMVDVTFSSGGEQETQRADVDLPTCPTYADCEGEKDDSPKTILAGSQSFCEASDKDVAPVRDDHTDPQSEVIVVDMNDANQDSAEAEAMQIDSVSKGSSSDLPAALRSTDSNQLAEQVSPCPKEHEKLEETSGEIGGGNSNRSRTDGDSHIMNLVGYSEDSDEDDSIQVADVGDVGSKETTHYDISAVARGAEPGDGPCTEPTCETAVHVHECNADVAISEDGHGTTALGSVQVSTTELKDLESGRCLEHGIGTPVALQEGTAVATEPEAKKEVDEPTQNEDVELAAIKPEAVEHAGTEADPSKEASIPPQEETTAVALVTGPEQNEEADAPTQVEPVAIVPDSMEHASTEVDQSIETSVRLPEKTSVIPGTEPEEKKVEASSQEDNVEAVAAEPEPAGSQENAEVSTKPSPMEIESVQETAMLGEAETRQQLPLPSAEGVVAEASEPPEVTAMKEPELLSTEPAPDGENAKLGEAKAEQLLQQPSSCEAMAAVTGELPSAAGAKTDGTSDVVADESPAVVGEEVLNTETAPDGKNPRPSEADTAQSPPLPEEGKAVAATEPANLEEAEATDGK
atggcttcatcacagcatgttgaagtggaggctgcgaagctacttcaaaaactcattctggaatcaaaggatgagcccgctaaattagcaacaaaactttatgtgatatgtcaacatatgaagttaagtggaaaagagcagtctcttccctatcaggtcatatctagggccatggagactgttgtaagtcaacatggaattgatatggatgcactgcgatcatcacgagttccatttgccggcggtccacaagcagtagattctagtggcgttatgtctaaggacaaggagatcattggtggtcagtcttccatggttggaagtgatgcatcccagagcagcggtcaagctgcattatggcatttgccaccaggttcagcagatatggcaaggcctggggtgtatattccaggcagggttccagcaggacaaaataggggtgatgtcgcaggatctgatattcatcaaggctccatgtcgcaaaagagtggcaggtcctctggagtcgaaagccctgcaagtctgcaaatggaggacactagatctatgaattcacatgattctttgaagtccgatgaaaaaacaagcaagaaagcttcctcttccaagagaaaaaggatggattcaaaagcagcaggggatatgcaatctgaagaaaactcaaaatcagatggtatctcaagtggacaaaatattagaaaaaggaaacaggttggcaaagcaggtgcacaaggtcagccctccaggggagctgagcctgagcaatcacatatactgcaaggtgctactgctcaggtgccacccttacctggtggtgcatcatttttcagggctcaccaggaaggtccaccagcttctgctgggaggactattgacaatactaaaccatcaaacccgttcgcaatgtcacaagtttcaaattttgctgaagggctggcttctggtagtatccccactgagttgcagaaaagtatactgggaggaacaaatatgtttaacactggttttggctggaatcaaagttcacaaggttcagctattaagaatactcaaggttctgttgccaacttaatgcgaccaggagttaaggttgaagggaaaattaatgtagggtcacaaggagcttttaaccctactcccacatcgcagatggattttcccaaaatccctccttacatgtcttcctcctttggaggtggctcacagtttctggacaagggcaaggattcggcttctggcaataccggcactgaacttcattctgctgctaaagttggagttaacatggggattgtgcatggcagtccaatgcaagaaaggcaaaatattaccagagcaccacagagggccgaatcatctttgcaagaagccagattgtcttcgctcccgaatagaaatgttgggccatatcaaacgtctcacatctctccaaacacacctttcaaagaacaacagttaaagcagctccgagcacagtgcttagtatttcttgcattcagaaataatatgcagcccagaaaggtgcaccttgaaattgccttaggtggaggccccactgcagagggtggcggcgcgggtcagggaggtaacgagagcagagtggctgatggttctgtaagggaaaacggaaacagtcaggaaaactctgctattttcggcagccaaagtgatatgtctagactcccatccacatctgcaggcagcattgcagaggctgactcttcactgaaggactcggaaattaagaagaagatcaatatagctgaacatgagaagtcatcgatggaaatggaaaatatccagcaagctgttatgcagggaactggttcaagttctgaaatgcgctcccaagaaatagcatcccctgtgccatctggaccacagcagtcatactttcagggagataaaagaagaaatgcccctgaggcctacaggacggatgcagaaaatttgaacaggaatttaagtttcggaggccagggaccatcttctttgggtggtaatagacaacatccaaattttgaagctgctgttttgaccaaagatcgattacaggatgaagcatctaaagaatcatatccaccttcgaggcttcatcacatgcctatcgatggttacaactccaatttaccaggaaaggatctaactccagatacagatagaaatgaggttgaacattgtacccagatgggggagatgtctgatcgatcagctgatgaaggagatgacgatctatttgagcatgatgattttgcatcaactcctccaaaatacacaatgactgaaaaatggatcgtggattatcaaaagagaaaatatggagaaaatgaaaagaaggtattagagcagcagagcgcacataaaaggatgtcagcatcctatcagaagttaaaggaaagtgttagttcatctgaagatcttactgcaaagacaaagagtgtcattgaattgaaaaagcttcaacttctctcacttcaacgtcgtgtgcgcagtgaattcttgtcagactttttcaagcctaatacagctgatttggagcgtgtaaaagcagtaaagaaacaccggcatggacgccgtgtgaaacagcttgaaaaaattgaacagaaaatgaaggaggaaaggcaaaaaagaatacgtgagaggcaaaaagagttctttgctgatatagagtctcacagagagagactggaggatagtttcaaggctaaaagagagcgtctaaagggtttcaatcgatatataaaagagttccacaagaggaaagagcgaattcatcgggagaagctggataggatccagcgggagaaaattaacttgcttaagaacaatgacgttgaagggtatcttaggatggtccaggatgcaaaatctgaccgtgttaagcaactactacgagagactgagaaatatctacagaaacttggggccaaattacgaggtgacagctcaatggatggccgttcttatgtttctggtaagggcgtcactgcaaacgatgttgaagacgagagctaccagccacagaattatcttgagagcaacgagaagtactatcagttggcccacagtgtgaaggagattgtaaatgaccagcctacttatcttaatggtgggaaattgcgggagtaccagatgaacggtttgcgttggctggtttcattgtacaataataatttgaatggaattttagctgacgagatggggcttggtaaaacagttcaagtaatctctttgttgtgctaccttatggaaacaaaaaatgaccggggcccatttcttgtggttgtaccatcctctgttctttctggatgggtatctgaactcaacttctgggcacctagtataaataaaattgcttattttggtcctccagaagaaaggcgcagactgttcaaagagatgattgttcaacagaagttcaatgttcttttgacaacatatgagtacttgatgaacaaacatgataggccaaaactaagcaaaatacagtggcactatataataatcgatgaagggcaccgcataaagaatgcgtcttgtaagctcaatgctgatctgaagctttatcggagttctcatcggctattgttgacaggaacacctctgcagaataatcttgaggagctgtgggcacttttgaactttctgttgcccaatatatttaactcatccgaagatttctctcagtggtttaacaaaccatttgaaagcaatggtgataactcagctgatgaggccttactttcagaggaggaaaacttgctgatcataaaccgtcttcaccaagttcttcggccctttgtactccgaagacttaagcataaggttgaaagtgaattgccagggaagattgaaagacttgtaagatgcgagccatcagcttatcagaaacttctgatgacaagggtggaagacaaccttggtggaattggagcagttaaggttcgctcggtgcacaattctgtcatggaattgaggaacatatgcaaccatccataccttagccagcttcatgttgaggagattgagggtcatctacctaggcactacctgccatctattgtgaggctgtgtgggaaacttgagatgttggacagattgctacccaaactcaaagctactggccatagggttctacttttttctacaatgacaagattgcttgatgtgatggaggattatctggtatggaaaaagtatcagtaccttcggttagatggacacacttctgggcatgagagaggagcacttattgatagatttaatgatcctgattctccagctttcatttttctgctaagtatccgagcaggaggcgttggtgtcaatcttcaagcagctgatactgtcatcatatttgatactgattggaatcctcaggttgacttgcaagcacaggctagagcccacagaattggtcaaaagaaggaggttcttgttttacgtttagaaactgtccgaactgtagaagagcaagtcagggcttcggcagaacataaattaggcgttgctaatcagagtataactgctggatttttcgacaacaacacaagtgctgaagatcggagggagtatcttgagtcacttctacgtgagtgtaaaaaggaagaatcagctccagtgttagatgatgatgctctgaataatattcttgcccgcagcgaagatgagatcgacatatttgaatctattgacaagcaaagactagatgatgaaatggctgtatggctaaaggttgttcaggatggttcagttagtgggctagacccctcagtattgccaccccgccttgtgtctgatgatgatctgaagcccttctgtcatgctatgaagatttacgagtcttcaaatgtaaaaaatgtgaaggtaaatgtgaggaagaagggcgagcttggcggccttgatacaaagcattacggaaggggaaaacgtgctcgtgaggtccggtcttatgaggatcaatggaccgaagaagaatttgaaaaactttgtcaggctgaatctcctgactcacctcaacctggtggtgtattgaaggatatagatatctctaaagagagtaagttggaggtacctgcagaaagttcaatagacccaaaagaaagttcaatagatccagtcgaagccaaaacggtgccagtcctggctgttccagactcctcaccaccagtcccgtctgttccagactcctcaccagcaaagcggcgaagaggtagacctagaaggtcagacgtttcagtatctcctgttatgtccccagcaaaagctgtccaacaagaggcaggaactacacttggcagttctgcaccagcaagtaccatcgattctgcagcaccaactgctaccatccattctactggtccagatgttaccacccattctgctgcaccagttgctgccatcaaaccagatattggtgcagaagttaaggctactgcttttgttgctgctgtaccaactgctaccatgaaacccgagattggtactgaagttacggaccatgttgttttggaagggtctatagcaaaggaagttggtccggcggtagagagcggtcatgacccagtagctgccagtgcagcccctcatccaccagctcctgctacatctagaggcagaaagacccaaacagttgaaacccctcgcagacgaggccgaaaaccaaaatctctttcctcatctagtgctggtgatgttaatataaaccctgtggttgcaattggtagtggacctgcttctgtgggttctccatatcctcaaggggatatgcctgcaagtctcatgtcaagatttcagaaggatttggttacaggtaggcctgttacgtcattgccagaggcagttaagggcatctccgcccctgaaggtacgacacctgttgccgaagataaacacactggaactgcaataagctcggacaatgccagcttactaatgccaaagatcattcacaacgaaaatgttggatttgttcaagtgagctctgagcaagttttttctgcatcagtacctactttaactgccgtctcaggtggaatattgaaagcatcacatattctcttggcagataagcctgccgagaagcaaagtgcttcacgccgtcgcagaaagaaagcgcctggtggtgaggatactggagtaagcactaggcaaagagcagctatgaagaaatctgatggtattcctggtaccactgacaatgttggtgcggacacgagcacagctgagaagctaggagcagtgaatgtaaaagatggcagttcacttcaagatactcccaaggaattaccaaatataaactctcctccatatgacaagtctgggtatgactctcaaccaagaacacctatagcagttcccattagtgaagctgcacttcctagtggttccggtaatgcccatgttgcttattctgatataactcctaggatacctaccaatcctgatgttcaagataaaccagtaaatctgcacataggagcacctctagcggcagccacacaacctgaagtgccatgtaagacagggaatgaccatgttgcagtgtgttctgtggtcactaccacacattctgaaacggttactgaaaaaccattgctaaatcctgttagtgaagtagcaaatgtccaggtcgaagcacctagttcttcacttcataattcaggtaagaacatcagtacagtgccttcagaggtcaatagtgtcgctcccagtaaggcatcaggtaggaggaggaaaggtcctgcctctgaaccacgcaccagaagtaaagccgcaacagctgcatgtgaacgtcgtgctcgactagctggaccaaagcagacaggtgatgcgagaaaattagaaatattggcaagcccaagcacggcggtttgtgtttcttcagttgagcaacaggaaaccgccctggcagagcctctcaccgcttctgtctgcgaaccgcagaagaatgctgagagtcatgtacgtggtggaatgtctactccgacggggatactagatgccccaaagcaaattgctacccagtcaattacagcatgtactgaagaaacaaataacagtctaagcacccagactcctgcacttcccatatccagagaaagtattctttccatgggtgacaagcaaggtgttggagttgataccatacatggacaaacaaagatggttttggctgcagaactgacatctgcaaatgatgaacataagctgcatgaagtacatgataagactgctgatggtaatatactccaacacagtgcggcaaatgacacactccaggataaaactgatagcattgctggtttggacctagcctctcgtcatagaattggtgatttggaaatggagaagggtgattctaaaacagtgatgttaccagactgccaaaccccttttgatgcctcagttaaggatattaacgatactcttgcccccacagaagctgatgtcagtgatctgcaaagtgaggctgctgctattgatgtgactagtcctaagcaagatactatggtagttgaagcactttacactaatcctggaggttctgctagtcatctgcctgctgctttacaatcaacggactcaaaccagcatgcagaacggaaaggaagttcagataacagtggctctaaaatttttgcatctgggaagaaaacagaggaaatggaaggaactttggataagaatacggatcacaatcttattcaggcaaatgccaatatagctttaggaagatattctccttcagaggacaaaagagaggacagttgtgcccatgtagttgatggtgggctgttgggaagcaaacaaactcttcctgaagtcgtttctgctgtaaacactgatggctctgaggaagcactcaatgcttcgtctacccactcgaataaagatgccaccttggtttgtgaagtaacaaaggatcctgagagtcatgtatcagtgtctgtactggcctctgctgctatgaacgctggtgatgactctgaggaagttcacaatgttccatccacccattctgatagagggggcagcatggtagaagttgacgcgtctagagatgatgctacctctatttgcgaagtacgcaaggatcctgagagtaatgtatctggtgagttgtcgatgccagtacggttagcggagcttgagttagaactgccaaaccaatccaaatcttctagccagtctagcgcagtaaatgctgatgagacaaaggccagtatcaacattcagactacttcattggtagaatcaggagaacaaaaatcacccagaaatggtgcacatgagttgaaagaagggatggagttggctgggcctaagattgagtgcaccatacaaatgccgagtcccgatgataagagttctgaggctcatagtttggcacaacgggagatggtttcgggtgcagaacaagcatctatgaaagatgataaagaaaacaagatggttgatgttacattttcgtctggtggggaacaagaaacacagcgagctgatgtagacttgcccacatgtccaacatatgcagattgtgagggtgaaaaggacgattcccctaaaactattttggcaggcagccaatctttttgtgaagcctcagataaggacgttgccccagtgagagatgatcacactgatccgcaaagtgaagttattgttgttgatatgaatgatgccaaccaagactctgctgaagcggaagctatgcagattgatagtgtctccaaaggatcttcaagtgatttgcctgctgctttacgatcgaccgattcaaatcagctggcagaacaagtatctccttgtccgaaagaacatgagaaattggaagaaacttctggtgaaattggtggtggcaattccaatcgtagtcggactgatggtgattctcatattatgaatctagttggttattcggaagactcagatgaggacgattctatccaggtagctgatgttggtgatgtgggaagtaaagaaaccactcattatgacatctcagctgtcgctagaggagcagaaccaggagatggaccctgcacagagcctacttgtgaaactgctgttcatgtgcacgaatgcaatgcggacgttgctatttctgaggatggtcatggcacaacggcccttggcagcgtccaagtgtctacgacagaactaaaggatttggagagtggaagatgtctagaacatggaataggaacccctgtggctcttcaggagggaactgctgtcgctacagaaccagaagcaaagaaagaggtcgacgaacctactcaaaatgaagatgttgagctggctgccataaagccagaggcggtggagcatgctggtacagaggccgatccaagtaaagaagcatctatacctcctcaagaggaaaccactgctgtagccttggttacaggaccggaacaaaatgaagaagcagatgcacctactcaagtcgaaccagttgctatagtgccagattccatggagcatgctagtaccgaagttgatcaaagtatagaaacatctgtgcgtctcccagaaaaaacttctgttatacctggtacggaaccagaagagaagaaagtagaggcatcctcccaagaggataatgttgaagcagttgctgcagagccagaacctgctggatcccaggaaaatgcagaagtttctaccaagcctagtcctatggagatagagtcggttcaggaaacagctatgctgggagaagctgaaaccaggcagcaactgccacttccgtctgccgagggcgtggtagccgaggctagtgaacctccagaggtgactgctatgaaggaaccagagttgctgagcactgaaccagcacccgatggtgaaaatgctaagcttggagaagccaaagctgaacagctgttgcagcaaccttcatcctgcgaggctatggcagcagtcacaggagagcttcctagcgcagcgggagcgaaaacggatggaacttcagacgtggtggctgatgagtctcctgctgtcgtgggagaggaggtgctcaacactgaaactgcacctgatggtaaaaatccaaggccgagcgaggctgatacggcgcagtcgccacctttgcctgaagagggcaaggccgttgcagctaccgagcctgccaaccttgaggaggcggaggctactgatgggaagtag

SEQ ID NO: 5 - protein, 3390 aa, Triticum aestivum
MASSQHVEVEAAKLLQKLILESKDEPAKLATKLYVICQHMKLSGKEQSLPYQVISRAMETVVSQHGIDMDALRSSRVPFAGGPQAVDSSGVMSKDKEIIGGQSSMVGSDASQSSGQAALWHLPPGSADMARPGVYIPGRVPAGQNRGDVAGSDIHQGSMSQKSGRSSGVESPASLQMEDTRSMNSHDSLKSDEKTSKKASSSKRKRMDSKAAGDMQSEENSKSDGISSGQNIRKRKQVGKAGAQGQPSRGAEPEQSHILQGATAQVPPLPGGASFFRAHQEGPPASAGRTIDNTKPSNPFAMSQVSNFAEGLASGSIPTELQKSILGGTNMFNTGFGWNQSSQGSAIKNTQGSVANLMRPGVKVEGKINVGSQGAFNPTPTSQMDFPKIPPYMSSSFGGGSQFLDKGKDSASGNTGTELHSAAKVGVNMGIVHGSPMQERQNITRAPQRAESSLQEARLSSLPNRNVGPYQTSHISPNTPFKEQQLKQLRAQCLVFLAFRNNMQPRKVHLEIALGGGPTAEGGGAGQGGNESRVADGSVRENGNSQENSAIFGSQSDMSRLPSTSAGSIAEADSSLKDSEIKKKINIAEHEKSSMEMENIQQAVMQGTGSSSEMRSQEIASPVPSGPQQSYFQGDKRRNAPEAYRTDAENLNRNLSFGGQGPSSLGGNRQHPNFEAAVLTKDRLQDEASKESYPPSRLHHMPIDGYNSNLPGKDLTPDTDRNEVEHCTQMGEMSDRSADEGDDDLFEHDDFASTPPKYTMTEKWIVDYQKRKYGENEKKVLEQQSAHKRMSASYQKLKESVSSSEDLTAKTKSVIELKKLQLLSLQRRVRSEFLSDFFKPNTADLERVKAVKKHRHGRRVKQLEKIEQKMKEERQKRIRERQKEFFADIESHRERLEDSFKAKRERLKGFNRYIKEFHKRKERIHREKLDRIQREKINLLKNNDVEGYLRMVQDAKSDRVKQLLRETEKYLQKLGAKLRGDSSMDGRSYVSGKGVTANDVEDESYQPQNYLESNEKYYQLAHSVKEIVNDQPTYLNGGKLREYQMNGLRWLVSLYNNNLNGILADEMGLGKTVQVISLLCYLMETKNDRGPFLVVVPSSVLSGWVSELNFWAPSINKIAYFGPPEERRRLFKEMIVQQKFNVLLTTYEYLMNKHDRPKLSKIQWHYIIIDEGHRIKNASCKLNADLKLYRSSHRLLLTGTPLQNNLEELWALLNFLLPNIFNSSEDFSQWFNKPFESNGDNSADEALLSEEENLLIINRLHQVLRPFVLRRLKHKVESELPGKIERLVRCEPSAYQKLLMTRVEDNLGGIGAVKVRSVHNSVMELRNICNHPYLSQLHVEEIEGHLPRHYLPSIVRLCGKLEMLDRLLPKLKATGHRVLLFSTMTRLLDVMEDYLVWKKYQYLRLDGHTSGHERGALIDRFNDPDSPAFIFLLSIRAGGVGVNLQAADTVIIFDTDWNPQVDLQAQARAHRIGQKKEVLVLRLETVRTVEEQVRASAEHKLGVANQSITAGFFDNNTSAEDRREYLESLLRECKKEESAPVLDDDALNNILARSEDEIDIFESIDKQRLDDEMAVWLKVVQDGSVSGLDPSVLPPRLVSDDDLKPFCHAMKIYESSNVKNVKVNVRKKGELGGLDTKHYGRGKRAREVRSYEDQWTEEEFEKLCQAESPDSPQPGGVLKDIDISKESKLEVPAESSIDPKESSIDPVEAKTVPVLAVPDSSPPVPSVPDSSPAKRRRGRPRRSDVSVSPVMSPAKAVQQEAGTTLGSSAPASTIDSAAPTATIHSTGPDVTTHSAAPVAAIKPDIGAEVKATAFVAAVPTATMKPEIGTEVTDHVVLEGSIAKEVGPAVESGHDPVAASAAPHPPAPATSRGRKTQTVETPRRRGRKPKSLSSSSAGDVNINPVVAIGSGPASVGSPYPQGDMPASLMSRFQKDLVTGRPVTSLPEAVKGISAPEGTTPVAEDKHTGTAISSDNASLLMPKIIHNENVGFVQVSSEQVFSASVPTLTAVSGGILKASHILLADKPAEKQSASRRRRKKAPGGEDTGVSTRQRAAMKKSDGIPGTTDNVGADTSTAEKLGAVNVKDGSSLQDTPKELPNINSPPYDKSGYDSQPRTPIAVPISEAALPSGSGNAHVAYSDITPRIPTNPDVQDKPVNLHIGAPLAAATQPEVPCKTGNDHVAVCSVVTTTHSETVTEKPLLNPVSEVANVQVEAPSSSLHNSGKNISTVPSEVNSVAPSKASGRRRKGPASEPRTRSKAATAACERRARLAGPKQTGDARKLEILASPSTAVCVSSVEQQETALAEPLTASVCEPQKNAESHVRGGMSTPTGILDAPKQIATQSITACTEETNNSLSTQTPALPISRESILSMGDKQGVGVDTIHGQTKMVLAAELTSANDEHKLHEVHDKTADGNILQHSAANDTLQDKTDSIAGLDLASRHRIGDLEMEKGDSKTVMLPDCQTPFDASVKDINDTLAPTEADVSDLQSEAAAIDVTSPKQDTMVVEALYTNPGGSASHLPAALQSTDSNQHAERKGSSDNSGSKIFASGKKTEEMEGTLDKNTDHNLIQANANIALGRYSPSEDKREDSCAHVVDGGLLGSKQTLPEVVSAVNTDGSEEALNASSTHSNKDATLVCEVTKDPESHVSVSVLASAAMNAGDDSEEVHNVPSTHSDRGGSMVEVDASRDDATSICEVRKDPESNVSGELSMPVRLAELELELPNQSKSSSQSSAVNADETKASINIQTTSLVESGEQKSPRNGAHELKEGMELAGPKIECTIQMPSPDDKSSEAHSLAQREMVSGAEQASMKDDKENKMVDVTFSSGGEQETQRADVDLPTCPTYADCEGEKDDSPKTILAGSQSFCEASDKDVAPVRDDHTDPQSEVIVVDMNDANQDSAEAEAMQIDSVSKGSSSDLPAALRSTDSNQLAEQVSPCPKEHEKLEETSGEIGGGNSNRSRTDGDSHIMNLVGYSEDSDEDDSIQVADVGDVGSKETTHYDISAVARGAEPGDGPCTEPTCETAVHVHECNADVAISEDGHGTTALGSVQVSTTELKDLESGRCLEHGIGTPVALQEGTAVATEPEAKKEVDEPTQNEDVELAAIKPEAVEHAGTEADPSKEASIPPQEETTAVALVTGPEQNEEADAPTQVEPVAIVPDSMEHASTEVDQSIETSVRLPEKTSVIPGTEPEEKKVEASSQEDNVEAVAAEPEPAGSQENAEVSTKPSPMEIESVQETAMLGEAETRQQLPLPSAEGVVAEASEPPEVTAMKEPELLSTEPAPDGENAKLGEAKAEQLLQQPSSCEAMAAVTGELPSAAGAKTDGTSDVVADESPAVVGEEVLNTETAPDGKNPRPSEADTAQSPPLPEEGKAVAATEPANLEEAEATDGK

SEQ ID NO: 6 - DNA, 30970 bp, Triticum aestivum
  source 1..30970: mol_type = genomic DNA
  exon 1..229
  exon 4915..5028
  exon 5107..5168
  exon 7938..8143
  exon 8218..8940
  exon 9029..9231
  exon 9647..9846
  exon 9927..9991
  exon 10071..10900
  exon 11073..11170
  exon 11279..11464
  exon 17362..17542
  exon 17691..17855
  exon 17934..17977
  exon 18216..18272
  exon 18418..18514
  exon 18622..18794
  exon 18871..19084
  exon 19271..19396
  exon 19480..19569
  exon 22063..22179
  exon 22278..22358
  exon 22445..22552
  exon 22705..22874
  exon 23012..23090
  exon 23173..23247
  exon 24210..24307
  exon 24391..24498
  exon 24606..24663
  exon 24747..24968
  exon 25053..27240
  exon 27328..28491
  exon 28618..28692
  exon 28765..28830
  exon 28913..29683
  exon 29786..30970
aaaaaaacggggaagaaaaaggaggcaagcagtgcacaggtctagtggaaaatggcggaggcggcgtgctcgacctcgggcacgtagctcacgcgcagctcaccgttccccgtcgcgctctccagagaccccgcgccgccgccggcgaccagcagctcccccgtgcggcggctccgcgtctccacccgtctcgttctcccgctagggtttcccccgatccccaatcactgtaagccgcgaagacttgtctcgctagtttccttctggtttaagctcacgggagcgtgcgcgtggtccccgagtgggtggatttgggggttgcggtctcggatcttgcgcgatcagtgtagcgctgttcccagctagggttagttcgtagaagcataagctgggaactgaaactcgtggagccttatgtcatttgggtcagcgagctgcttctgtagcgagaacttataagctctgagcgcgtcatgtggagtaattggcctattctgtgcaataatcccatctttaaacattcgtctcttttccggttccgttagggatcttttgggtgtgacttgggtttattccttgtatgcattgcctagtcatgacctgattggttagcttttagttgcacttaattggtcggtgaattgtgttatagggtgggatgtcttgttagtgaagcttgatcagtatcatgcatctgattgcttttctcaaagagtggcactatttttttagaccaaatgagtggcactatttcgttgttatccacagaatttttagcatgtggagcggtcccacgctaccatgaagcaagaaataccagtttttaactttagctcagcatatactgatatctctgctactttctctagagcagcttgaatgcacgccattgtgatgcctgctattaatttacatagcattacatgtggtgaacatgcaaattctatagcaacttttttggaagttctgtttttggtagctatgtaactgtagagtatgcctgtttgcaatttactaaacctgctgctctgcattaacagtttgcatctacaaagattagctctgaaattcatgctgctgtatctgtactctctttcgaacttggatccataataattttgattccaaattttaaagacaaaatctctaaaaccctctataagcatccatgatttctcagactaaaaataggaggggcatggcagcgatctccataatctaaaaacaaaggagtatgatcagaaacctcgctagcaaaggcttgcaacatagacaaaggacaatgttcctcccatttagggcagaagaatactctatctagtttttcaaaggtagcatcctccaaattatttacccacatgaaatttctcccatttaaaggcttctctctcaactcggcgtgttaaaaatgatgtattaaacacaaaactctagtgatcagtatcattggatttgtttttttcacagctctttcctattatgttaaaatccccacctactaaacatggtagaggattatcatgatatattctagccaactcatctaggaacttagcttttccttccaagtgcgcatcaccataagcagtaatgagatccgaattaaatttggcaatcttatcaaaaagtaatattctaataaagtactctcccctctccacttggataatatcaaacacatttttactaatacccactaaaatcccactggacctccacctaggatgatttcaatgccactattttttttctaccactcaaagagtgtagttcattgttagaaaaaaaatgttttctggtttccaaaagaccaataaaatccaatctatgatcaattatcgtgtggtgggccttggagaaacacaaagtcccagcaaagtacattaccctcatcaaggacatgtacaataatgttgtgacaagtgttcgaacaagtgatgtcgacaccgatgacttcccgattaagataggactgcatcaggggtcagctttgagcccttatctttttgcattggtgatggatgaggtcacaaggggtatacaaggagatatcccatggtgtatgctctttgcggatgatgtggtgctagttgacgatagtcggacgggggtaaataggaagttagagttatggagacaaaccttggaatcgaaagggtttaggcttagtagaactaaaaccgagtacatgatgtgcggtttcagtactactagctgtgaggaggaggaggttagccttgatggccaggtggtacctaggaaggacacctttcggtatttggggtcaatgttgcaggaggatgggggtattgatgaagatgtgaaccatcgaatcaaagccggatggatgaagtggcgccaagcttctggcattctctgtgacaagagagtgccacaaaagctaaaaggcaagttctacaggacggcggttcgacccgcaatgttgtatggcgcggagtgttggccgactaaaagacgacatgttcaacagttaggtgtggcggagatgcgtatgttgagatggatgtgtggccacacgaggaaggatcgagtccggaatgatgatatacgagatagagttggggtagcaccaattgaggagaagcttgtccaacatcgtttgagatggtttgggcatattcagcgcaggcctccagaagctccagtgcatagcggacggctaaagcgtgcggagaatgtcaagagagggcggggtcgaccgattttgacatgggaggagtccgttaagagagacctgaaggattggagtatcgacaaagagctagctatggacaggggtgcgtggaagcttgctatccatgtgccagagccatgagttggttgcgagatcttatgggtttcacctctagcctaccccaacttgcttgggactaaaggctttgttgttgttgttgttgttgttgttgttgttatgatcaattatcatttccctaacatatctcttttggagatcttgtcccaaacctctaacaattcaatccaaaagacctcttgcattacaacttggatggaccttaggcatgagtccggaagaaggtttcgaggagtcgcatcacaagcccgcgaccatccaccccatcccacgaggccttcctaacgcaagattccgtgctttgtcgagacgacgaaacctattattaaaatattgttgtatttgtttttgtccatgtacgtatgaacccaagctaactatactcaaaaccgcgttacgaagaatacctctagttgggagttgttttcataacaacaagcctacaattacaccttgttatatttcattgagatggtcctagatttatgaaatggaatttgatcctgaattttccgtttccacgtcaaaagtgtatgaattggaatcgtgattccactccgattccaacatttgcttttcgagaacaagactgacccagtttttctttcgttcgattctcctagaatcttgagaatcgggagaaagaacttggcctccggcatttgtttagggataacacgccatggccctggccccaacgaagctgaaagcccagcccaccgggtacccactgccctcggccctcgggcctcggccctcacccatttccactagctaaatactggtaaaccccccctcctctctcccccaccccaccacacacacaagacagcggccagagaagaggaactgaaaagaaaaaaagggaagaaaaaggaggcaagcagtgcacagatctagtggaaaatggcggaggcggcatgctcgacctcgggtacgtagctcacgcgcagctcatcgtttcccgtcgcgctctccagagaccccgcgccgccgccggcgaccaccagcttccccgtcggcggctccgcgtctccacccgtctcgttctcccgctagggtttccctcgatccccaatcactgtaagccgcgaagacttgtcttgctagtttccttctggttcaagctcacgggagcgtgcgcgtggtccccgaatgggtggatttgggggtcgtggtctcagatctcgcgcgattagtgtagctctgttcccagctagggttagttcgtagaagcataagttgggaactggaattcgtggagccttatgtgatttgggtcagcgagctgcttctgtagcgagaacttgtagctctgagcgcgccatgtggagtaattggcctattctgtgcaataatctcatctttaaacatttcgtctttttcccggttccgatagggattatttgggtgtgacttgggtttattccttgtgtgcattgcctagtcatgacctgattggttagcttttggttgcacttaattggtctgtgaattgtgttatagggtgggatgtcttgttagtgaagcttgatcagtatcacgcatctgattgcttttctcaaagagtggcactatttgtttttagatcaaatgagtggcgctattttgttgttattcacagaatttgtggagcggtcccacgctatcatgaagcaagaaataccattttttaactttagctcagcatatagtggtatctctgctactttctccagagcagcttgaatgcatgccattgtgatgcctgctattaatttacatagcattacatgtggtgaacatgcaaattctatagcaacttttttggaagttctgttattggtagctatttaactgtagggtatgcctgtttgcaatttactaaacctgctgctctgcattaacagtttgcgtctacaaaattagctctgaaattcatgctgctgtatctgtactcaatgtactgtatttgattatcgaaatctatcacgtttgttttcctacattaactaatggcgtactggtttgcctcttataacttataatttatataatttatttatcttctttttgattgatcttattttgatggcaagcagagtttgcaaatggcttcatcacagcatgttgaagtggaggctgcgaagctacttcaaaaactcattctggaatcaaaggatgagcccgctaaattagcaacaaaactttatgtggtatgcagcgcaaccgatatacaggacatgaaaagccttaactcaaccataaccttgtttctttgttcaatgttctagatatgtcaacatatgaagttaagtggaaaagagcagtctcttccctatcaggtcatatctaggtaaatatttcttttgttcttggctatcttttcagaagttttttttgccatcaattttactgtaaatattagtcaaatattctgttagaaaaacactactctctccgatccatattaattgatgctggtttagttgtattaactttgtactaaaccagtgtcaactaatttggattggggggagtagttaaagttctaccttgtgtcttagacatgttgtcttgttattcttgactttcagatttgataattgttgatgtgttgttcttatgttcgaaagttctgcttatttaattataattatgccatcatcaaactagatttcacacatcagttagtactcattgtcaattctggaatagcatacaaggagggggcctaaccatctagatgctgttgcagcgaggttgtagcttggtactctccctaggtactaaatgttgctccaactagtttaggtgaagaaaataggaataagcagaaagaccagacgcccctggacacaggctcaatgagggagacaggaggggattgaagctcagtgatggacactttcctcatctatgtagtgaactgttaatacacacttacacagtagtacgatatccacaaccccaaaatgcatgggcaaattgaagttcaacatcctccctctgagcagcctttctcatggagatggagattgaggagggagagaagtcgttggaggatggcaagagggagcggcagagaagtgcaagtaggagtaagatgggagtagcgagctgtcatttggaggcttacaactgataatatttgtcttttggttgacatgttagcctgtagtaatagatcttgattcttgaaatcctctatccttgatgggagtagcgagatttttaagactatttgattgtgtttggctgggctgtggattttgagcttggcctgggcctgagtttggtgctgatttgtgcctggccaggctggcctgggcatgaagcgtttggttggtggcctggatgtaatagcctattggttgatagtagctctgaataaaatataaataaaagctctagacaaagctatttgcatgggatagcgtgcccaggcaggtttatagatggccaggcatccatttccatacgcctgccccaggctaacgcccgtgcctggtgctccagccaggctaatcaacatgaaaaatgctccaggccaggcaagcatttcattgctcaggacaccatcgaaacaacctccaggctagtatcaggcaagctccaggccaggcataaagaggtgaggaagcgaaccaaactgaccctttctgaaagcagatgcaagagatgtaccgtgggaaagctgctgtggacggtgtgttgtgagaaagctgtgaagccatttggcaaactagctgtctgaagtgcggctgcggggataaatgtctgaaatacccttaaaagccgagacattggatacatactgtttaatgataaaaacatcattacaggttgacctagttcgtaaatatagctattcaaccagttacctagttaattatttcatggagtttttgttttaatgcatattaataaaaatatatatagctctacatatcacaaaatagatgcaccagtgccatacaaaatttacatatcaacagacacatcaatctggttccagtctgaccataggctactactgccatacaacataaacatatcaccaaaaaatgcaatggtcgtacatctccagtggggcaaatctggagaaaggaacgacatgtacatgggcgagggaagcggcagtagtacacctcgaatgggggatgtagcagaggtcaggcagccatggtcggcggtggccttgctcgtccgagtaaccttggacactggtggaggtagatgagggggtgggggtggagcagggaagaggagtccaattgaccgaggtggatgaagggatggaagcatccaccggcggtcttgcggcgacgtgccgtcagtgacatgggagcgagctggtgaccagcagctggccggcggtgctaatgaaccctagaatcgccagaggtgggggacgagaaaaggaccttactcgatgggtttggtagagctgtctctcgtggacgtaccggctggattattttggcggtgaaggtgagtaatttgatctcaagtggatgtaggttcagggagccatgcagccaaagccagaaaagcacctcttcgtccgctttcactcgtacatgtgttttgcgatggctttcaagggaatcgcgttcgctcgttttgccgtttggttgtgatttcagctctgaaggagagaaatccacagcgaaagccaaaccaaacgcagcctttgccttagacaatttaagagtgtagaaccttgcgcgcaccatttgtctggaatcaatcatcagtgctgtcaactggagctatcgttttccataaatttggggttgtttttgcaccaaaagaattaagtatcttttgtttggtagagcttatactccattatgatattgagtgcgttatggtttatactctatagtaggtggtgtcagatgatttaccaaatgtactgtttgcaacgtgtagtataagtatagtaatacaaataatccagtttggttaggtttactgtacctgagtgtttgtaatttcaaatgaaaggattctgtgtatgtcagagagttctatcaaactttcaatttttctctagcttgacttctctcctctttctagtttctaagatgcccataacatccgtaatttttgcctgcagggccatggagactgttgtaagtcaacatggaattgatatggatgcactgcgatcatcacgagttccatttgccggcggtccacaagcagtagattctagtggcgttatgtctaaggacaaggagatcattggtggtcagtcttccatggttggaagtgatgcatcccagagcagcggtcaagctgcattatggcatttgccaccaggtaaccaaccaatttggaaaggaaactgcagtcactgttttggagatgtgatatgatttattttatattattaggttcagcagatatggcaaggcctggggtgtatattccaggcagggttccagcaggacaaaataggggtgatgtcgcaggatctgatattcatcaaggctccatgtcgcaaaagagtggcaggtcctctggagtcgaaagccctgcaagtctgcaaatggaggacactagatctatgaattcacatgattctttgaagtccgatgaaaaaacaagcaagaaagcttcctcttccaagagaaaaaggatggattcaaaagcagcaggggatatgcaatctgaagaaaactcaaaatcagatggtatctcaagtggacaaaatattagaaaaaggaaacaggttggcaaagcaggtgcacaaggtcagccctccaggggagctgagcctgagcaatcacatatactgcaaggtgctactgctcaggtgccacccttacctggtggtgcatcatttttcagggctcaccaggaaggtccaccagcttctgctgggaggactattgacaatactaaaccatcaaacccgttcgcaatgtcacaagtttcaaattttgctgaagggctggcttctggtagtatccccactgagttgcagaaaagtatactgggaggaacaaatatgtttaacactggttttggctggaatcaaagttcacaaggttcagctattaagaatactcaaggttctgttgccaacttaatgcgaccaggagttaaggttgaaggtacttccattaaaaaataatgacataacagcattgtgaaagacttgaattacaaatatttaccttaatgagcttgcttatactgcagggaaaattaatgtagggtcacaaggagcttttaaccctactcccacatcgcagatggattttcccaaaatccctccttacatgtcttcctcctttggaggtggctcacagtttctggacaagggcaaggattcggcttctggcaataccggcactgaacttcattctgctgctaaagttggagttaacatggggattgtgcatgtaaggcctgtagtttaatccttaaagacccggggtgttaacatgctatttcggctacagtttggcccttctaaaaaatcttttaattgaaaagctaatattttttgctgtgttcgccaatggtaacctgttacggaagtgcctagtagtaatggtataatgcagggtattcatttgcataagattgtactcgagcttcgaacacaagtgtattgcacgccggtttcgtgtatgtctatttgcgtgccttgatagactttctgccaggtttcaggttgatcaaccgataaataagctgtttctgcctgcaagattaataattttgttgtctggtcatttagtgatatgttaattgatttctgtatctcaagtagaggtgctttatttgatgcatccatgtaatacgactttgcagggcagtccaatgcaagaaaggcaaaatattaccagagcaccacagagggccgaatcatctttgcaagaagccagattgtcttcgctcccgaatagaaatgttgggccatatcaaacgtctcacatctctccaaacacacctttcaaagaacaacagttaaagcagctccgagcacagtgcttagtatttcttgcattcaggtacatgcttagagcactgtaggatgattggtatccgaagttcatctctgtagtactaatttagctactctttcttgtagaaataatatgcagcccagaaaggtgcaccttgaaattgccttaggtggaggccccactgcagagggtaagaactaagaacagaaaacattgtgtgagctgacaaggtttctgtactcatgatgagcttataattaaataaacaggtggcggcgcgggtcagggaggtaacgagagcagagtggctgatggttctgtaagggaaaacggaaacagtcaggaaaactctgctattttcggcagccaaagtgatatgtctagactcccatccacatctgcaggcagcattgcagaggctgactcttcactgaaggactcggaaattaagaagaagatcaatatagctgaacatgagaagtcatcgatggaaatggaaaatatccagcaagctgttatgcagggaactggttcaagttctgaaatgcgctcccaagaaatagcatcccctgtgccatctggaccacagcagtcatactttcagggagataaaagaagaaatgcccctgaggcctacaggacggatgcagaaaatttgaacaggaatttaagtttcggaggccagggaccatcttctttgggtggtaatagacaacatccaaattttgaagctgctgttttgaccaaagatcgattacaggatgaagcatctaaagaatcatatccaccttcgaggcttcatcacatgcctatcgatggttacaactccaatttaccaggaaaggatctaactccagatacagatagaaatgaggttgaacattgtacccagatgggggagatgtctgatcgatcagctgatgaaggagatgacgatctatttgagcatgatgattttgcatcaactcctccaaaatacacaatgactgaaaaatggatcgtggattatcaaaagagaaaatatggagaaaatgaaaagaaggtattagagcagcagagcgcacataaaaggatgtcagcatcctatcagaagttaaaggtctctctctgccttcctcacatttatttttgaaatgggggagtgtcatttagaaatactgtgtacatatttatgagtttttgcgagttcctgtttcatatgtccagttttccctcactgtagcagctgtaattgttggttgcaaaattttaagttcttgttcatcctacaggaaagtgttagttcatctgaagatcttactgcaaagacaaagagtgtcattgaattgaaaaagcttcaacttctctcacttcaacgtcgtgtgcgcaggtttgcttgccattggagatcatcagtcttcagtttctctccttgtgcttaccgtatgtttctatggctgtaacttccctattctaatttcttgcttatattgggcagtgaattcttgtcagactttttcaagcctaatacagctgatttggagcgtgtaaaagcagtaaagaaacaccggcatggacgccgtgtgaaacagcttgaaaaaattgaacagaaaatgaaggaggaaaggcaaaaaagaatacgtgagaggcaaaaagagttctttgctgatatagagtctcacaggttggatgactatatttgattcttcattctgacccctttagtatgtagatgttatttaaattttttcttacgcaatattctcaagtatttgtggcatctatgctccgtttttacagtactgatgatttggggtctatttggtatttgccaatgcagtgactatcaagctttactttcattttggtattgtgtataggctaatatcatctgcattagagccacaacaaaagctgtttacattattcttgctgttgtgtcgcagactcaccttgttttggctgtttcgtatgtgtgtgtggcggctctgctaagaacgggaggactggatgcctccttctaggtcagtacctccacatgggcttgggccctaagtgacaaggcttgatgggcttgggcccataccggttcaacactccccctcaagatgggtggtagatatctatcatccccatcttgtcacatgccaagttacagtccttcgttcccagtccctttgtcaagcaatctgcaaactgctgcccagagctgacgtgagtaagactgatgataccagcatcaagtttctccttaatgaagaagcgatcaatttccacatgttttgtcctatcatgctgaactgggttattagcaatagctatagctgactgattgtcacaccacaccttcaagggtcccttcctcagaagtttcaactcgctcagtaggtacttcacccagagcatctcacataacccttgagataaagctctatactcggcttctgctgttgatctagacacaacaggttgtttcttgcttctccacgacaccaagtttcctcccacaaacacacagtagccagaagttgatcttctatcatcttgacaactggcccaatcagagtcactatagccatccacttcaagatgtccactcttcgcaaaccacaaccctttacctggagtccccttcaagtatctcagaattctgtgcacaatatcaagatgcccactccttggttcatgcatgtatctgctcaccacacccacggcatacgtaatgtcaggcctggtatgacacaagtacaataacctcccaactagtttctgataatcttccttattcaccagctcgcctgactgagctgtcacttgatgattttgttcaatcggcgtaggggctgcacggcatcccatcatgcccatgtcactcaagagatccaaggtgtatttcctttggcacaaagatattcccttctctgtccgggccacttcaatcccaaggaagtattttaggttgcccaaatccttcacctcaaactcattgctcagacaccccttcaatctctttatttcctcctcatcatctccggtgatgataatgtcgtccacataaactgcaagaatggtgatctttcgattagagagtgagtgtctgtagaacaccgtgtgatcaccattacattgaccataccccatagcacggacagcacgcctgaacctatcaaaccaagccctcggcgattgcttcagtccatacaaggatttcttcagcctgcataccttccccgttgtcagtgaagtaccaaaacctggtggtatctccatgtacacttcttcctgcaactcaccatgcaagaaggcattcttgacatctaattgatgcaatttccacccaaagtttgcagcacaggaaaccaatatccttactgtgttcatctttgccactggagcaaacgtctcgtcatagtcaattccataagtttgactatatcctctggcgaccaatctggccttataccgttccaccttcccctcaggattctgcttcactgtatagatccacttacaactcactgctttctttcctgccggcaatgtggttagcacccacgtcttatttttcctcagtgcttccaactcttctatcattgctttatgccacttcggatcttgctttgcagccttccaatcctttgggattgacacagtttgaagagaggcaacaaacactctataggaaggagacaaagcctcataagacacaaaatttccaatgtcatgatcatccaaaaactccagtggtaaagccttctcagccgcttcacgtgtcccctttcgcaacgcaataggtagctccactgtgttagatgagcttgcaccactgccttgctgctccccctgcactgactgctccccctgcacttgttgctccccctcctgcacaagtggctgccgccgagaatataccagacgagtgtcagatgagtcatgcacctgtggcacttgtggctctcgccgagagtacactagggggatcttctgccaccgatctcgaacagggagctggagattaccaatctgaatggaacccacggttggttggacccgtacctgcacatcaccatcaatgagagtaccaaccgaaattgtacccacaattggctggacttgaacctgcacatcatcatcatcaatgttagtgcccacagaatccgcgtgagtgtgagatacagccttctccccatcttgaccatcttgcacagagtggaaatggtcaagctcttgaaacaacacacttagatctgttggctcaccatagaatggctcagactccctgaaggttacgtccatactgacaaacctgcgtttctctgagggacaccaacatttatatccctgctgactagaagaatagcccagaaaaatacacttcactgcccgcggatcaagttttccaacagaaggacggtgatctcgaacaaaacaagtactgccaaacaactttgggggaacaacaaacttagtttctccatatactagctcacacggagatttcatgcttagtattcttgatggtgtcctgttgatcaagtatgtggctgtcataactgcttcactccacaagaatttgggcacattcatcataaacatcaatgaccgggcaacctcaagaatatgccgatttttcctttctgccactccattctgaggaggggtgtctgggcatgaagtttgatgaagaataccgtgatcagacaagtaagccccaaatgtgttgttcacatactctgtcccattgtcagtcctgatcacctgcacctgcacctgaaactgattcttcaccaaggcatggaaattctgaaaacagctaaacacctcatctttgtgacgcatcaaataaatccaagtcatacgagaatagcaatcgatgaatgtaacaaagtatttcattccattcattgatacaactgggctcttccatacatccgaatgaataagcataaaaggagatatgctcctaagccccttactcacatatgaggctcgtgtgtgtttggcatattcgcaagcatcacatgtcaacttgcccttgcctatcccacacataacatccggaaagattctactcatcttatcaaaagatatatggcccatcctacagtgatggatcatcgcctccttctccttgtcctccatggtcgcagcacacaccaagtccggctgcacctcctggtccatgtaccagagccccctacgcctggtgccagtcccaaccgtctgactcgtctgtcgctcctgaatcacgcacccgaatttgtcaaggatcacacgacagtcaatttgatcaattagagcactgaaagagaccaaattgacaggaaaagccggcacatgtaaaactgaggatagggagatggtcggagtgcacttgactgtgccaacccccatgacaggctggtttgtgccatcagcagtttgcatagtgcgcgggtgagatggagggtgcttattgtaagactcaaacatgcaggatttactagcaacatgcttagatgctccagagtcaagaacccactctggagcactctcattagaagcaagagatgccttttccggattaccttcatcagtggaggcccagagagcaaagtctcatagttagcatcatctgcatctttgccttttgacgtcccagtgtctcctgccactgccatgtgagccctctgatctcctgagtgtcctgagtaaccacctctgcccatagaagcctgaccccttgaggtccctgagtatccacctctgcaagttccccctctgttgtatcccctgcctctgccacgagttggacaggcccacttccagtgacctatctccccacaaagatgacatttgttgggatcgctccactccatgcgctcagtgacagcaaatgtcgaagccggcacagccttcatgtctgcatgctcaagagatagccgcacctcctcttgagacattgcagcaatagcctcctcaatagagggcagaagaggttggtgcaacagggaagccctcctgccatgaaagcaacctctaagaccctccaacagtttcagcacacgcctgcgtgcaatccacttgcgccctgactcgatgcaagccgcatcatagagttccagagggtcgcagttatcctgctctgcccacagagcctgcagctctgccacatatgccatcactgacatgtcgtcaccttgatgcagccgactgatcttcccctcaatctgagcaattagcatgacattgcccttgcctgagtacaaagtggacagagtcgtccatatcgcagcggatgtggatagcccctccacagagcgtccaatggggggcactaccgagttcaacaaccagccaatgagcacagagtttatgaccttccatctctttccctccacagtagtcttgtctcctggttcagcaacaacatccaacaagtgcccatcaagctccttctgttccacagccagcaacgccctccgggaccagctcagataattggtagtcccctctaacttcatgtccatgggtgacagttcgatcttctgagccacttcctgtcgaggaacgatggccccagatttcgactcctcgaggaacttagctagcttctcgaaagcctcagcaaggcctgttggctcactcatcttcggagacaggctctacacacccaacaacaacagcagcaagcacagccgcacacagtcctctgcagaatcagcagcaacagtccgctgcacacatacagcaaggccctctgttctttctccccctctgctcacactccgcacgcgcagcagcaacaataagcagcaccttcctctcttcaatcccagcagccaggacacaacggcaacgagcagagccgtgcggactcgctctctccctccgcgcgaacgacagcagcacgcctctcctgctctccacgttcgctgttcctccggctcttctcctcgtcctgcgccacagccgcacgcctccacgcgcacagccgccgttgatttcccgctggcccgcgcagccgccgtgcgctcgccgccgtgacgcgcagccgcacgcgcgcgctcgcacacagccacgtccgcccagatgcgccgccgcctccccaccggactccgccgccggccggcgactaggccaccgtcgccgtcgtccccagcacctcgcctgcgtctgataccatgttgtgtcgcagactcaccttgttttggctgtttcgtatgtgtgtgtggcggctctgctgagaacgggaggactggatgcctccttctaggtcagtacctccacatgggcttgggccctaagtgacaaggcttgatgggcttgggcccataccggttcaacacttgcagctaaataaagtccatggtggagcacagcaaaaacaagctggccttaaataatcaaacataagtaagctaagctgaaataagtaaatggtggtttttaagtaaacatgttgctaaaagaactggatcagaatagctgattcaacctagtcagtagtcacctttgtaaacgctgcctgtctgtgtttacaccccctcaacattttacccatgtcatttggtaataatgccttgcctttgtaacttgcagagagagactggaggatagtttcaaggctaaaagagagcgtctaaagggtttcaatcgatatataaaagagttccacaagaggaaagagcgaattcatcgggagaagctggataggatccagcgggagaaaattaacttgcttaagaacaatgacgttgaagggtatcttaggatggtccaggtgagtcttatttgctttgtttctcatcatgttcttctatattagcttaacccttcacacgtcaaaaaaagaaaagcttaacccttcattttattttctcaatatttattggacgaagtcacatctgctaagtgttactgctttgcaggatgcaaaatctgaccgtgttaagcaactactacgagagactgagaaatatctacagaaacttggggccaaattacgaggtgacagctcaatggatggccgttcttatgtttctggtaagggcgtcactgcaaacgatgttgaagacgagagctaccagccacaggttttattatctctttgttttagtcaacgtctaggtgcatttttgttgaatatttacttaattttgttctcctttcagaattatcttgagagcaacgagaagtactatcagttggcccacaggtactacatggattaaatagactttcatgcttcatttagtaaatccttatcaatgtctgcctagcataaattatgtactacctaactttctaatcctccatcttattcatactttttttttgaactttaccatcttattcatacttctttgccattgaattttctaattcttttttttgagattactgaacttactaattctgccttgtattcatacatatttgtttattttttctagtgtgaaggagattgtaaatgaccagcctacttatcttaatggtgggaaattgcgggagtaagttgtgctgctattttccctgcttttacctccttttcattttaagtgtattttgacattattgttactgacttgtgtcctgctacaatctgtttaaccatccagtacatatttccttgatctattacttgctgtattacaggtaccagatgaacggtttgcgttggctggtttcattgtacaataataatttgaatggaattttagctgacgagatggggcttggtaaaacagttcaagtaagatccagtacaacgccatctcaacatttattgttcggtttgtatgttatctgatctaagcaagtgtctgaattctgcttacactgcccttgctactttctcaggtaatctctttgttgtgctaccttatggaaacaaaaaatgaccggggcccatttcttgtggttgtaccatcctctgttctttctggatgggtatctgaactcaacttctgggcacctagtataaataaaattgcttattttggtcctccagaagaaaggcgcagactgttcaagtaaattctgaatttatagttcgatactttgtcacagttcatgtgaacattttattaaccaagctaattttttcagagagatgattgttcaacagaagttcaatgttcttttgacaacatatgagtacttgatgaacaaacatgataggccaaaactaagcaaaatacagtggcactatataataatcgatgaagggcaccgcataaagaatgcgtcttgtaagctcaatgctgatctgaagctttatcggagttctcatcggctattgttgacaggaacacctctgcaggttctaaagcttgcacttatactttcacacttgatcctgtatttgttgcttttcaatgaatgttcttttcaaggaatgtatgaacggcttgctcatatatttatttaatggtcttgggtctctgtatgaagtattctattatgcatatatgtcaagttgctaacttcttgtaacttcttcttgaagaataatcttgaggagctgtgggcacttttgaactttctgttgcccaatatatttaactcatccgaagatttctctcagtggtttaacaaaccatttgaaagcaatggtgataactcagctgatgaggtaatgctgccgtttttcatgatacaacattgttttcttggaaggaaactgtgtttgactccaatcatcttctttcttaaaaggccttactttcagaggaggaaaacttgctgatcataaaccgtcttcaccaagttcttcggccctttgtactccgaagacttaagcataaggtattgattttatttgctatcttaatgcttgtgttgaaatcactggcactgtaggaattcaccatgcaatttatttgaaattccaagttccaacaggagatctatgctatgcttagctattcaacctcattatctcaaactgagggagttccagccttccagaattgcatccagtgatcacattggcagaacccttgcttctaaccgaaacctagtaatagtagggagacagataagaaaataattgcttgatgtctttattgatgtgagggcctagccttatatagctggctacatagatatatggaaataaagtaacaatcttggaagcttatctagttatttaaaagaaatctaataaccagtaaccaactagagatgaaatctgttacgtatttgcttaaggcagaccagggggttagactttaggcgttggctgtatgcctaaccccacttgtcacacattataagctcatattatttgagcagtacacatgttccttaaatatgtgtgacctatcaggagttactcacagcatgtaattcggctttcaatatgtcagctgattcagtagacattgcttgatgttccttacttctttttccatttgaagtctttatatgttgcatttgttgggatgattcatgtttttgtattgtacgaatgctgagctgggcattgcagtggtgaagagctaaatattgtccataactaggttcaatagcacaacgcaacacaatatagcaacgtcaaactggttcttgttagctttgttgctctacatgatctgtaatttaaaaattccatggacaagatttctctatgtgcttgtacacatccatctagctgcctgaatgccaaaaaatgttgcttattctgtttctcaatatatgctactttggcataccagtacaagcacggtcacacttttcaagtttgaccaccaacatattaaaaacatctagattttcacatcagaaaaacactagtagctcttccactagagttgctctacaagtttttttgaaaactagttgctctacaagttgtagatgcttttatgaatgtggattttctcaactagttgccgctgcaccctactctagcatccatcgcgaaaagttctaaaaagacgggaattttgtagatgtacagtttgctataatatgcgcagctgataaatggccatttgtgtattgtgcgaaaaattaagagatgagtgtctagtatagcaactatatgtgcacacatggtcacactcactcttaaagcatatgtgcgagcattttgtatatctatgactttttttcgctttttgataaagaattacgtgctttccatcttcacattcttgtgaaatgcataagatataattttgccaactactatacaaacatataatcattaagaccatgaataggaaagcatctttcatttataaacggtgagtgctccatatttcttagtttatgattactagtaaaaggtactgattctgttcctaaatgtaagacgtttttagaagtgcaaaaacgtcttacatttatgaacagagggtagattatacgatttgaacagaaatcatggtatttggcaatgttcaaaaaatcattaactggtagctgcttggtcggctggcgataagggatttataggtgaatcggccagttaacggcaaatataccagttaattcgcctataagtcaattaatcggctactcggtgacccactgagtagggattaattggccagttaactgatttatcggccgatattctgacaatacttaattatgataattttcgatcatgtggtgtagacgtgcaaatttgttttttagaggttggtgaaccaatcttgcaaccggttcattgatttttaaaatttaatatttgaagcaaatttgttacgccaaaagtcaaaattttgaatatgaaaactgaattttttttgtgataaattttcacaaaagaataaccgaaagtattgaaattatgcctgatagttccaaatagtcaagaaaactcgatcaaactacatattaattggttcttatgctaatgaccagctgaaaaattggttttggcaggagcactgttgatggtgtgtaaatcaagttcaaaactgctgtttataagtagagattatgattactttaagttgcaacttagttaaaaaagcaactcatatgtccatgcccccttttctcttggttttgaattgatttttgtttagactttagaaccgttgatgtcgaataaatttgaaagaagcaccaatcattggagctccaaccatttgtacttctttgaaacttattcgacatcaacggttctaaagtctaaacaaaaaactactattgtgatgctgtgtgggaaactagctcgtcaggttggggatttgatattgtttcccaattgtttctcatctttgtttgtatctagaccatctggatggtgcaatagtttcaattgtgttttactgtcttcaggttgaaagtgaattgccagggaagattgaaagacttgtaagatgcgagccatcagcttatcagaaacttctgatgacaagggtggaagacaaccttggtggaattggagcagttaaggtgcgtagtgtgtgactgttcgagttgtttattttaatgtttcacttgtcagatatttcacaggttcttatttgtaatatgtgtcttaaaatttttaggttcgctcggtgcacaattctgtcatggaattgaggaacatatgcaaccatccataccttagccagcttcatgttgaggaggtagagcatgattctgccttgtcgccacattctggctatttttgtttcctcttgggcatcaccagccatatggattgtctatgcagattgagggtcatctacctaggcactacctgccatctattgtgaggctgtgtgggaaacttgagatgttggacagattgctacccaaactcaaagctactggccatagggtaagtggattttactggtagcgtggtaggtttgtaaagatctcctactcgtatgtcgcatgaattgtattttcttgaacaagtctcacatcaaacttgcattatctgagttgaagttgtcgttcgttccttgttccttccttggcatgcaggttctacttttttctacaatgacaagattgcttgatgtgatggaggattatctggtatggaaaaagtatcagtaccttcggttagatggacacacttctgggcatgagagaggagcacttattgatagatttaatgatcctgattctccagctttcatttttctgctaaggtaaaatattggttcagtatattgtggtgtaggaggcattatataaatagaacatagtgaactcatgaatccttatcggccaatttaattaattaatatttgatatctaaggcctacttcacccctgttttctgtagtatccgagcaggaggcgttggtgtcaatcttcaagcagctgatactgtcatcatatttgatactgattggaatcctcaggtagctaaagttccttcagtgttgtcactctatgttgtaagatttgttttacataaatatatcttttccttgattatttcaggttgacttgcaagcacaggctagagcccacagaattggtcaaaagaaggaggttcttgttttacgtttagaaactgtaagtgcacactgacagttcgcttatcaccaggagtaaatatgtagaaactgaaatgaacaaggaacatttgtttgctaacaaggagatggtagttaataaatagagcaagtcgccagttgagtcctttgtgttgcatagggtttgtttgagcatcttagatcaatagttagatacgtgacttatgtggtattctaaatgaagaactggtccagatttactcaataccactccaccatggggatgggcccccatgcataaacagcaccctgcttgcactttcttcctcacttcatgtaaaagggttaattcggaggtgcaatgttttgactcatgactcatcatgcattatatgctactatgcccacactagaatctggattccaatactgcttgggttttcctctctttgtgccaatttgtggctgttgtgttgctgcgctgccttggaacctagctatagggatctttactgttttcttgtatattttggtgatataactccaaaagaagttactttcaactgctccctccgagaattcgcttctgaatatctttccatggagaatatcacgagtgtagttattgctgtgtttccagtctctgttttacttaaatgctttgtatctgtcaattagtaggggtacgcatggtcatttctcattaactctctcagatttagtgctctctttgtccgttcgcttgatgaagtaactatccatatgtggaaaaaggtactgcactaggtaccagatcgtgactgctctctacggagcctttgtcttcttggctgtttatttctctaagcttggacagaacccactagcgttttgtgacactgccaatatgataggaataaatgctgcctgttatgctctaaccagaaccaatgcattctattacttcaactgaaaatttcaatacgcctgttcctgacttggatgtaccttgttgaatttaaggtccgaactgtagaagagcaagtcagggcttcggcagaacataaattaggcgttgctaatcagagtataactgctggatttttcgacaacaacacaaggtcaattcttctactcggttaagattttagcttttctagctctcttttttcctttccttcatgctagatggtaacaattgcagtgctgaagatcggagggagtatcttgagtcacttctacgtgagtgtaaaaaggaagaatcagctccagtgttagatgatgatgctctgaataatattcttgcccgcaggtaagactgagtttgctgttagtattatttaagcattgttttaacaatctctgtcactcctggtactttatctaattacatgacatatcacatttctctccttgcagcgaagatgagatcgacatatttgaatctattgacaagcaaagactagatgatgaaatggtatactaaattcctttactttgtacatgtttatttctgctaatattttgtgcatcccaatttgattcttgtaccccttgtaggctgtatggctaaaggttgttcaggatggttcagttagtgggctagacccctcagtattgccaccccgccttgtgtctgatgatgatctgaagcccttctgtcatgctatgaagatttacgagtcttcaaatgtaaaaaatgtgaaggtaaatgtgaggaagaagggcgagcttggcggccttgatacaaagcattacggaaggggaaaacgtgctcgtgaggtcagttgcattatcatcttctgtatgtctctctattattggttgaagtatttgtttgctaatttcattatatatcctttgtaggtccggtcttatgaggatcaatggaccgaagaagaatttgaaaaactttgtcaggctgaatctcctgactcacctcaacctggtggtgtattgaaggatatagatatctctaaagagagtaagttggaggtacctgcagaaagttcaatagacccaaaagaaagttcaatagatccagtcgaagccaaaacggtgccagtcctggctgttccagactcctcaccaccagtcccgtctgttccagactcctcaccagcaaagcggcgaagaggtagacctagaaggtcagacgtttcagtatctcctgttatgtccccagcaaaagctgtccaacaagaggcaggaactacacttggcagttctgcaccagcaagtaccatcgattctgcagcaccaactgctaccatccattctactggtccagatgttaccacccattctgctgcaccagttgctgccatcaaaccagatattggtgcagaagttaaggctactgcttttgttgctgctgtaccaactgctaccatgaaacccgagattggtactgaagttacggaccatgttgttttggaagggtctatagcaaaggaagttggtccggcggtagagagcggtcatgacccagtagctgccagtgcagcccctcatccaccagctcctgctacatctagaggcagaaagacccaaacagttgaaacccctcgcagacgaggccgaaaaccaaaatctctttcctcatctagtgctggtgatgttaatataaaccctgtggttgcaattggtagtggacctgcttctgtgggttctccatatcctcaaggggatatgcctgcaagtctcatgtcaagatttcagaaggatttggttacaggtaggcctgttacgtcattgccagaggcagttaagggcatctccgcccctgaaggtacgacacctgttgccgaagataaacacactggaactgcaataagctcggacaatgccagcttactaatgccaaagatcattcacaacgaaaatgttggatttgttcaagtgagctctgagcaagttttttctgcatcagtacctactttaactgccgtctcaggtggaatattgaaagcatcacatattctcttggcagataagcctgccgagaagcaaagtgcttcacgccgtcgcagaaagaaagcgcctggtggtgaggatactggagtaagcactaggcaaagagcagctatgaagaaatctgatggtattcctggtaccactgacaatgttggtgcggacacgagcacagctgagaagctaggagcagtgaatgtaaaagatggcagttcacttcaagatactcccaaggaattaccaaatataaactctcctccatatgacaagtctgggtatgactctcaaccaagaacacctatagcagttcccattagtgaagctgcacttcctagtggttccggtaatgcccatgttgcttattctgatataactcctaggatacctaccaatcctgatgttcaagataaaccagtaaatctgcacataggagcacctctagcggcagccacacaacctgaagtgccatgtaagacagggaatgaccatgttgcagtgtgttctgtggtcactaccacacattctgaaacggttactgaaaaaccattgctaaatcctgttagtgaagtagcaaatgtccaggtcgaagcacctagttcttcacttcataattcaggtaagaacatcagtacagtgccttcagaggtcaatagtgtcgctcccagtaaggcatcaggtaggaggaggaaaggtcctgcctctgaaccacgcaccagaagtaaagccgcaacagctgcatgtgaacgtcgtgctcgactagctggaccaaagcagacaggtgatgcgagaaaattagaaatattggcaagcccaagcacggcggtttgtgtttcttcagttgagcaacaggaaaccgccctggcagagcctctcaccgcttctgtctgcgaaccgcagaagaatgctgagagtcatgtacgtggtggaatgtctactccgacggggatactagatgccccaaagcaaattgctacccagtcaattacagcatgtactgaagaaacaaataacagtctaagcacccagactcctgcacttcccatatccagagaaagtattctttccatgggtgacaagcaaggttctctctctctctctctctgctgttattattcattgtttggtagtaacaatggctcatgctgatgcccatgatgccttttttcaggtgttggagttgataccatacatggacaaacaaagatggttttggctgcagaactgacatctgcaaatgatgaacataagctgcatgaagtacatgataagactgctgatggtaatatactccaacacagtgcggcaaatgacacactccaggataaaactgatagcattgctggtttggacctagcctctcgtcatagaattggtgatttggaaatggagaagggtgattctaaaacagtgatgttaccagactgccaaaccccttttgatgcctcagttaaggatattaacgatactcttgcccccacagaagctgatgtcagtgatctgcaaagtgaggctgctgctattgatgtgactagtcctaagcaagatactatggtagttgaagcactttacactaatcctggaggttctgctagtcatctgcctgctgctttacaatcaacggactcaaaccagcatgcagaacggaaaggaagttcagataacagtggctctaaaatttttgcatctgggaagaaaacagaggaaatggaaggaactttggataagaatacggatcacaatcttattcaggcaaatgccaatatagctttaggaagatattctccttcagaggacaaaagagaggacagttgtgcccatgtagttgatggtgggctgttgggaagcaaacaaactcttcctgaagtcgtttctgctgtaaacactgatggctctgaggaagcactcaatgcttcgtctacccactcgaataaagatgccaccttggtttgtgaagtaacaaaggatcctgagagtcatgtatcagtgtctgtactggcctctgctgctatgaacgctggtgatgactctgaggaagttcacaatgttccatccacccattctgatagagggggcagcatggtagaagttgacgcgtctagagatgatgctacctctatttgcgaagtacgcaaggatcctgagagtaatgtatctggtgagttgtcgatgccagtacggttagcggagcttgagttagaactgccaaaccaatccaaatcttctagccagtctagcgcagtaaatgctgatgagacaaaggccagtatcaacattcagactacttcattggtagaatcaggagaacaaaaatcacccagaaatggtgcacatggtactccctatctctatcccctctttccccctctctctcccaccaaccatgatcctgtacacattccctggtgtatgctgattgttattcttatccagctagtgtatcttttttatgttttgccagagttgaaagaagggatggagttggctgggcctaagattgagtgcaccatacaaatgccgagtcccgatgataagagtatgctctgttattactttctgttgtagtagagacgggccagggggctcatgcacatctgcaccttttcaggttctgaggctcatagtttggcacaacgggagatggtttcgggtgcagaacaagcatctatgaaaggtatagtcaggttttaaatttctgaattaattaacgcatggtcaatagttactcatggatagtgtatctaacatatgtacagatgataaagaaaacaagatggttgatgttacattttcgtctggtggggaacaagaaacacagcgagctgatgtagacttgcccacatgtccaacatatgcagattgtgagggtgaaaaggacgattcccctaaaactattttggcaggcagccaatctttttgtgaagcctcagataaggacgttgccccagtgagagatgatcacactgatccgcaaagtgaagttattgttgttgatatgaatgatgccaaccaagactctgctgaagcggaagctatgcagattgatagtgtctccaaaggatcttcaagtgatttgcctgctgctttacgatcgaccgattcaaatcagctggcagaacaagtatctccttgtccgaaagaacatgagaaattggaagaaacttctggtgaaattggtggtggcaattccaatcgtagtcggactgatggtgattctcatattatgaatctagttggttattcggaagactcagatgaggacgattctatccaggtagctgatgttggtgatgtgggaagtaaagaaaccactcattatgacatctcagctgtcgctagaggagcagaaccaggagatggaccctgcacagagcctacttgtgaaactgctgttcatgtgcacgaatgcaatgcggacgttgctatttctgaggatggtcatggcacaacggcccttggcagcgtccaagtgtctacgacagaactaaaggatttggagagtggaagatgtctagaacatggaataggtacttctttatctgcttgctttattcatcaaagcccaccgaacaaagaacttagttatgctatttcagtaattcctgaccctgttgatcatgatggcacaggaacccctgtggctcttcaggagggaactgctgtcgctacagaaccagaagcaaagaaagaggtcgacgaacctactcaaaatgaagatgttgagctggctgccataaagccagaggcggtggagcatgctggtacagaggccgatccaagtaaagaagcatctatacctcctcaagaggaaaccactgctgtagccttggttacaggaccggaacaaaatgaagaagcagatgcacctactcaagtcgaaccagttgctatagtgccagattccatggagcatgctagtaccgaagttgatcaaagtatagaaacatctgtgcgtctcccagaaaaaacttctgttatacctggtacggaaccagaagagaagaaagtagaggcatcctcccaagaggataatgttgaagcagttgctgcagagccagaacctgctggatcccaggaaaatgcagaagtttctaccaagcctagtcctatggagatagagtcggttcaggaaacagctatgctgggagaagctgaaaccaggcagcaactgccacttccgtctgccgagggcgtggtagccgaggctagtgaacctccagaggtgactgctatgaaggaaccagagttgctgagcactgaaccagcacccgatggtgaaaatgctaagcttggagaagccaaagctgaacagctgttgcagcaaccttcatcctgcgaggctatggcagcagtcacaggagagcttcctagcgcagcgggagcgaaaacggatggaacttcagacgtggtggctgatgagtctcctgctgtcgtgggagaggaggtgctcaacactgaaactgcacctgatggtaaaaatccaaggccgagcgaggctgatacggcgcagtcgccacctttgcctgaagagggcaaggccgttgcagctaccgagcctgccaaccttgaggaggcggaggctactgatgggaagtagttagcgtgcaaaaatggaagcagatgttgcgttgaagaacctctgccgttagatcagacagagcatgtttgggctgatgaaactgagaagtaccttagactttatgcaagtgttgtatgtagaacataattaagaaacctgttgtattcagaggagttgttggtacataagttataactacctagtccctttgcaatgctagtagtaccttgttgca

SEQ ID NO: 7 - DNA, 10149 bp, Triticum aestivum
  source 1..10149: mol_type = other DNA
  CDS 1..10149: protein_id = 8; translation = MASSQHVEVEAAKLLQKLILESKDEPAKLATKLYVICQHMKLSGKEQSLPYQVISRAMETVVSQHGIDMDALRSSRVPFAGGPQAVDSSGLMSKDKEVIGGQSSMVGSDASQSSGQAALWHLPPGSADMARPGVYIPGRVPAGQNRGDVTGSDIHQGSMSQKSGRSSGVESPASLQMEDTRSMNSHDSLKSDEKTSKKASSSKRKRMDSKAAGDMQSEENSKSDGISSGQNIRKRKQVGKAGAQGQPSRGAEPEQSHILQGATAQVPPLPGGASFFRAHQEGPPASAGRTIDNTKPSNPFAMSQVSNFAEGLASGSIPTELQKSILGGTNMFNTGFGWNQSSQGSAIKNTQGSVANLMRPGVNVEGKINVGSQGAFNPTPTSQMDFPKIPPYMSSSFGGGSQFLDKGKDSASGNTGTELHSAAKVGVNMGIVHGSPIQERQNITRAPQRAESSLQEARLSSLPNRNVGPYQTSHISPNTPFKEQQLKQLRAQCLVFLAFRNNMQPRKVHLEIALGGGPTAEGGGAGQGGNESRVADGSVRENGNSQENSAIFGSQSDMSRLPSTSAGSIAEADSSLKDSEIKKKINIAEHEKSSMEIENIQQAVMQGTGSSSEMRSQEIASPVPSGPQQSYFQGDKRRNAPETYRTDAENLNRNLSFGGQGPSSLGGNRQHPNFEAGVLTKDRLQDEASKESYPPSRLHHMPIDGYNSNLPGKDLTPDTDRNEVEHCTQMGEMSDRSADEGDDDLFEHDDFASTPPKYTMTEKWIMDYQKRKYGENEKKVLEQQSAHKRMSASYQKLKESVSSSEDLTAKTKSVIELKKLQLLSLQRRVRSEFLSDFFKPNTADLERVKAVKKHRHGRRVKQLEKIEQKMKEERQKRIRERQKEFFADIESHRERLEDSFKAKRERLKGFNRYIKEFHKRKERIHREKLDRIQREKINLLKNNDVEGYLRMVQDAKSDRVKQLLRETEKYLQKLGAKLRGDSSMDGRSYVSGKGVTANDVEDESYQPQNYLESNEKYYQLAHSVKEIVNDQPTYLNGGKLREYQMNGLRWLVSLYNNNLNGILADEMGLGKTVQVISLLCYLMETKNDRGPFLVVVPSSVLSGWVSELNFWAPSINKIAYFGPPEERRRLFKEMIVQQKFNVLLTTYEYLMNKHDRPKLSKIQWHYIIIDEGHRIKNASCKLNADLKLYRSSHRLLLTGTPLQNNLEELWALLNFLLPNIFNSSEDFSQWFNKPFESNGDNSADEALLSEEENLLIINRLHQVLRPFVLRRLKHKVESELPGKIERLVRCEASAYQKLLMTRVEDNLGGIGAVKVRSVHNSVMELRNICNHPYLSQLHVEEIEGHLPRHYLPSIVRLCGKLEMLDRLLPKLKATGHRVLLFSTMTRLLDVMEDYLVWKKYQYLRLDGHTSGHERGALIDRFNDPDSPAFIFLLSIRAGGVGVNLQAADTVIIFDTDWNPQVDLQAQARAHRIGQKKEVLVLRLETVRTVEEQVRASAEHKLGVANQSITAGFFDNNTSAEDRREYLESLLRECKKEESAPVLDDDALNNILARSEDEIDIFESIDKQRLDDEMAVWLKVVQDGSVSGLDPSVLPPRLVSDDDLKPFCHAMKIYESSNVKNVKVNVRKKGELGGLDTKHYGRGKRAREVRSYEDQWTEEEFEKLCQAESPDSPQPGGALKDIDISKESKLEVPAESSIDPKESSIDPVEAKTVPVLAVPDSSPPVLSVPDSSPAKRRRGRPRRSDVSVSPVMSPAKAVQQEAGTTLGSSAPASTIDSAAPTATIHSTGPDVTTHSAAPVAAIKPVIGTEVKATAFVAAVPTATMKPEIGTEVTDHVVLEGSIAKEVGPAVESGHDPVAASAAPHPPAPATSRGRKTQAVETPRRRGRKPKTLSSSSAGDVNTNPVVAIGSGPASVGSPYPQGDMPSSHASLMSRFQKDLVTGRPVTSLPEGVKGISAPEGTTPVAEGKHTGTAISLDNASSLMPKIIHNEKVGFVQASSEQVFSASVPTLTAVSGGILKASHVLLADKPAEKQSASRRRRKKAPGGEDTGVSTRQRAAMKKSDGIPGTTDNVGADMSTAEKLGAVNVKDGSSLQDTPKELPNINSPPYDKSGYDSQPRTPIAVPISEAAAPSGSGNAHVAYSDITPRIPTNPDVQDKPVNLHTGAPLAAASQPVAVCSVVTTTHSETVTEKPLLNPVSELANVQVEPPSSSLHNSGENISTVPSEVNSVAPSKASGRRRKGPASEPRTRSKAATAACERRARLAGSKQTSDARKLEISASPSTVVCVSSVEQQETALAEPLTAYVCEPQKNAESHVRGGMSTPMGILDAPKQIATQSITACTEETNSSLSTQTPALPISRKSNLSMGDKQGVGVDTIHGQTNMVLAAELASANDEHKLHEVHDKTADGNILQHSAAHDTLQDKTDSIAGLNLASRHRISDLEMEKDDSNTVMLPDCQTPFDASVKDSKDTLAPTEADVSDLQNEAAAIDVTSPKQDTMVVEALHTNSGGSASHLPAALRSTGSNQHAEGKGSSKNSGSKFFASGKKTEEMEGTLDKNTDHNLIQANANIALGRHSPSDDKREDSCAHVVDGGLSGSKQTLPEVVSAVNTDGSEEALNASSTHSNKDATLVCEVTKDPESHVSVSVLASAAMNAGDDCAEVHNVPSTHSERGGSMVEVDASRDDATSICEVRKDPESNVSGELSMPVGLAELELELPNQSKSSSQSSAVKADETKASINIQTTSLVESGEQKSPRNGAHEEMELAGPKIECTIQMLSPDDKSSEAHSLAQREMVSGAEQASMKDDRENKMVDVIFLSGGEQETQRADVDLPTSPRYADCEGEKDHSPKTILAGSQSFCEASDKDVAPVKDDHTDPQSEVNVVDMNGTNQDSAETEAMQIDGVSKGSSSDLPAALRSTNSNQPAEQDGLENSPSISACPKENEKLEETSDEIGGGNSNRSRTDGDSHIMNLVGYSEDSDEDDSIQVADVGDVGCKETTHDDISAVARGAEPGDGPCTEPTCETAVHVPEAISEDGHGTTALGSVQVSTTEIKDLESGRCLEHGTGTPVVLQEGTAVATEPEAKKEVDEPTQNEDVEPAAIKPEAVEHAGTEADPSKEASIPPQEETAAVALVTGPEQNEEADAPTQVEPVAIVPDSMEHASTQVDQSIETAVRLPDETSVIPGTEPEEKKVEASPQEDNVGAVAAEPEPAGTQENAEVSTQPSPMEIELAQETAMLGEAETRQQLPLPSAEGVIAEASEPPSTEVTAMKEPELLSTEPAPDGENAKLGEAEAEQLSQQPSSCEAMAVTGELPSTAGAKTDGTSDVVASPAVVGEEVLNTETAPDGKNPRPSEADTAQSPPLPEEGKAVAATEPANLEEAEANDGK
atggcttcatcacagcatgttgaagtggaggctgcgaagctacttcaaaaactcattctggaatcaaaggatgagcccgctaaattagcaacaaaactttacgtgatatgtcaacatatgaagttaagtggaaaagagcagtctcttccctatcaggtcatatctagggccatggagactgttgtaagtcaacatggaattgatatggatgcattgcgatcatcacgagttccatttgccggcggtccacaagcagtagattctagtggccttatgtctaaggacaaggaggtcattggtggtcagtcttccatggttggaagtgatgcatcccagagcagcggtcaagctgcattatggcatttgccaccaggttcggcagatatggcaaggcctggggtgtatattccaggcagggttccagcaggacaaaataggggtgatgtcacaggatctgatattcatcaaggctccatgtcgcaaaagagtggccggtcctctggagtcgaaagccctgcaagtctgcaaatggaggacactagatctatgaattcacatgattctttgaagtccgatgaaaaaacaagcaagaaagcttcctcttccaagagaaaaaggatggactcaaaagcagcaggggatatgcaatctgaagaaaattcaaaatcagatggtatctcaagtggacaaaatattagaaaaaggaaacaggttggcaaagctggtgcacaaggtcagccctccaggggagctgagcctgagcaatcacatatactgcaaggtgctactgctcaggtgccacccttacctggtggtgcatcatttttcagggctcaccaggaaggtccaccagcttctgctgggaggactattgacaatactaaaccatcaaacccgttcgcaatgtcacaagtttcaaattttgctgaagggctggcttctggtagtatccccactgagttgcagaaaagtatactgggaggaacaaatatgtttaacactggttttggctggaatcaaagttcacaaggttcagctattaagaatactcaaggttctgttgccaacttaatgcggccaggagttaatgttgaagggaaaattaatgtagggtcacaaggagcttttaaccctactcccacatcgcagatggatttccccaaaatccctccttacatgtcttcttcctttggaggtggctcacagtttctggacaagggcaaggactcggcttctggcaataccggcactgaacttcattctgctgctaaagttggagttaacatggggattgtgcatggcagtccaattcaagaaaggcaaaatattaccagagcaccacagagggccgaatcatctttgcaagaagccagattgtcttcgctcccgaatagaaatgttgggccatatcaaacgtctcacatctctccaaacacacctttcaaagaacaacagttaaagcagctccgagcacagtgcttagtatttcttgcattcagaaataatatgcagcccagaaaggtgcaccttgaaattgccttaggtggaggccccactgcagagggtggcggcgcaggtcagggaggtaatgagagcagagtggctgatggttctgtaagggaaaacggaaacagtcaggaaaactctgctattttcggcagccaaagtgatatgtctagactcccgtccacatccgcaggcagcattgcagaggctgattcttcactgaaggactcggaaattaagaagaagatcaatatagctgaacatgagaagtcatcgatggaaatagaaaatatccagcaagctgttatgcagggaactggttcaagttctgaaatgcgctcccaagaaatagcatcccctgtgccatctggaccacagcagtcatactttcagggagataaaagaagaaatgcccctgagacctacaggacggatgcagaaaatttgaacaggaatttaagtttcggaggccagggaccatcttctttgggtggtaatagacaacatccaaattttgaagctggtgtcttgaccaaagatcgattacaggatgaagcatctaaagaatcatatccaccttcgaggcttcatcacatgcctatcgatggttacaactccaatttaccaggaaaggatctaactccagatacagatagaaatgaggttgaacattgtacccagatgggggagatgtctgatcgatcagctgatgaaggagatgacgatctatttgagcatgatgattttgcatcaactcctccaaaatacacaatgactgaaaaatggatcatggattatcaaaagagaaaatatggagaaaatgaaaagaaggtattagagcagcagagcgcacataaaaggatgtcagcatcctatcagaagttaaaggaaagtgttagttcatctgaagatcttactgcaaagacaaagagtgtcattgaattgaaaaagcttcaacttctctcacttcaacgtcgtgtgcgcagtgaattcttgtcagactttttcaagcctaatacagctgatttggagcgtgtaaaagcagtaaagaaacaccggcatggacgccgtgtgaaacagcttgaaaaaattgaacagaaaatgaaggaggaaaggcaaaaaagaatacgcgagaggcaaaaagagttctttgctgatatagagtctcacagagagagactggaggatagtttcaaggctaaaagagagcgtctaaagggtttcaatcgatatataaaagagttccacaagaggaaagagcgaattcatcgggagaagctggataggatccagcgggagaaaattaacttgcttaagaacaatgatgtcgaagggtatcttaggatggtccaggatgcaaaatctgaccgtgttaagcaactactacgggagactgagaaatatctacagaaacttggggccaaattacgaggtgacagctcaatggacggccgttcttatgtttctggtaagggcgtcactgcaaacgatgttgaagacgagagctaccagccgcagaattatcttgagagcaacgagaagtactatcagttggcccacagtgtgaaggagattgtaaatgaccagcctacttatcttaatggtgggaaattgcgggagtaccagatgaacggtttgcgttggctggtttcattgtacaataataatttgaatggaattttagctgacgagatggggcttggtaaaacagttcaagtaatctctttgttgtgctaccttatggaaacaaaaaatgaccggggcccatttcttgtggttgtaccatcctctgttctttctggatgggtatctgaactcaacttctgggcacctagtataaataaaattgcttattttggtcctccagaagaaaggcgcagactgttcaaagagatgattgttcaacagaagttcaatgtccttttgacaacatatgagtacttgatgaacaaacatgataggccaaaactaagcaaaatacagtggcactatataataatcgatgaagggcaccgtataaagaatgcgtcttgtaagctcaatgctgatctgaagctttatcggagttctcatcggctattgctgacaggaacacctttgcagaataatcttgaggagctgtgggcacttttgaactttctgttgcccaatatatttaactcatccgaagatttctctcagtggtttaacaaaccatttgaaagcaatggtgataactcagctgatgaggccttactttcagaggaggaaaacttgctgatcataaaccgtcttcaccaagttcttcggccctttgtactccgaagacttaagcataaggttgaaagtgaattgccagggaagattgaaagacttgtaagatgcgaggcatcagcttatcagaaacttctgatgacaagggtggaagacaaccttggtggaattggagcagttaaggtccgctcggtgcacaattctgtcatggaattgaggaacatatgcaaccatccataccttagccagcttcatgttgaggagattgagggtcatctacctaggcactacctgccatctattgtgaggctgtgtgggaaacttgagatgttggacagattgctacccaaactcaaagctactggccatagggttctacttttttctacaatgacaagattgcttgatgtgatggaggattatctggtatggaaaaagtatcagtaccttcggttagatggacacacttctgggcatgagagaggagcacttattgatagatttaatgatcctgattctccagctttcatttttctgctaagtatccgagcaggaggcgttggtgtcaatcttcaagcagctgatactgtcatcatatttgatactgattggaatcctcaggttgacttgcaagcacaggctagagcccacagaattggtcaaaagaaggaggttcttgttttacgtttagaaactgtccgaactgtagaagagcaagtcagggcttcggcagaacataaattaggcgttgctaatcagagtataactgctggattttttgacaacaacacaagtgctgaagatcggagggagtatcttgagtcacttctacgtgagtgtaaaaaggaagaatcagctccagtgttagatgatgatgctctgaataatattcttgcccgcagcgaagatgagatcgacatatttgaatctattgacaagcaaagactagatgatgaaatggctgtatggctaaaggttgttcaggatggttcagttagtgggctagacccctcagtattgccaccccgccttgtgtctgatgatgatctgaagcccttctgtcatgctatgaagatttacgagtcttcaaatgtaaaaaatgtgaaggtaaatgtgaggaagaagggcgagcttggtggccttgatacaaagcattacggaaggggaaaacgtgctcgtgaggtccggtcttatgaggatcaatggaccgaagaagaatttgaaaaactttgtcaggctgaatctcctgactcacctcaacctggtggtgcattgaaggatatagatatctctaaagagagtaagttggaggtacctgcagaaagttcaatagacccaaaagaaagttcaatagatccagttgaagccaaaacggtaccagtcctggctgttccagactcctcaccaccagtcctgtctgttccagactcctcaccagctaagcggcgaagaggtagacctagaaggtcagacgtttcagtatctcctgttatgtccccagcaaaagctgtccaacaagaggcaggaactacacttggcagttctgcaccagcaagtaccatcgattctgcagcaccaactgctaccatccattctactggtccagatgttaccacccattctgctgcaccagttgctgccatcaaaccagttattggtacagaagttaaggctactgcttttgttgctgctgtaccaactgctaccatgaaacccgagattggtactgaagttacggaccatgttgttttggaagggtctatagcaaaggaagttggtccggcggtagagagcggtcatgacccagtagctgccagtgcagcccctcatccaccagctcctgctacgtctagaggcagaaagacccaagcagttgaaacccctcgcagacgaggccgtaaaccaaaaactctttcctcatctagtgctggtgatgttaatacaaaccctgtggttgcaattggtagtggacctgcttctgtgggttctccataccctcaaggggatatgccctcatcacatgcaagtctcatgtcaagatttcagaaggatttggttacaggtaggcctgttacgtcattgccagagggagttaagggcatctccgcccctgaaggtacgacacctgttgccgaaggtaaacacactggaactgcaataagcttggacaatgccagctcactaatgccaaagatcattcacaacgaaaaagttggatttgttcaagcgagctctgagcaagttttttctgcatcagtacctactttaactgccgtctcaggtggaatattgaaagcatcacatgttctcttggcagataagcctgcagagaagcaaagtgcttcacgccgtcgcagaaagaaagcgcctggtggtgaggatactggagtaagtactaggcaaagagcagctatgaagaaatctgatggtattcctggtaccactgacaatgttggcgcggacatgagcacagctgagaagctaggagcagtgaatgtaaaagatggcagttcacttcaagatactcccaaggaattaccaaatataaactctcctccatatgacaagtctgggtatgactctcaaccaagaacaccaatagcagttcccattagtgaagctgcagctcctagtggttccggtaatgcccatgttgcttattctgatataactcctaggatacctaccaatcctgatgttcaagataaaccagtaaatctgcacacaggagcacctctagccgcagcctcacaacctgttgcagtgtgttctgtggtcactaccacacattctgaaacggttactgaaaaaccattgctaaatcctgttagtgaactagcaaatgtccaggtcgaaccacctagttcttcacttcataattcaggtgagaacatcagtacagtgccttcagaggtcaatagtgtcgctcccagtaaggcatcaggtaggaggaggaaaggtcctgcctctgaaccacgcaccagaagtaaagccgcaacagctgcatgtgaacgtcgtgctcgattagctggatcaaagcagacaagtgatgcgagaaaattagaaatatcggcaagcccaagcacggtggtttgtgtttcttcagttgagcaacaggaaaccgccctggcagagcctctcactgcttatgtctgcgaaccgcagaagaatgctgagagtcatgtacgtggtggaatgtctactccgatggggatactagatgccccaaagcaaattgctacccagtcaattacagcatgtactgaagaaacaaatagcagtttaagcactcagactcctgcacttcccatatccagaaaaagtaatctttccatgggtgacaagcaaggtgttggagttgataccatacatggacaaacaaatatggttttggctgcagaactggcatctgcaaatgatgaacataagctgcatgaagtacatgataagactgctgatggtaatatactccaacacagtgcggcgcatgacacactccaggataaaactgatagcattgctggtttgaacctagcttctcgtcatagaattagtgatttggaaatggaaaaggatgattctaatacagtgatgttaccagactgccaaaccccttttgatgcctcagttaaggatagtaaggatactcttgcccccacagaagctgatgtcagtgatctgcaaaatgaggctgctgctattgatgtgactagtcctaagcaagatactatggtagttgaagcactgcacactaattctggaggttctgctagtcatctgcctgctgctttacgatcaacgggctcaaaccagcatgcagaagggaaaggaagttcaaagaacagtggctctaaattttttgcatctgggaagaaaacagaggaaatggaaggaactttggataagaatacggatcacaatcttattcaggcaaatgccaatatagctttaggaagacattctccttcagatgacaaaagagaggacagttgtgcccatgtagttgatggtggcctgtcgggaagcaaacaaactcttcctgaagtcgtttctgcagtaaacactgatggctctgaggaagcactcaatgcttcatctacccattcgaataaagatgccaccttggtttgtgaagtaacaaaggatcctgagagccatgtatcagtgtctgtactggcctctgctgctatgaacgctggtgatgactgtgcggaagttcacaatgttccatccacccattctgaaagagggggcagcatggtagaagttgatgcgtctagagatgatgctacctctatttgtgaagtacgcaaggatcctgagagtaatgtatctggtgagttgtcgatgccagtagggttagcggagctcgagttagaactgccaaaccaatccaaatcttctagccagtctagcgcagtaaaggctgatgaaacaaaggccagtatcaacattcagactacttcattggtagaatcaggagaacaaaaatcacccagaaatggtgcacatgaagagatggagttggctgggcctaagattgagtgcacaatacaaatgctgagtcctgatgataagagttctgaggctcatagtttggcacaacgcgagatggtttcgggtgcagaacaagcatctatgaaagatgatagagaaaacaagatggttgatgttatatttttgtctggtggggaacaagaaacacagcgagctgatgtagacttgcccactagtccaagatatgcagattgtgagggtgaaaaggaccattcccctaaaactattttggcaggcagccaatctttttgtgaagcctcagataaggacgttgccccagtgaaagatgatcacactgatccgcaaagtgaagttaatgttgttgatatgaatggtaccaaccaagactcagctgaaaccgaagctatgcagattgatggtgtctccaaaggatcttcaagtgatttgcctgctgctttacgatcgaccaattcaaatcagccggcagaacaagatggattagagaatagtccctctatatctgcttgtccgaaagaaaatgagaaattggaagaaacttctgatgaaattggtggtggcaattccaatcgtagtcggactgatggtgattctcatattatgaatctagttggttattcggaagactcagatgaggacgattctatccaggtagctgatgttggtgatgtgggatgtaaagaaactactcatgatgacatctcagctgtcgctagaggagcagaaccaggagatggaccctgcacagagcctacttgtgaaactgctgttcatgtgcctgaagctatttctgaggatggtcatggcacaacggcccttggcagtgtccaagtgtctacgacggaaataaaggatttggagagtggaagatgtctagaacatggaacaggaacccctgtggttcttcaggagggaactgctgtcgctacagaaccagaagcaaagaaagaggtcgacgaacctactcaaaatgaagatgttgagccggctgccataaagccagaggcagtggagcatgctggtacagaagctgatccaagtaaagaagcatctatacctccacaagaggaaaccgctgctgtagccttggttacaggaccggaacaaaatgaagaagcagatgcacctactcaagtcgaacccgttgccatagtgccagattccatggagcatgctagtacccaagttgatcaaagtatagaaacagctgtgcgtctcccagacgaaacttctgttatacctggtacggaaccagaagagaagaaagtagaggcatccccccaagaggataatgttggagcagttgccgcagagccagaacctgctggaacccaggaaaatgcagaagtttctactcagcctagtcctatggagatagagttggctcaggaaacagctatgctgggagaagctgaaaccaggcagcaactgccacttccgtctgccgagggcgtgatagccgaggctagtgaacctccaagcacagaggtgactgctatgaaggaaccagagttgctgagcactgaaccagcacccgatggtgaaaacgcgaagcttggagaagccgaagctgaacagctgtcgcagcaaccttcatcctgcgaggctatggcagtcacaggagagcttcctagcacagcgggagcgaaaacggatggaacttcagacgtggtggcgtctcctgctgtcgtgggagaggaggtgctcaacactgaaactgcacctgatggtaaaaatccaaggccgagcgaggctgatacggcgcagtccccacctttgccggaggagggcaaggccgtggcagctactgagcctgccaaccttgaggaggcggaggctaatgatggaaagtag

SEQ ID NO: 8 - protein, 3382 aa, Triticum aestivum
MASSQHVEVEAAKLLQKLILESKDEPAKLATKLYVICQHMKLSGKEQSLPYQVISRAMETVVSQHGIDMDALRSSRVPFAGGPQAVDSSGLMSKDKEVIGGQSSMVGSDASQSSGQAALWHLPPGSADMARPGVYIPGRVPAGQNRGDVTGSDIHQGSMSQKSGRSSGVESPASLQMEDTRSMNSHDSLKSDEKTSKKASSSKRKRMDSKAAGDMQSEENSKSDGISSGQNIRKRKQVGKAGAQGQPSRGAEPEQSHILQGATAQVPPLPGGASFFRAHQEGPPASAGRTIDNTKPSNPFAMSQVSNFAEGLASGSIPTELQKSILGGTNMFNTGFGWNQSSQGSAIKNTQGSVANLMRPGVNVEGKINVGSQGAFNPTPTSQMDFPKIPPYMSSSFGGGSQFLDKGKDSASGNTGTELHSAAKVGVNMGIVHGSPIQERQNITRAPQRAESSLQEARLSSLPNRNVGPYQTSHISPNTPFKEQQLKQLRAQCLVFLAFRNNMQPRKVHLEIALGGGPTAEGGGAGQGGNESRVADGSVRENGNSQENSAIFGSQSDMSRLPSTSAGSIAEADSSLKDSEIKKKINIAEHEKSSMEIENIQQAVMQGTGSSSEMRSQEIASPVPSGPQQSYFQGDKRRNAPETYRTDAENLNRNLSFGGQGPSSLGGNRQHPNFEAGVLTKDRLQDEASKESYPPSRLHHMPIDGYNSNLPGKDLTPDTDRNEVEHCTQMGEMSDRSADEGDDDLFEHDDFASTPPKYTMTEKWIMDYQKRKYGENEKKVLEQQSAHKRMSASYQKLKESVSSSEDLTAKTKSVIELKKLQLLSLQRRVRSEFLSDFFKPNTADLERVKAVKKHRHGRRVKQLEKIEQKMKEERQKRIRERQKEFFADIESHRERLEDSFKAKRERLKGFNRYIKEFHKRKERIHREKLDRIQREKINLLKNNDVEGYLRMVQDAKSDRVKQLLRETEKYLQKLGAKLRGDSSMDGRSYVSGKGVTANDVEDESYQPQNYLESNEKYYQLAHSVKEIVNDQPTYLNGGKLREYQMNGLRWLVSLYNNNLNGILADEMGLGKTVQVISLLCYLMETKNDRGPFLVVVPSSVLSGWVSELNFWAPSINKIAYFGPPEERRRLFKEMIVQQKFNVLLTTYEYLMNKHDRPKLSKIQWHYIIIDEGHRIKNASCKLNADLKLYRSSHRLLLTGTPLQNNLEELWALLNFLLPNIFNSSEDFSQWFNKPFESNGDNSADEALLSEEENLLIINRLHQVLRPFVLRRLKHKVESELPGKIERLVRCEASAYQKLLMTRVEDNLGGIGAVKVRSVHNSVMELRNICNHPYLSQLHVEEIEGHLPRHYLPSIVRLCGKLEMLDRLLPKLKATGHRVLLFSTMTRLLDVMEDYLVWKKYQYLRLDGHTSGHERGALIDRFNDPDSPAFIFLLSIRAGGVGVNLQAADTVIIFDTDWNPQVDLQAQARAHRIGQKKEVLVLRLETVRTVEEQVRASAEHKLGVANQSITAGFFDNNTSAEDRREYLESLLRECKKEESAPVLDDDALNNILARSEDEIDIFESIDKQRLDDEMAVWLKVVQDGSVSGLDPSVLPPRLVSDDDLKPFCHAMKIYESSNVKNVKVNVRKKGELGGLDTKHYGRGKRAREVRSYEDQWTEEEFEKLCQAESPDSPQPGGALKDIDISKESKLEVPAESSIDPKESSIDPVEAKTVPVLAVPDSSPPVLSVPDSSPAKRRRGRPRRSDVSVSPVMSPAKAVQQEAGTTLGSSAPASTIDSAAPTATIHSTGPDVTTHSAAPVAAIKPVIGTEVKATAFVAAVPTATMKPEIGTEVTDHVVLEGSIAKEVGPAVESGHDPVAASAAPHPPAPATSRGRKTQAVETPRRRGRKPKTLSSSSAGDVNTNPVVAIGSGPASVGSPYPQGDMPSSHASLMSRFQKDLVTGRPVTSLPEGVKGISAPEGTTPVAEGKHTGTAISLDNASSLMPKIIHNEKVGFVQASSEQVFSASVPTLTAVSGGILKASHVLLADKPAEKQSASRRRRKKAPGGEDTGVSTRQRAAMKKSDGIPGTTDNVGADMSTAEKLGAVNVKDGSSLQDTPKELPNINSPPYDKSGYDSQPRTPIAVPISEAAAPSGSGNAHVAYSDITPRIPTNPDVQDKPVNLHTGAPLAAASQPVAVCSVVTTTHSETVTEKPLLNPVSELANVQVEPPSSSLHNSGENISTVPSEVNSVAPSKASGRRRKGPASEPRTRSKAATAACERRARLAGSKQTSDARKLEISASPSTVVCVSSVEQQETALAEPLTAYVCEPQKNAESHVRGGMSTPMGILDAPKQIATQSITACTEETNSSLSTQTPALPISRKSNLSMGDKQGVGVDTIHGQTNMVLAAELASANDEHKLHEVHDKTADGNILQHSAAHDTLQDKTDSIAGLNLASRHRISDLEMEKDDSNTVMLPDCQTPFDASVKDSKDTLAPTEADVSDLQNEAAAIDVTSPKQDTMVVEALHTNSGGSASHLPAALRSTGSNQHAEGKGSSKNSGSKFFASGKKTEEMEGTLDKNTDHNLIQANANIALGRHSPSDDKREDSCAHVVDGGLSGSKQTLPEVVSAVNTDGSEEALNASSTHSNKDATLVCEVTKDPESHVSVSVLASAAMNAGDDCAEVHNVPSTHSERGGSMVEVDASRDDATSICEVRKDPESNVSGELSMPVGLAELELELPNQSKSSSQSSAVKADETKASINIQTTSLVESGEQKSPRNGAHEEMELAGPKIECTIQMLSPDDKSSEAHSLAQREMVSGAEQASMKDDRENKMVDVIFLSGGEQETQRADVDLPTSPRYADCEGEKDHSPKTILAGSQSFCEASDKDVAPVKDDHTDPQSEVNVVDMNGTNQDSAETEAMQIDGVSKGSSSDLPAALRSTNSNQPAEQDGLENSPSISACPKENEKLEETSDEIGGGNSNRSRTDGDSHIMNLVGYSEDSDEDDSIQVADVGDVGCKETTHDDISAVARGAEPGDGPCTEPTCETAVHVPEAISEDGHGTTALGSVQVSTTEIKDLESGRCLEHGTGTPVVLQEGTAVATEPEAKKEVDEPTQNEDVEPAAIKPEAVEHAGTEADPSKEASIPPQEETAAVALVTGPEQNEEADAPTQVEPVAIVPDSMEHASTQVDQSIETAVRLPDETSVIPGTEPEEKKVEASPQEDNVGAVAAEPEPAGTQENAEVSTQPSPMEIELAQETAMLGEAETRQQLPLPSAEGVIAEASEPPSTEVTAMKEPELLSTEPAPDGENAKLGEAEAEQLSQQPSSCEAMAVTGELPSTAGAKTDGTSDVVASPAVVGEEVLNTETAPDGKNPRPSEADTAQSPPLPEEGKAVAATEPANLEEAEANDGK

SEQ ID NO: 9 - DNA, 24652 bp, Triticum aestivum
  source 1..24652: mol_type = genomic DNA
  exon 1..259
  exon 3842..3955
  exon 4034..4095
  exon 6484..6689
  exon 6763..7485
  exon 7574..7776
  exon 8191..8390
  exon 8471..8535
  exon 8615..9444
  exon 9586..9683
  exon 9792..9977
  exon 10471..10651
  exon 10800..10964
  exon 11043..11086
  exon 11323..11379
  exon 11521..11617
  exon 11725..11897
  exon 11974..12187
  exon 12355..12480
  exon 12564..12653
  exon 15326..15442
  exon 15541..15621
  exon 15708..15815
  exon 15964..16133
  exon 16270..16348
  exon 16431..16505
  exon 17884..17981
  exon 18065..18172
  exon 18280..18337
  exon 18421..18642
  exon 18727..20893
  exon 20984..22147
  exon 22274..22339
  exon 22412..22477
  exon 22560..23339
  exon 23442..24652
agacagcggccagagaagaggaactgaaaagaaaaaacggggaagaaaaaggaggcaagcagtgcacaggtctagtggaaaatggcggaggcggcgtgctcgacctcgggcacgtagctcacgcgcagctcatcgttccccgtcgcgttctccagagaccccgcgccgccgccggcgaccaccagctcccccgtgcggcggctccgcgtctccacccgtctcgttctcccgctagggtttcccccgatccccaatcactgtaagccgcggagacttgtctcgctagtttccttctggttcaagctcacgggagcgtgcgtgtggtccccgagtgggtggatttgggggtcgcggtctcggatcttgagcgatcagtgtagctctgttctcagctagggttagttcgtagaagcataagttgggaactgggattcgtggagccttatgtgatttgggtcagcgagctgcttctgtagcgagaacttataagctctgagcgcgccatgtggagtaattggcctattctgtgcaataatctcatctttaaacatttcgtctttttcccggttccgatagggattttttgggtgtgacttgggtttattccttgtgtgcattgcctagttatgacctgattggttagcttttggttgcacttaattggtctgtgaattgtgttataggttgggatgtcttgttagtgaagcttgatcagtatcacgcatctgattgcttttctcaaagagtggcactatttttgtagaccaaatgagtggcgctatttcgttgttattcacagaatttgtagcatgtggagtggtcccacgctatcatgaagcaagaaataccattttttaactttagctcagcatatagtgatatctctgctactttcttcagagcagcttgaatgcatgccattgtgatgcctgctattaatttatatagcattacatgtatagcaacttttttggaagttctgttattggtagctatgtaactatagagtatgcctgtttgcaatttactaaacctgctgctctgcattaacagtttgcgtctacaaagattagctctgaaattcatgctgctgtatctgtactctctttcgaattggatccataatatttttcattccaaattttgaagacaaaatctctaaaaccctctgtaagcatccattatttctcagactaaaaataggaggggcatggcagcgatccccataatctgaaaacaaaggagtatgatcagaaacctccctagcaaaggcttgcaacatagacaaaggacaatgttcctcccatttagggcagaagaatactctatctagttttccaaaggtagcatcctccaaattatttacccacatgaaatttctcccaatttaaggcttctctctcaactcgtcgtgttaaaaatgatgtattaaacacaaaactctagtgatcagtatcattggatttgtttttttcacagctctttccaattatgttaaaatccccacctactaaacatggtagaggattatcatgatatattctagccaactcatctaggaagttagcttttccttccaagtgcgcattaccataaacagtaatgagatccgaattaaatttggcaatcttatcaaaaagtaatattctaataaagtactctcccctctccacttggataatatcgaacacatttttactaatacccactaaaatcccactggacctccacctaggatgatttcaatgccactattttttttctaccactcaaagagtgtagttcattgttagaaaaaaatgttttgtggtttccaaaagaccaaaaaatccaatctatgatcaattatcatttccctaacatatctcttttggagatcttgtcccaaacctctaacaattcaatccaaaagacatctcacgttacaacttggatggacctcaggcatgagtccgggagaaggtttcgaggagtcgcatcacaagcctgcgaccatccaccccatcccaccaagccttcctaacgcaagactccgtgctttgtcaagacgacgaaacctattattaaaatattgttgtatttgtttttgtccatgtacgtatgcacccaagctaactatacttaaaaccgagttatgaagaatacctctagttggaagttgttttcataacaacaagcctacaattacaccttgttatatttcgttgagatggtcctagatttatgaaaaggaatttgatcctgaatttttcgtttccacgtcaaaagtgtatgtgtcaccttgaattggaatcgtgattccacaccgattccaacatttgcttttcgagaacaagactccgacccagtttttctttcgttcgattctcctagaatcttgagaatcgggaaaagaacttggcctccgattgtttagggataacacaccatggccctggccctggccccaacgaagctgaaagcccagcccactgggtacccacggccctcggccctcacccatttccactagctaaatactggtaaacccccctcccttctcccccaccccaccacacacacaagacagcggccagagaagaggaactgaaaagaaaataaaggggaagaaaaaggaggcaagcagtgcacagatctagtggaaaatggcggaggcggcgtgctcgacctcgggcacgtagctcacgtgcagctcatcgttccccgtcgcgctctccagagaccccgcgccgccgccggtgaccaccagcttccccgtgcggcggctccgcgtctccacccgtctcgttctccatctagggtttcccccgatccccaatcactgtaagctgcgaagacttgtctcgctagtttccttctggttcaagctcacaggagcatgcgcgtggtccccgagtgggtggattttggggttggggtctcggatcttgcgcgatcagtgtagctctgttcccagctagggttaattcatagaagcataagttgggaactggaattcgtggagccttatgtgatttgggtcagcgagctgcttctgtagcgagaacttataagctctgagcgcgccatgtggagtaattggcctattctgtgcaataatctcatctttaaacatttcttctttttcccggttccgatggggattttttgggtgtgacttgggtttattccttgtgcattgcctagtcatgacctgattggttagcttttggttgcacttaattggtctgtgaattgtgttatagggtgggatgtcttgttagtgaagcttgattagtatcacacatctgattgcttttctcaaagagtggcactatttttttagaccaaatgagtggcgctatttcgttgttattcacataatttgtaggatgtggagcggtcccatgctatcatgaagcaagaaataccattttttaactttagctcagcatatagtgatatctctgctactttctccagagcagcttgaatgcatgccattgtgatccctgctattaatttacatagcatacatgtggtgaacatgcaaattctatagcaacttttttggaagttctgttattggtagctatgtaactgtagagtatgcctgtttgcaatttactaaacctgctgctctgcattaacagtttgcgtctacaaaaattagctctgaaattcatgctgctgtatctgtactcaatgtactgtatttgattatcgaaatctataacgtttgttttcctacattaactactggcgtactggtttgcctcttataacttataatttataaatgttagttggattacggtttatttatcttctttttgattgatcttattttgatggcaagcagagtttgcgaatggcttcatcacagcatgttgaagtggaggctgcgaagctacttcaaaaactcattctggaatcaaaggatgagcccgctaaattagcaacaaaactttacgtggtatgcagcgcaaccgatatacaggacatgaaaagccttaactcaaccataaccttgtttctttgttcaatgttctagatatgtcaacatatgaagttaagtggaaaagagcagtctcttccctatcaggtcatatctaggtaaatatttcttttgttcttggctatcttttcagaagttttttttgccatcaattttactttaaatattagtcaaatattctgttagaaaaacaccactccctccgatccatattaattgatgctggtttagttgtattaactttgtactaaaccagtgtcaactaatttggattggggggagtagttaaagttctaccttgtgtcttacacatgctatcttgttattcttgactttcagatttgataattgttgatgtgttgttcttatgttcgaaagttctgcttatttaattataattatgccatcatcaaactagatttcacacatcagttagtacttattgtcaattgtggaatagtatacaaggagggggcctaaccatctaaatgctgttgcagcgaggttgtagcttggtactctccctaggtactaaatgttgctccaactagtttaggtgaagaaaataggaataagcagaaagaccagaggcccctggacacaggctcaatgagggagacaggaggatattgaagctcagtgatggacactttcctcatctatgtagtgaactgttaatacacacttacacagtagtatgatatccacaaccccaaaatgcatgggcaaattggagttcaacatcctccctctgagcagcctttctcatggagatggagattgaggagggagagaagtcgttggaggatggcaagagggagtggcagagaagtgcaagtagaagtaagatgggagtagcgagctgtcatttggaggcttaccactgataatatttttcttttggttgacatgttagcctgtagtaatagatctcgattcttgaaatcctctatccttgatggaagtagcgagcttttaaagactatttgattgtgtttggctgggctgtggattttctgaaagcagatgcaagagatgtgccatgggaaagctgctgtggactgtgtgttgtgagaaagctgtgaagccatttggcaaactagctgtctgaaatgcggctgcgggaataaatgtctgaaatacccttaaaagccgagacattggatacatactgtttaatggtaaaaacatcattacaggttgacctagttcgtaaatatagctattcaaccagttacctagttaattatttcatggagtttttgttttattgcatattaacgaaaatgcatatagctctacatatcacaaaatagatgcactagtgccatacaaaatttacatatcaacagacacattaatctggttccagtggggcataggctactactgccatacaacataaacatatcaccaaaaaatgcaatggtcgtacatctccagtggggcaaatctggagaaaggaacgacatgtacatgggcgagggaagcggcagtagcacacctcgaatgggggatgtagcagaggaggtcaggcacccatggtcggcggcggccttgctcgtctgagtaaccttgggcactggtggaggtagatgagggggtgggggtggagcggggaagaggaggccaattgaccgaggtggatgaaggaatggaagcatccaccggcggtcttgcggcggcgtgccgtcagcgacatgggagcgagctggtgaccagcagctggccggcggtgctaatgaaccctagaatcgccagaggtgggggacgagaaaagggccttgctcgatgggcttggtagagttgtctctggtggacgtaccggctggattattttggcggcaaaggtgagtaatttgatctcaagtggatgtaggttcgggcagccatgcagccaaagccagaaaagcacctcttcggccgctttcacccgtacatgtgttttgcgatggctttcaagggaaccgcgttcgctcattttgccgtttggttgtgatttcagctgtgaaggagagaaatccacagcgaaagccaaaccgaacgcagcctttgccttggacaatttaagagtgtagaaccttgagcgcaccttttgtctggaatcaatcatcagtgttgtcaactgaagctgtcgttttccataaatttggggttgtttatgcaccaaaagaattaagtatcttttgtttgttagagcttatactccattatgatattgagtgcgctatggtttatactctatagtaggtggtgccagatgatttaccagatgtactgtttgcaatgtgtagtataagtatagtaatacaaataatccagtttggttaggtctacttcacctgattgtttgtaatttcaaatgaaaggattctgcgtatgtcagaaagttctatttttgtctacttccaatttttctctagcttgacttctctcctctttctagtttctaagatgcccgtaacatccgcaatttttgtctgcagggccatggagactgttgtaagtcaacatggaattgatatggatgcattgcgatcatcacgagttccatttgccggcggtccacaagcagtagattctagtggccttatgtctaaggacaaggaggtcattggtggtcagtcttccatggttggaagtgatgcatcccagagcagcggtcaagctgcattatggcatttgccaccaggtaaccaaccaacttgaaaaggaaactgcagccactgttttggagatgtgatatgatttttttatattattaggttcggcagatatggcaaggcctggggtgtatattccaggcagggttccagcaggacaaaataggggtgatgtcacaggatctgatattcatcaaggctccatgtcgcaaaagagtggccggtcctctggagtcgaaagccctgcaagtctgcaaatggaggacactagatctatgaattcacatgattctttgaagtccgatgaaaaaacaagcaagaaagcttcctcttccaagagaaaaaggatggactcaaaagcagcaggggatatgcaatctgaagaaaattcaaaatcagatggtatctcaagtggacaaaatattagaaaaaggaaacaggttggcaaagctggtgcacaaggtcagccctccaggggagctgagcctgagcaatcacatatactgcaaggtgctactgctcaggtgccacccttacctggtggtgcatcatttttcagggctcaccaggaaggtccaccagcttctgctgggaggactattgacaatactaaaccatcaaacccgttcgcaatgtcacaagtttcaaattttgctgaagggctggcttctggtagtatccccactgagttgcagaaaagtatactgggaggaacaaatatgtttaacactggttttggctggaatcaaagttcacaaggttcagctattaagaatactcaaggttctgttgccaacttaatgcggccaggagttaatgttgaaggtacttccattaaaaaataatgacataacagcatatttaaagacttgaattacaaatatttaccttaatgagcttgcttacactgcagggaaaattaatgtagggtcacaaggagcttttaaccctactcccacatcgcagatggatttccccaaaatccctccttacatgtcttcttcctttggaggtggctcacagtttctggacaagggcaaggactcggcttctggcaataccggcactgaacttcattctgctgctaaagttggagttaacatggggattgtgcatgtaaggcctgtagtttaatccttaaacggggtgttaacatgctatttcggctacagtttggcccttctgaaaaaccttttaattgaaaagctaatattttttgctgtgttcgccaatggtaacttgttacgggaatgcctagtagtaatggtataatgcagggtattcatttgcataagattgtaatcgagcttcgaacacaagtgtattattgcatgccagtttcgtgtatgtctatttgcgtgccttgatagactttctgccaggttttaggttgatcaaccgataaataagctgtttctgcctgcaagattaagaattttgttgtctggtcatttaatgatatgttaattgatttttgtatctcaagtagaggtgctttatttgatgcatccatgtaatacgactttgcagggcagtccaattcaagaaaggcaaaatattaccagagcaccacagagggccgaatcatctttgcaagaagccagattgtcttcgctcccgaatagaaatgttgggccatatcaaacgtctcacatctctccaaacacacctttcaaagaacaacagttaaagcagctccgagcacagtgcttagtatttcttgcattcaggtacatgcttagagcactgtaggatgattggtatccgaagttcatctctgttgtactaatttagctactctttcttgtagaaataatatgcagcccagaaaggtgcaccttgaaattgccttaggtggaggccccactgcagagggtaagaactaagaacagaaaacattgtgtgagttgacagggtttctgtactcatgatgagcttataattttataaacaggtggcggcgcaggtcagggaggtaatgagagcagagtggctgatggttctgtaagggaaaacggaaacagtcaggaaaactctgctattttcggcagccaaagtgatatgtctagactcccgtccacatccgcaggcagcattgcagaggctgattcttcactgaaggactcggaaattaagaagaagatcaatatagctgaacatgagaagtcatcgatggaaatagaaaatatccagcaagctgttatgcagggaactggttcaagttctgaaatgcgctcccaagaaatagcatcccctgtgccatctggaccacagcagtcatactttcagggagataaaagaagaaatgcccctgagacctacaggacggatgcagaaaatttgaacaggaatttaagtttcggaggccagggaccatcttctttgggtggtaatagacaacatccaaattttgaagctggtgtcttgaccaaagatcgattacaggatgaagcatctaaagaatcatatccaccttcgaggcttcatcacatgcctatcgatggttacaactccaatttaccaggaaaggatctaactccagatacagatagaaatgaggttgaacattgtacccagatgggggagatgtctgatcgatcagctgatgaaggagatgacgatctatttgagcatgatgattttgcatcaactcctccaaaatacacaatgactgaaaaatggatcatggattatcaaaagagaaaatatggagaaaatgaaaagaaggtattagagcagcagagcgcacataaaaggatgtcagcatcctatcagaagttaaaggtctctctctgcgagttcctgtttcatatgtgtacatatttatgagtttttgcgagttcctgtttcatatgttcagtttttcctcactgtagcagctgtaattgttggttgcaaaattttaagttcttgttcatcctacaggaaagtgttagttcatctgaagatcttactgcaaagacaaagagtgtcattgaattgaaaaagcttcaacttctctcacttcaacgtcgtgtgcgcaggtttgcttgccattggagatcatcagtcttcagtttctctccttgtgcttaccacatgtttctatggctgtaacttccctattctaatttcttgcttatatttggcagtgaattcttgtcagactttttcaagcctaatacagctgatttggagcgtgtaaaagcagtaaagaaacaccggcatggacgccgtgtgaaacagcttgaaaaaattgaacagaaaatgaaggaggaaaggcaaaaaagaatacgcgagaggcaaaaagagttctttgctgatatagagtctcacaggttggatgactatatttgattcttcattctgacccctttagtatggagatgttatttaaattttttcttacacagtattctcaagtatttgtggcatctatgctctgtttgtacagtactgatgatttggggtctatttgccaatgcagtgactatcaagctttactttcattttggtattgtgtataggctaatatcatctgcattagagccacaacaaaagcagtttacattattcttgcagctaaataaaatccatggtggagcacagcaaaaacaagctggcccttaaataatcaaacataagtaagctaagctgaaataagtaaatggtggtttcttaagtaaatatattgctaaaagaactggatcggaatagctgattcaacctagtcagtagtcacctttgtaaacgctgtctgtctgtgtttacaccccatcaacattttacccatgtcatttggtaataatgccttgcctttgtaacttgcagagagagactggaggatagtttcaaggctaaaagagagcgtctaaagggtttcaatcgatatataaaagagttccacaagaggaaagagcgaattcatcgggagaagctggataggatccagcgggagaaaattaacttgcttaagaacaatgatgtcgaagggtatcttaggatggtccaggtgagtcttatttgctttgtttctcatcatgttcttctatattagcttaacccttcacacgtcaaaaaaagaaaagcttaacccttcattttagtttctcaatatttattggacgaagtcacatctgctaagtgttgctgctttgcaggatgcaaaatctgaccgtgttaagcaactactacgggagactgagaaatatctacagaaacttggggccaaattacgaggtgacagctcaatggacggccgttcttatgtttctggtaagggcgtcactgcaaacgatgttgaagacgagagctaccagccgcaggttttattatctctttgttttagtcaacgtctaggtgcatttttgttgaatatttacttaattttgttctccttccagaattatcttgagagcaacgagaagtactatcagttggcccacaggtactacatggattaaatagactttcatgcttcatttagtaaatccttatcaatgtctgcctagcataaattatgtactacctaactttctaatcctccatcttcttcatacttttttttgaactttaccatcttattcatacttctttgccactgaactttctaattcttttttttagattactgaacttactaattctgctttgtattcatacacatttgtttattttttctagtgtgaaggagattgtaaatgaccagcctacttatcttaatggtgggaaattgcgggagtaagttgtgctgctattttccctgcttttaccttctcattttaagtgtatttttgacattattgttactgacttgtcctgctacaatctgtttaaccatccagtacacatttccttgatctattacttgctgtattacaggtaccagatgaacggtttgcgttggctggtttcattgtacaataataatttgaatggaattttagctgacgagatggggcttggtaaaacagttcaagtaagatccagtacaacgccatctcagcatttattgttcggcttgtatgttatctgatctaaacaagtgtctgaattctgcttacactgcccttgctactttgtcaggtaatctctttgttgtgctaccttatggaaacaaaaaatgaccggggcccatttcttgtggttgtaccatcctctgttctttctggatgggtatctgaactcaacttctgggcacctagtataaataaaattgcttattttggtcctccagaagaaaggcgcagactgttcaagtaaattctgaatttatagttcgatactttatcacagttcatgtgaacattttattaaccaagctaattttttcagagagatgattgttcaacagaagttcaatgtccttttgacaacatatgagtacttgatgaacaaacatgataggccaaaactaagcaaaatacagtggcactatataataatcgatgaagggcaccgtataaagaatgcgtcttgtaagctcaatgctgatctgaagctttatcggagttctcatcggctattgctgacaggaacacctttgcaggttctaaagcttgcacttatactttcacacttgatcctgtatttgttgcttttcaaggaatgcatgaacggcttgctcatatatttatttaatggtcttgggtctctgtatgaagtattctattatgcatatatttcaagttgctaacttctcgtaacttcttgaagaataatcttgaggagctgtgggcacttttgaactttctgttgcccaatatatttaactcatccgaagatttctctcagtggtttaacaaaccatttgaaagcaatggtgataactcagctgatgaggtaaagctgccgtttttcatgatacaacattgttttcttggaaggaaactgtgtttgactccaatcatcttctttcttaaaaggccttactttcagaggaggaaaacttgctgatcataaaccgtcttcaccaagttcttcggccctttgtactccgaagacttaagcataaggtattgattttattcgctatctttatgcttgtgttgaaatcactggcactgtaggaattcaccatgcaatttatttgaaattccaagttccaacaggagatctatgctatgcttagctattcaacctcattatctcaaactgagggagttccagccttccagaattgcatccactgatcacatcggcagaacccttgcttctaaccgaaacctagtcatagtagggagacagataagaaaataattgcttgatgtctttattgatgtgagggcctagccttatatagctggctacatagatatatggaaataaactaacaatcttggaagcttaactagttatttaaaagaaatctaataaccagtaaccaactagaggtgaaatttgttacgtatttgcttaaggcagagcagggggttagacttgaggcattggctgtatgcctgaccccacttgtcacacattataagctcatattatatgagtagtacacatgttccttaaatatgtgtgacctatcaggagttactcacagcatgtaattcggctttcagtatgtcagctgattcagtagacattgcttgatgttccttacttctttttccatttgaagtctttatatgttgcatttgttcggatgattcatatttttgtattgtacgaatgctgagctgggcattgcagtggtgaagagctaaatattgtccataactaggttcaacagcacaacgcaacacaatatagcaacgtcaaactggttctttttagctttgttgctctacatgatctgtaatttaaaaattccatggacaagatttctctatgtgcttgtacacatccatctagctgcctgaatgccaaaaaatgttgcttattctgtttctcaatatatgccactttggcatatcagtacaagcacggtcacacttttcaagtttgaccaccaacatattaaaaacatctagattttcacatcagaaaaacactcgtagctcttccactagagttgctctacaaattgtagatacttttatgaatgtggattttctcaactagttgccgctgtaccctactctagcatccatcgcgaaaagttttaaagagatgggaatttcgtagatgtacagttttgctataatatgtgcagctgataaatgaatgaccatttgtgtattgtgcaaaaaattaaaagatgagtgtctagtatagcaactatatgtgcacacatggtcacactcacccttaaagcatatgtgcgagtattttgcatatctatgacttttttttgctttttgataaagaattacgtgctttccaccttcacatttttgtgaaatgcataagatataattttgccaactactatacaaacatatactccctccgtccgaaaatacttgtcatcaaaatggacaaaaagggatgcatctagaactaaaatacatctagatatatccccttttattcattttgatgacaagtatttccggacggagggagtaatcattaagaccatgaacaggaaagcatctttcatttataaacggtgagtgctccatatttcttagtttatgattactagtaaaaggtactaactctgttcctaaatgtaagacgtttttagaactgcaaaaacatcttacatttatgaacagagggtagagtatacgattcgaacagaaatcatggtatttggcaatgttcaaaaaatcattaactggtagctgcttggtcggctggcgataagggatttataggtgaatcggccagtttaatggcaaatatatcagttaattggcctataagtcaattaatcggctactcggtgacccactgagtagggattaattggccagttaactgatttaccggccgatattctgacaatacttaattatgataattttcgaccatgtggtgtagacgtgcaactttgttttttagaggttggtgaaccaatcttgcaaccggttcattgatttttaaaatttgatatttgaagcaaatttgttactccaaaagtcaaaattttgaatatgaaaactgacttttttgtgataaaattttcacaaaagaataaccgaaagtattgaaattatgcctgataatttcaaatagtcaagaaaactcgatcaaactacatattaattggttcttatgctaatgaccagctgaaaaattggttttggcaggagcactgtagatggtgtgtaaatcaagttcaaaactgctgtttacaagtactccctccgtaaagaaataaagagcgtttagatcactagatctaaatgctcttatatttatttacagagggagtagtagagattatgattactttaagttgcaacttagttaaaaagcaactcatatgtccatgcccccttttctcttggttttgaattgatttttgtttagactttagaaccgttgatgtcgaataaatttgaaagaagcaccaatcattggagctccaaccatttgtacttctttcaaacttactcaacatcaacggttctaaagtctaaacaaaaagctactattgtgatgctgtgtgggaaactagctcgtcaggttggggacttgatattgtttcccaattgtttctcgtctttgtttgtatctagatcatctggatggtgcaatagtttcaattgtgttttactgtcttcaggttgaaagtgaattgccagggaagattgaaagacttgtaagatgcgaggcatcagcttatcagaaacttctgatgacaagggtggaagacaaccttggtggaattggagcagttaaggtgcgtagcgtgtgactgttcgagttgtttattttaatgtttcacttgtcagatatttcacaggttcttatttgtaatatgtgtcttaaattttttaggtccgctcggtgcacaattctgtcatggaattgaggaacatatgcaaccatccataccttagccagcttcatgttgaggaggtagagcatgattctgccctgtcgccacattctggctatttttgtttcctcttgggcattaccagccatatggattttctatgcagattgagggtcatctacctaggcactacctgccatctattgtgaggctgtgtgggaaacttgagatgttggacagattgctacccaaactcaaagctactggccatagggtaagtggattttattggtagtgtggtaggtttgtaaaggcctcctactcgtatgtcgcatgaattgtattttcttgaacaagtcacacatcaaacttgcattatctgagttgaagttgtcgttcgttccttgttccttggcatgcaggttctacttttttctacaatgacaagattgcttgatgtgatggaggattatctggtatggaaaaagtatcagtaccttcggttagatggacacacttctgggcatgagagaggagcacttattgatagatttaatgatcctgattctccagctttcatttttctgctaaggtaaaatattggttcagtatattgtgctgtaggaggtattatataaatagaacatagtgaactcatgaatccttatcggccaatttgattaattaatatttgatatctaaggcctacttcacccctatttctgtagtatccgagcaggaggcgttggtgtcaatcttcaagcagctgatactgtcatcatatttgatactgattggaatcctcaggtagctaaagttccttcagtgttgtcactctatgttgtaagatttgttttacataaatatatcttttccttgattatttcaggttgacttgcaagcacaggctagagcccacagaattggtcaaaagaaggaggttcttgttttacgtttagaaactgtaagtgcacactgacagttcgcttatcacctggagtaaatatgtagaaaccaaaatgaacaaggaacatttgtttgctaacaaggaaatggtagttaacaaatagaacaagtcgccagttgagtcctttgtgttgcatagggtttgtttgagcatcttagatcaatagttagatatgtggcttatgtggtattctaaatgaagaactggtccagatttactcaatgccactccaccatggggatgtgcccccatgcatgaacagcaccctgcttgcactttcttcctcacttcatgtaaaagggttaattcggaggtgcaatgttttgactcatcatgcattatatgctactatgcccacactggaatctggattccaaacccactaaggtcaccactctaaacaggctggatgttggagcctagatacatatctgtacgtcacagtattgtctttattggtgatgataaagtcatcctagtattgtttttatctaaatttgagtaattttcacgactgcaacaacaaagcctttataattttcacgactacgtataaagaattaagaaccagcaccattgctcgcacaagtttctggaacactcattaataaactgtaaggctgtagctgtctaattttgtcatataactcacatttttcttgaaagcttctcaattatatacctgaaagtgtcctttgttttatgtcattttgtgtatttaggtattttgttggtatttaatattgcttgttttcagatttattcaagaaattagtgatgtgcctggtctatcttcattgtattatagcttgggttttcctctctttgcgccaatttgtggctgttgtgttgctgcgctgctttggaacctagctatagggatctttactgttttcttgtatattttggtgatatgactccaaaagaagttactttcaactgcctccctcggagaattcgcttctgaatatctgtccatggagaatatcacgagtgtagttattgctgtgtttccagtctattcttaaatgctttgtatctgtcaattagtaggggtacgcatggtcatttctcattaactctcagatttagtgctctctttgtccgttcgcttgatgaagtaactatccatatgtggaaaaagttactgcactagctaccagatcgcgactgctctctacggagcctttgtcttcttggctgtttatttttctaagcttggacagaacccactagcgatttatgacactgccacaaatatgataggaataaatgctgcctgttatgttctaaccagaaccaatgcattgtattacttcaactgaaaatttcaatacgcctgttcctgacttggatgtaccttgttgaatttaaggtccgaactgtagaagagcaagtcagggcttcggcagaacataaattaggcgttgctaatcagagtataactgctggattttttgacaacaacacaaggtcaattcttctactcggttaagattttagcttttctagctctcttttttcctttccttcatgctaggtggtaacaattgcagtgctgaagatcggagggagtatcttgagtcacttctacgtgagtgtaaaaaggaagaatcagctccagtgttagatgatgatgctctgaataatattcttgcccgcaggtaagactgagtttgctgttagtattatttaagcattgttttaacaatctctgtcactcctgatactttatctaattgcatgacatatcacttttctctccttgcagcgaagatgagatcgacatatttgaatctattgacaagcaaagactagatgatgaaatggtatactaaattcctttactttgtacatgcttatttctgctaatattttgtgcataccaatttaattcttgtatcccttgtaggctgtatggctaaaggttgttcaggatggttcagttagtgggctagacccctcagtattgccaccccgccttgtgtctgatgatgatctgaagcccttctgtcatgctatgaagatttacgagtcttcaaatgtaaaaaatgtgaaggtaaatgtgaggaagaagggcgagcttggtggccttgatacaaagcattacggaaggggaaaacgtgctcgtgaggtcagttgcattatcatcttctatacgtctctctattattggttgaagtatttgtttgctaatttcattatatatcctttgtaggtccggtcttatgaggatcaatggaccgaagaagaatttgaaaaactttgtcaggctgaatctcctgactcacctcaacctggtggtgcattgaaggatatagatatctctaaagagagtaagttggaggtacctgcagaaagttcaatagacccaaaagaaagttcaatagatccagttgaagccaaaacggtaccagtcctggctgttccagactcctcaccaccagtcctgtctgttccagactcctcaccagctaagcggcgaagaggtagacctagaaggtcagacgtttcagtatctcctgttatgtccccagcaaaagctgtccaacaagaggcaggaactacacttggcagttctgcaccagcaagtaccatcgattctgcagcaccaactgctaccatccattctactggtccagatgttaccacccattctgctgcaccagttgctgccatcaaaccagttattggtacagaagttaaggctactgcttttgttgctgctgtaccaactgctaccatgaaacccgagattggtactgaagttacggaccatgttgttttggaagggtctatagcaaaggaagttggtccggcggtagagagcggtcatgacccagtagctgccagtgcagcccctcatccaccagctcctgctacgtctagaggcagaaagacccaagcagttgaaacccctcgcagacgaggccgtaaaccaaaaactctttcctcatctagtgctggtgatgttaatacaaaccctgtggttgcaattggtagtggacctgcttctgtgggttctccataccctcaaggggatatgccctcatcacatgcaagtctcatgtcaagatttcagaaggatttggttacaggtaggcctgttacgtcattgccagagggagttaagggcatctccgcccctgaaggtacgacacctgttgccgaaggtaaacacactggaactgcaataagcttggacaatgccagctcactaatgccaaagatcattcacaacgaaaaagttggatttgttcaagcgagctctgagcaagttttttctgcatcagtacctactttaactgccgtctcaggtggaatattgaaagcatcacatgttctcttggcagataagcctgcagagaagcaaagtgcttcacgccgtcgcagaaagaaagcgcctggtggtgaggatactggagtaagtactaggcaaagagcagctatgaagaaatctgatggtattcctggtaccactgacaatgttggcgcggacatgagcacagctgagaagctaggagcagtgaatgtaaaagatggcagttcacttcaagatactcccaaggaattaccaaatataaactctcctccatatgacaagtctgggtatgactctcaaccaagaacaccaatagcagttcccattagtgaagctgcagctcctagtggttccggtaatgcccatgttgcttattctgatataactcctaggatacctaccaatcctgatgttcaagataaaccagtaaatctgcacacaggagcacctctagccgcagcctcacaacctgttgcagtgtgttctgtggtcactaccacacattctgaaacggttactgaaaaaccattgctaaatcctgttagtgaactagcaaatgtccaggtcgaaccacctagttcttcacttcataattcaggtgagaacatcagtacagtgccttcagaggtcaatagtgtcgctcccagtaaggcatcaggtaggaggaggaaaggtcctgcctctgaaccacgcaccagaagtaaagccgcaacagctgcatgtgaacgtcgtgctcgattagctggatcaaagcagacaagtgatgcgagaaaattagaaatatcggcaagcccaagcacggtggtttgtgtttcttcagttgagcaacaggaaaccgccctggcagagcctctcactgcttatgtctgcgaaccgcagaagaatgctgagagtcatgtacgtggtggaatgtctactccgatggggatactagatgccccaaagcaaattgctacccagtcaattacagcatgtactgaagaaacaaatagcagtttaagcactcagactcctgcacttcccatatccagaaaaagtaatctttccatgggtgacaagcaaggttctctctctctctctctctctctgctgttattattcattgtttggtagtaacaatggctcatgctgatgctcatgatgcctttttcaggtgttggagttgataccatacatggacaaacaaatatggttttggctgcagaactggcatctgcaaatgatgaacataagctgcatgaagtacatgataagactgctgatggtaatatactccaacacagtgcggcgcatgacacactccaggataaaactgatagcattgctggtttgaacctagcttctcgtcatagaattagtgatttggaaatggaaaaggatgattctaatacagtgatgttaccagactgccaaaccccttttgatgcctcagttaaggatagtaaggatactcttgcccccacagaagctgatgtcagtgatctgcaaaatgaggctgctgctattgatgtgactagtcctaagcaagatactatggtagttgaagcactgcacactaattctggaggttctgctagtcatctgcctgctgctttacgatcaacgggctcaaaccagcatgcagaagggaaaggaagttcaaagaacagtggctctaaattttttgcatctgggaagaaaacagaggaaatggaaggaactttggataagaatacggatcacaatcttattcaggcaaatgccaatatagctttaggaagacattctccttcagatgacaaaagagaggacagttgtgcccatgtagttgatggtggcctgtcgggaagcaaacaaactcttcctgaagtcgtttctgcagtaaacactgatggctctgaggaagcactcaatgcttcatctacccattcgaataaagatgccaccttggtttgtgaagtaacaaaggatcctgagagccatgtatcagtgtctgtactggcctctgctgctatgaacgctggtgatgactgtgcggaagttcacaatgttccatccacccattctgaaagagggggcagcatggtagaagttgatgcgtctagagatgatgctacctctatttgtgaagtacgcaaggatcctgagagtaatgtatctggtgagttgtcgatgccagtagggttagcggagctcgagttagaactgccaaaccaatccaaatcttctagccagtctagcgcagtaaaggctgatgaaacaaaggccagtatcaacattcagactacttcattggtagaatcaggagaacaaaaatcacccagaaatggtgcacatggtactccctatctctatcccctctttccccctccctctctcaccaaccatgatcctgtacacattccccggtgtatgctgattgttattcttatccagctagtgtatcttttttatgttttgccagaagagatggagttggctgggcctaagattgagtgcacaatacaaatgctgagtcctgatgataagagtatgctctgttattactttctgttgtagtagagacgggccagggggctcatgcacatctgcaccttttcaggttctgaggctcatagtttggcacaacgcgagatggtttcgggtgcagaacaagcatctatgaaaggtataatctggttttaaatttctgaattaattaacgcatggtcaatagttactcatgggtagtttatctaacatatgtacagatgatagagaaaacaagatggttgatgttatatttttgtctggtggggaacaagaaacacagcgagctgatgtagacttgcccactagtccaagatatgcagattgtgagggtgaaaaggaccattcccctaaaactattttggcaggcagccaatctttttgtgaagcctcagataaggacgttgccccagtgaaagatgatcacactgatccgcaaagtgaagttaatgttgttgatatgaatggtaccaaccaagactcagctgaaaccgaagctatgcagattgatggtgtctccaaaggatcttcaagtgatttgcctgctgctttacgatcgaccaattcaaatcagccggcagaacaagatggattagagaatagtccctctatatctgcttgtccgaaagaaaatgagaaattggaagaaacttctgatgaaattggtggtggcaattccaatcgtagtcggactgatggtgattctcatattatgaatctagttggttattcggaagactcagatgaggacgattctatccaggtagctgatgttggtgatgtgggatgtaaagaaactactcatgatgacatctcagctgtcgctagaggagcagaaccaggagatggaccctgcacagagcctacttgtgaaactgctgttcatgtgcctgaagctatttctgaggatggtcatggcacaacggcccttggcagtgtccaagtgtctacgacggaaataaaggatttggagagtggaagatgtctagaacatggaacaggtatttctttatctgcttgcaatgttcatcaaagcccactgaacaaagaacttagttatgctatttcagtaattcctgaccctgttgagcatgatggcacaggaacccctgtggttcttcaggagggaactgctgtcgctacagaaccagaagcaaagaaagaggtcgacgaacctactcaaaatgaagatgttgagccggctgccataaagccagaggcagtggagcatgctggtacagaagctgatccaagtaaagaagcatctatacctccacaagaggaaaccgctgctgtagccttggttacaggaccggaacaaaatgaagaagcagatgcacctactcaagtcgaacccgttgccatagtgccagattccatggagcatgctagtacccaagttgatcaaagtatagaaacagctgtgcgtctcccagacgaaacttctgttatacctggtacggaaccagaagagaagaaagtagaggcatccccccaagaggataatgttggagcagttgccgcagagccagaacctgctggaacccaggaaaatgcagaagtttctactcagcctagtcctatggagatagagttggctcaggaaacagctatgctgggagaagctgaaaccaggcagcaactgccacttccgtctgccgagggcgtgatagccgaggctagtgaacctccaagcacagaggtgactgctatgaaggaaccagagttgctgagcactgaaccagcacccgatggtgaaaacgcgaagcttggagaagccgaagctgaacagctgtcgcagcaaccttcatcctgcgaggctatggcagtcacaggagagcttcctagcacagcgggagcgaaaacggatggaacttcagacgtggtggcgtctcctgctgtcgtgggagaggaggtgctcaacactgaaactgcacctgatggtaaaaatccaaggccgagcgaggctgatacggcgcagtccccacctttgccggaggagggcaaggccgtggcagctactgagcctgccaaccttgaggaggcggaggctaatgatggaaagtagttagcgtgcaaggatggaagcagatgttgcgttgaagaacctttgccgttagatcagacagagcatgcttgggatcaagagagaggatctaggggctgttgaaactgagaagtaccgtagattttatgcaaatgttgtatgtaaaacataattaagaaacctgttgtattcgaaggagtggagttgttggtacataagttataactacctagtcgctttgcaatactagtaccttgttgcacctga

SEQ ID NO: 10 - DNA, 10104 bp, Triticum aestivum
  source 1..10104: mol_type = other DNA
  CDS 1..10104: protein_id = 11; translation = MASSQHVEVEAAKLLQKLILESKDEPAKLATKLYVICQHMKLSGKEQSLPYQVISRAMETVVSQHGIDMDALRSSRVPFAGGPQAVDSSGVMSKDKEIIGGQSSMVGSDASQSSGQAALWHLPPGSADMARPGVYIPGRVPAGQNRGDVAGSDIHQGSMSQKSGRSSGVESPASLQMEDTRSMNSHDSLKSDEKTSKKASSSKRKRMDSKAAGDMQSEENSKSDGISSGQNIRKRKQVGKAGAQGQPSRGAEPEQSHILQGATAQVPPLPGGASFFRAHQEGPPASAGRTIDNTKPSNPFAMSQVSNFAEGLASGSIPTELQKSILGGTNMFNTGFGWNQSSQGSAIKNTQGSVANLMRPGVNVEGKINVGSQGAFNPTPTSQMDFPKIPPYMSSSFGGGSQFLDKGKDSASGNTGTELHSAAKVGVNMGIVHGSPMQERQNITRAPQRAESSLQEARLSSLPNRNVGPYQTSHISPNTPFKEQQLKQLRAQCLVFLAFRNNMQPRKVHLEIALGGGPTAEGGGAGQGGNESRVADGSVRENGNSQENSAIFGSQSDMSRLPSTSAGSIAEADSSLKDSEIKKKINIAEHEKSSMEIENIQQAVMQGTGSSSEMRSQEIASPVPSGPQQSYFQGDKRRNAPETYRTDAENLNRNLGFGGQGPSSLGGNRQHPNFEAAVLTKDRLQDEASKESYPPSRLHHMPIDGYSSNLPGKDLTPDTDRNEVEHCTQMGEMSDRSADEGDDDLFEHDDFASTPPKYTMTEKWIIDYQKRKYGENEKKVLEQQSAHKRMSASYQKLKESVSSSEDLTAKTKSVIELKKLQLLSLQRRVRSEFLSDFFKPNTADLERVKAVKKHRHGRRVKQLEKIEQKMKEERQKRIRERQKEFFADIESHRERLEDSFKAKRERLKGFNRYIKEFHKRKERIHREKLDRIQREKINLLKNNDVEGYLRMVQDAKSDRVKQLLRETEKYLQKLGAKLRGDSSMDGRSYVSGKGVTANDVEDESYQPQNYLESNEKYYQLAHSVKEIVNDQPTYLNGGKLREYQMNGLRWLVSLYNNNLNGILADEMGLGKTVQVISLLCYLMETKNDRGPFLVVVPSSVLSGWVSELNFWAPSINKIAYFGPPEERRRLFKEMIVQQKFNVLLTTYEYLMNKHDRPKLSKIQWHYIIIDEGHRIKNASCKLNADLKLYRSSHRLLLTGTPLQNNLEELWALLNFLLPNIFNSSEDFSQWFNKPFESNGDNSADEALLSEEENLLIINRLHQVLRPFVLRRLKHKVESELPGKIERLVRCEASAYQKLLMTRVEDNLGGIGAVKVRSVHNSVMELRNICNHPYLSQLHVEEIEGHLPRHYLPSIVRLCGKLEMLDRLLPKLKATGHRVLLFSTMTRLLDVMEDYLVWKKYQYLRLDGHTSGHERGALIDRFNDPDSPAFIFLLSIRAGGVGVNLQAADTVIIFDTDWNPQVDLQAQARAHRIGQKKEVLVLRLETVRTVEEQVRASAEHKLGVANQSITAGFFDNNTSAEDRREYLESLLRECKKEESAPVLDDDALNNILARSEDEIDIFESIDKQRLDDEMAVWLKVVQDGSVSGLDPSVLPPRLVSDDDLKPFCHAMKIYESSNVKNVKVNVRKKGELGGLDTKHYGRGKRAREVRSYEDQWTEEEFEKLCQAESPDSPQPGGVLKDIDISKESKLEVPAESSIDPKESSIDPVEAKTVPVLAVPDSSPPVPSVPDSSPAKRRRGRPRRSDVSVSPVMSPAKAVQQEAGTTLGSSAPASTIDSAAPTATIHSTGPDVTTHSAAPVAAIKPDIGTEVKATAFVAAVPTATMKPEIGTEVTDHVVLEGSIAKEVGPAVESGHDPVAASAAPHPPAPATSRGRKTQAVETPRRRGRKPKSLFSSSAGDININPVVAIGSGPASVGSPYPQGDMPASLMSRFQKDLVTGRPVTSLPEGVKGISAPESTTPVAEDKHTGTAISSDNANLLMPKIIHNENVGFVQASSEQVFSASVPTLTAVSGGILKASHILLADKPAEKQSASRRRRKKAPGGEDTGVSTRQRAAMKKSDGIPGTNDNVGADMSTAEKLGAVNVKDGSSLQDTPKELPNINSPPYDKSGYDSQPRTPIAVPISEAALPSGSGNAHVAYSDITPRIPTNPDGQDKPVNLHIGAPLAAASQPQVPCKTGNDHVAVCSVVTTTHSETVTEKPLLNPVSELANVQVEPPSSSLNSGKNISTVPSEVNSVAPSKASGRRRKGPASEPRTRSKAATAACERRARLAGPKQTGDARKLEILASPSTAVCVSSVEQQETALAEPPTASVCEPQKNAESHVRGGMSTPMGILDAPKQIATQSITACTEETNSSLSTQTPALPISRESNLSMGDKQGVGVYTIHGQTKMVLAAELASANDEHKLHEVHDKTADGNILQHSAANDTLQDKTDSIAGLDLASRHRIGDLEMEKGDSNTVMLPDCQTPFDASVKDIKDTLAPTEADVSDLQSEAAAIDVTSPKQDTMVVEALHTNSGGSASHLPAALQSTDSNQHAERKGSSENSGSKFFASGKKTEEMEGTLDKNTDNNLIQANADIALGRHSPSEDKREDSCAHVVDGGLLGSKQTLLEVVSAVNTDGSEEALNASSTHSNKDATSVCEVTKDPESHVRVSVLASAAMNARDDCEEVHNVPSTHSDRGGSMVEVDASRDDATSICEVCKDPESNVSGELSMPVGLAELELELPNQSKSSSQSSAVNADETKASINIQTTSLVESGEQKSPRNGAHELKEGMELAGPKIECTILMPSPDDKSSEAHSLAQREMVSGAEQASMKDDKRNKMVDVTFSSGEEQEIQRADVDLPTCPRYADCEGEKDHSPKTILAGSQSFCEASDKDVAPVKDDHTDPQSEVNVVDMNGANQDSAETEAMQIDGVSKGSSSDLPAALRSTDSNQPAEQDGLENSPSISACPKEHEKLEETSDEIGGGNSNRSRTDGDSHIMNLVGYSEDSDEDNSIQVADVGDVGSKETTHDGISAVPRGAEPGDGPCTEPTCETAVHVHEFNVDVAISEDGHGTMALGSVQASTTELKDLESGRCLEHGTGTPVALQEGTAVAAEPEAKKEVDEPKDVEPAAIKPEAVEHDGTEADPSKEASIPPQEETTAVALVTGPEQNEEADAPTQVKPVAVIPGTGPEEKKVEASTQEDNAEAVAAEPESARAQENAEASTQPSPMEIESVQETAMLGEAETRQQLPLPSAEGVVAEASEPPSIEVAAMKEPELLSTEPAPDGENAKLGEAEAEQLLQQPSSCEAMAVTGELPSAVGAKTDGTSDVAADESPAVVGEEVLNTETAPDGENPRPSEADTAQSPHLPEEGKAVAATEPANLEKAEANDGK
atggcttcatcacagcatgttgaagtggaggctgcgaagctacttcaaaaactcattctggaatcaaaggatgagcccgctaaattagcaacaaaactttacgtgatatgtcaacatatgaagttaagtggaaaagagcagtctcttccctatcaggtcatatctagggccatggagactgtcgtaagtcaacatggaattgatatggatgcattgcgatcatcacgagttccatttgccggcggtccacaagcagtagattctagtggcgttatgtctaaggacaaggagatcattggtggtcagtcttccatggttggaagtgatgcatcccagagcagcggtcaagctgcattatggcatttgccaccaggttcagcagatatggcaaggcctggggtgtatattccaggcagggttccagcaggacaaaataggggcgatgtcgcaggatctgatattcatcaaggctccatgtcgcaaaagagtggcaggtcctctggagtcgaaagccctgcaagtctgcaaatggaggacactagatctatgaattcacatgattctttgaagtctgatgaaaaaacaagcaagaaagcttcctcttccaagagaaaaaggatggattcaaaagcagcaggggatatgcaatctgaagaaaactcaaaatcagatggtatctcaagtggacaaaatattagaaaaaggaaacaggttggcaaagctggtgcacaaggtcagccctccaggggagctgagcctgagcaatcacatatactgcaaggtgctactgctcaggtgccacccttacctggtggtgcatcatttttcagggctcaccaggaaggtccaccagcttctgctgggaggactattgacaatactaaaccatcaaacccattcgcaatgtcacaagtttcaaattttgctgaagggctggcttctggtagtatccccactgagttgcagaaaagtatactgggaggaacaaatatgtttaacactggttttggctggaatcagagttcacaaggttcagctattaagaatactcaaggttctgttgccaacttaatgcggccaggagttaatgttgaagggaaaattaatgtagggtcacaaggagcttttaaccctactcccacatcgcagatggattttcccaaaatccctccttacatgtcttcttcctttggaggtggctcacagtttctggacaagggcaaggactcggcttctggcaataccggcactgaacttcattctgctgctaaagttggagttaacatggggattgtgcatggcagtccaatgcaagaaaggcaaaatattaccagagcaccacagagggccgaatcatctttgcaagaagccagattgtcttcgctcccgaatagaaatgttgggccatatcaaacgtctcacatctctccgaacacacctttcaaagaacaacagttaaagcagctccgagcacagtgcttagtatttcttgcattcagaaataatatgcagcccagaaaggtgcaccttgaaattgccttaggtggaggccccactgcagagggtggcggtgcaggtcagggaggtaacgagagcagagtggctgatggttctgtaagggaaaacggaaacagtcaggaaaactctgctattttcggcagccaaagtgatatgtctagactcccatccacatccgcaggcagcattgcagaggctgattcttcactgaaggactcggaaattaagaagaagatcaatatagctgaacatgagaagtcatcgatggaaatagaaaatatccagcaagctgttatgcagggaactggttcaagttctgaaatgcgctcccaagaaatagcatcccctgtgccatctggaccacagcagtcatactttcagggagataaaagaagaaatgcccctgagacctacaggacggatgcagaaaatttgaacaggaatttaggtttcggaggccagggaccatcttctttgggtggtaatagacaacatccaaattttgaagctgctgttttgaccaaagatcgattacaggatgaagcatctaaagaatcatatccaccttcgaggcttcatcacatgcctatcgatggttacagctccaatttaccaggaaaggatctaactccagatacagatagaaatgaagttgaacattgtacccagatgggggagatgtctgatcgatcagctgatgaaggagatgacgatctatttgagcatgatgattttgcatcaactcctccaaaatacacaatgactgaaaaatggatcatagattatcaaaagagaaaatatggagaaaatgaaaagaaggtattagagcagcagagcgcacataaaaggatgtcagcatcctatcagaagttaaaggaaagtgttagttcatctgaagatcttactgcaaagacaaagagtgtcattgaattgaaaaagcttcaacttctctcacttcaacgtcgtgtgcgcagtgaattcttgtcagactttttcaagcctaatacagctgatttggagcgtgtaaaagcagtaaagaaacaccggcatggacgccgtgtgaaacagcttgaaaaaattgaacagaaaatgaaggaggaaaggcaaaaaagaatacgcgagaggcaaaaagagttctttgctgatatagagtctcacagagagagactggaggatagtttcaaggctaaaagagagcgtctaaagggtttcaatcgatatataaaagagttccacaagaggaaagagcgaattcatcgggagaagctggataggatccagcgggagaaaattaacttgcttaagaacaatgacgtcgaagggtatcttaggatggtccaggatgcaaaatctgaccgtgttaagcaactactacgagagactgagaaatatctacagaaacttggggccaaattacgaggtgacagctcaatggacggccgttcttatgtttctggtaagggcgtcactgcaaacgatgttgaagacgagagctaccagccacagaattatcttgagagcaacgagaagtactatcagttggcccacagtgtgaaggagattgtaaatgaccagcctacttatcttaatggtgggaagttgcgggagtaccagatgaacggtttgcgttggctggtttcattgtacaataataatttgaatggaattttagctgacgagatggggcttggtaaaacagttcaagtaatctctttgttgtgctaccttatggaaacaaaaaatgaccggggcccatttcttgtggttgtaccatcctctgttctttctggatgggtatctgaactcaacttctgggcacctagcataaataaaattgcttattttggtcctccagaagaaaggcgcagactgttcaaagagatgattgttcaacagaagttcaatgtccttttgacaacatatgagtacttgatgaacaaacatgataggccaaaactaagcaaaatacagtggcactatataataatcgatgaagggcaccgtataaagaatgcgtcttgtaagctcaatgctgatctgaagctttatcggagttctcatcggctattgctgacaggaacacctctgcagaataatcttgaggagctgtgggcacttttgaactttctgttgcctaatatatttaactcatccgaagatttctctcagtggtttaacaaaccatttgaaagcaatggtgataactcagctgatgaggccttactttcagaggaggaaaacttgctgatcataaaccgtcttcaccaagttcttcggccctttgtactccgaagacttaagcataaggttgaaagtgaattgccagggaagattgaaagacttgtaagatgcgaggcatcagcttatcagaaacttctgatgacaagggtggaagacaaccttggtggaattggagcagttaaggtccgctcggtgcacaattctgtcatggaattgaggaacatatgcaaccatccataccttagccagcttcatgttgaggagattgagggtcatctacctaggcactacctgccatctattgtgaggttgtgtgggaaacttgagatgttggacagattgctacccaaactcaaagctactggccatagggttctacttttttctacaatgacaagattgcttgatgtgatggaggattatctggtatggaaaaagtatcagtaccttcggttagatggacacacttctgggcatgagagaggagcacttattgatagatttaatgatcctgattctccagctttcatttttctgctaagtatccgagcaggaggcgttggtgtcaatcttcaagcagctgatactgtcatcatatttgatactgattggaatcctcaggttgacttgcaagcacaggctagagcccacagaattggtcaaaagaaggaggttcttgttttacgtttagaaactgtccgaactgtagaagagcaagtcagggcttcggcagaacataaattaggcgttgctaatcagagtataactgctggatttttcgacaacaacacaagtgctgaagatcggagggagtatcttgagtcacttctacgtgagtgtaaaaaggaagaatcagctccagtgttagatgatgatgctctgaataatattcttgcccgcagcgaagatgagatcgacatatttgaatctattgacaagcaaagactagatgatgaaatggctgtatggctaaaggttgttcaggatggttcagttagtgggctagacccctcagtattgccaccccgccttgtgtctgatgatgatctgaagcccttctgtcatgctatgaagatttacgagtcttcaaatgtaaaaaatgtgaaggtaaatgtgaggaagaagggcgagcttggcggccttgatacaaagcattacggaaggggaaaacgtgctcgtgaggtccggtcttatgaggatcaatggaccgaagaagaatttgaaaaactttgtcaggctgaatctcctgactcacctcaacctggtggtgtattgaaggatatagatatctctaaagagagtaagttggaggtacctgcagaaagttcaatagacccaaaagaaagttcaatagatccagtcgaagccaaaacggtgccagtcctggctgttccggactcctcaccaccagtcccgtctgttccagactcctcaccagctaagcggcgaagaggtagacctagaaggtcagacgtttcagtatctcctgttatgtccccagcaaaagctgtccaacaagaggcaggaactacacttggcagttctgcaccagcaagtaccatcgattctgcagcaccaactgctaccatccattctactggtccagatgttaccacccattctgctgcacctgttgctgccatcaaaccagatattggtacagaagttaaggctactgcttttgttgctgctgtaccaactgctaccatgaaacccgagattggtactgaagttacggaccatgttgttttggaagggtctatagcaaaggaagttggtccggcggtagagagcggtcatgacccagtagctgccagtgcagcccctcatccaccagctcctgctacatctagaggcagaaagacccaagcagttgaaacccctcgcagacgaggccgaaaaccaaaatctcttttctcatctagtgctggtgatattaatataaaccctgtggttgcaattggtagtggacctgcttctgtgggttctccatatcctcaaggggatatgcctgcaagtctcatgtcaagatttcagaaggatttggttacaggtaggcctgttacgtcattgccagagggagttaagggcatctccgcccctgaaagtacgacgcctgttgccgaagataaacacactggaactgcaataagctcggacaatgccaacttactaatgccaaagatcattcacaatgaaaatgttggatttgttcaagcgagctctgagcaagttttttctgcatcagtacctactttaactgctgtctcaggtggaatattgaaagcatcacatattctcttggcagataagcctgccgagaagcaaagtgcttcacgccgtcgcagaaagaaagcgcctggtggtgaggatactggagtaagcactaggcaaagagcagctatgaagaaatctgatggtattcctggtaccaatgacaatgttggtgcggacatgagcacagctgagaagctaggagcagtgaatgtaaaagatggcagttcacttcaagatactcccaaggaattaccaaatataaactctcctccatatgacaagtctgggtatgactctcaaccaagaacacctatagcagtccccattagtgaagctgcacttcctagtggttccggtaatgcccatgttgcttattctgatataactcctaggatacctaccaatcctgatggtcaagataaaccagtaaatctgcacataggagcacctctagccgcagcctcacaacctcaagtgccatgtaagacagggaacgaccatgttgcagtgtgttctgtggtcactaccacacattctgaaacggttactgaaaaaccattgctaaatcctgttagtgaactagcaaatgtccaggtcgaaccacctagttcttcacttaattcaggtaaaaacatcagtacagtgccttcagaggtcaatagtgtcgctcccagtaaggcatcaggtaggaggaggaaaggtcctgcctctgaaccacgcaccagaagtaaagccgcaacagctgcatgtgaacgtcgtgctcgactagctggaccaaagcagacaggtgatgcgagaaaattagaaatattggcaagcccaagcacggcggtttgtgtttcttcagttgagcaacaggaaaccgccctggcagagcctcccaccgcttctgtctgcgaaccgcagaagaatgctgagagtcatgtacgtggtggaatgtctactccgatggggatactagatgccccaaagcaaattgctacccagtcaattacagcatgtactgaagaaacaaatagcagtctaagcactcaaactcctgcacttcccatatccagagaaagtaatctttccatgggtgacaagcaaggtgttggagtttataccatacatggacaaacaaagatggttttggctgcagaactggcatctgcaaatgatgaacataagctgcatgaagtacatgataagactgctgatggtaatatactccaacacagtgctgcaaatgacacactccaggataaaactgatagcattgctggtttggacctagcctctcgtcatagaattggtgatttggaaatggagaagggtgattctaatacagtgatgttaccagactgccaaaccccttttgatgcctcagttaaggatattaaggatactcttgcccccacagaagctgatgtcagtgatctgcaaagtgaggctgctgctattgatgtgactagtcctaagcaagatactatggtagttgaagcactgcacactaattccggaggttctgctagtcatctgcctgctgctttacaatcaacggactcaaaccagcatgcagaacggaaaggaagttcagagaacagtggctctaaattttttgcatctgggaagaaaacagaggaaatggaaggaactttggataagaatacggataacaatcttattcaggcaaatgccgatatagctttaggaagacattctccttcagaggacaaaagagaggacagttgtgcccatgtagttgatggtggcctgttgggaagcaaacaaactcttcttgaagtcgtttctgctgtaaacactgatggctctgaggaagcactcaatgcttcgtctacccattcgaataaagatgccacctcggtttgtgaagtaacaaaggatcctgagagccatgtaagagtgtctgtactggcctctgctgctatgaacgctcgtgatgactgtgaggaagttcacaatgttccatccacccattctgatagagggggcagcatggtagaagttgatgcgtctagagatgatgctacctctatttgcgaagtatgcaaggatcctgagagtaatgtatctggtgagttgtcgatgccagtagggttagcggagctcgagttagaactgccaaaccaatccaaatcttctagccagtcaagcgcagtaaatgctgatgaaacaaaggccagtatcaacattcagactacttcattggtagaatcaggagaacaaaaatcacccagaaatggtgcacatgagttgaaagaagggatggagttggccgggcctaagattgagtgcacaatactaatgccgagtcccgatgataagagttctgaggctcatagtttggcacaacgggagatggtttcgggtgcagaacaagcatctatgaaagatgataaaagaaacaagatggttgatgttacattttcgtctggtgaggaacaagaaatacagcgagctgatgtagacttgcccacttgtccaagatatgcagattgtgagggtgaaaaggaccattcccctaaaactattttggcaggcagccaatctttttgtgaagcctcagataaggacgttgccccagtgaaagatgatcacactgatccgcaaagtgaagttaatgttgttgatatgaatggtgccaaccaagactcagctgaaaccgaagctatgcagattgatggtgtctccaaaggatcttcaagtgatttgcctgctgctttacgatcgaccgattcaaatcagccggcagaacaagatggattagagaatagtccctctatatctgcttgtccgaaagaacatgagaaattggaagaaacttctgatgaaattggtggtggcaattccaatcgtagtcggactgatggtgattctcatattatgaatctagttggttattcggaagactcagatgaggacaattctatccaggtagctgatgttggtgatgtgggaagtaaagaaactactcatgatggcatctcagctgtccctagaggagcagaaccaggagatggaccctgcacagagcctacttgtgaaactgctgttcatgtgcacgaattcaatgtggacgttgctatttctgaggatggtcatggcacaatggcccttggcagcgtccaagcgtctacgacggaactaaaggatttggagagtggaagatgtctagaacatggaacaggaacccctgtggctcttcaggagggaactgctgtcgctgcagaaccagaagcaaagaaagaggtcgacgaacctaaagatgttgagccggctgccataaagccagaggcggtggagcatgatggtacagaagccgatccaagtaaagaagcatctatacctcctcaagaggaaaccactgctgtagccttggttacaggaccggaacaaaatgaagaagcagatgcacctactcaagtcaaaccagttgctgttatacctggtacgggaccagaagagaagaaagtagaggcatccacccaagaggataatgctgaagcagttgccgcagagccagaatctgctagagcccaggaaaatgcggaagcttctactcagcctagtcctatggagatagagtcagttcaggaaacagctatgctgggagaagctgaaaccaggcagcaactgccacttccgtctgccgagggtgtggtggccgaggctagtgaacctccaagcatagaggtggctgctatgaaggaaccagagttgctgagcactgaaccagcacctgacggtgaaaatgcgaagcttggagaagccgaagctgaacagctgttgcagcaaccttcatcctgcgaggctatggcagtcacaggagagcttcctagcgcagtcggagcgaaaacggatggaacttcagacgtggcagctgatgagtctcctgctgtcgtgggagaggaggtgctcaacactgaaactgcacctgatggtgaaaatccaaggccgagcgaggctgatacggcgcagtcgccacatttgcccgaggagggcaaggccgttgcagctaccgagcctgccaaccttgagaaggcggaggccaatgatggaaagtag

SEQ ID NO: 11 - protein, 3367 aa, Triticum aestivum
MASSQHVEVEAAKLLQKLILESKDEPAKLATKLYVICQHMKLSGKEQSLPYQVISRAMETVVSQHGIDMDALRSSRVPFAGGPQAVDSSGVMSKDKEIIGGQSSMVGSDASQSSGQAALWHLPPGSADMARPGVYIPGRVPAGQNRGDVAGSDIHQGSMSQKSGRSSGVESPASLQMEDTRSMNSHDSLKSDEKTSKKASSSKRKRMDSKAAGDMQSEENSKSDGISSGQNIRKRKQVGKAGAQGQPSRGAEPEQSHILQGATAQVPPLPGGASFFRAHQEGPPASAGRTIDNTKPSNPFAMSQVSNFAEGLASGSIPTELQKSILGGTNMFNTGFGWNQSSQGSAIKNTQGSVANLMRPGVNVEGKINVGSQGAFNPTPTSQMDFPKIPPYMSSSFGGGSQFLDKGKDSASGNTGTELHSAAKVGVNMGIVHGSPMQERQNITRAPQRAESSLQEARLSSLPNRNVGPYQTSHISPNTPFKEQQLKQLRAQCLVFLAFRNNMQPRKVHLEIALGGGPTAEGGGAGQGGNESRVADGSVRENGNSQENSAIFGSQSDMSRLPSTSAGSIAEADSSLKDSEIKKKINIAEHEKSSMEIENIQQAVMQGTGSSSEMRSQEIASPVPSGPQQSYFQGDKRRNAPETYRTDAENLNRNLGFGGQGPSSLGGNRQHPNFEAAVLTKDRLQDEASKESYPPSRLHHMPIDGYSSNLPGKDLTPDTDRNEVEHCTQMGEMSDRSADEGDDDLFEHDDFASTPPKYTMTEKWIIDYQKRKYGENEKKVLEQQSAHKRMSASYQKLKESVSSSEDLTAKTKSVIELKKLQLLSLQRRVRSEFLSDFFKPNTADLERVKAVKKHRHGRRVKQLEKIEQKMKEERQKRIRERQKEFFADIESHRERLEDSFKAKRERLKGFNRYIKEFHKRKERIHREKLDRIQREKINLLKNNDVEGYLRMVQDAKSDRVKQLLRETEKYLQKLGAKLRGDSSMDGRSYVSGKGVTANDVEDESYQPQNYLESNEKYYQLAHSVKEIVNDQPTYLNGGKLREYQMNGLRWLVSLYNNNLNGILADEMGLGKTVQVISLLCYLMETKNDRGPFLVVVPSSVLSGWVSELNFWAPSINKIAYFGPPEERRRLFKEMIVQQKFNVLLTTYEYLMNKHDRPKLSKIQWHYIIIDEGHRIKNASCKLNADLKLYRSSHRLLLTGTPLQNNLEELWALLNFLLPNIFNSSEDFSQWFNKPFESNGDNSADEALLSEEENLLIINRLHQVLRPFVLRRLKHKVESELPGKIERLVRCEASAYQKLLMTRVEDNLGGIGAVKVRSVHNSVMELRNICNHPYLSQLHVEEIEGHLPRHYLPSIVRLCGKLEMLDRLLPKLKATGHRVLLFSTMTRLLDVMEDYLVWKKYQYLRLDGHTSGHERGALIDRFNDPDSPAFIFLLSIRAGGVGVNLQAADTVIIFDTDWNPQVDLQAQARAHRIGQKKEVLVLRLETVRTVEEQVRASAEHKLGVANQSITAGFFDNNTSAEDRREYLESLLRECKKEESAPVLDDDALNNILARSEDEIDIFESIDKQRLDDEMAVWLKVVQDGSVSGLDPSVLPPRLVSDDDLKPFCHAMKIYESSNVKNVKVNVRKKGELGGLDTKHYGRGKRAREVRSYEDQWTEEEFEKLCQAESPDSPQPGGVLKDIDISKESKLEVPAESSIDPKESSIDPVEAKTVPVLAVPDSSPPVPSVPDSSPAKRRRGRPRRSDVSVSPVMSPAKAVQQEAGTTLGSSAPASTIDSAAPTATIHSTGPDVTTHSAAPVAAIKPDIGTEVKATAFVAAVPTATMKPEIGTEVTDHVVLEGSIAKEVGPAVESGHDPVAASAAPHPPAPATSRGRKTQAVETPRRRGRKPKSLFSSSAGDININPVVAIGSGPASVGSPYPQGDMPASLMSRFQKDLVTGRPVTSLPEGVKGISAPESTTPVAEDKHTGTAISSDNANLLMPKIIHNENVGFVQASSEQVFSASVPTLTAVSGGILKASHILLADKPAEKQSASRRRRKKAPGGEDTGVSTRQRAAMKKSDGIPGTNDNVGADMSTAEKLGAVNVKDGSSLQDTPKELPNINSPPYDKSGYDSQPRTPIAVPISEAALPSGSGNAHVAYSDITPRIPTNPDGQDKPVNLHIGAPLAAASQPQVPCKTGNDHVAVCSVVTTTHSETVTEKPLLNPVSELANVQVEPPSSSLNSGKNISTVPSEVNSVAPSKASGRRRKGPASEPRTRSKAATAACERRARLAGPKQTGDARKLEILASPSTAVCVSSVEQQETALAEPPTASVCEPQKNAESHVRGGMSTPMGILDAPKQIATQSITACTEETNSSLSTQTPALPISRESNLSMGDKQGVGVYTIHGQTKMVLAAELASANDEHKLHEVHDKTADGNILQHSAANDTLQDKTDSIAGLDLASRHRIGDLEMEKGDSNTVMLPDCQTPFDASVKDIKDTLAPTEADVSDLQSEAAAIDVTSPKQDTMVVEALHTNSGGSASHLPAALQSTDSNQHAERKGSSENSGSKFFASGKKTEEMEGTLDKNTDNNLIQANADIALGRHSPSEDKREDSCAHVVDGGLLGSKQTLLEVVSAVNTDGSEEALNASSTHSNKDATSVCEVTKDPESHVRVSVLASAAMNARDDCEEVHNVPSTHSDRGGSMVEVDASRDDATSICEVCKDPESNVSGELSMPVGLAELELELPNQSKSSSQSSAVNADETKASINIQTTSLVESGEQKSPRNGAHELKEGMELAGPKIECTILMPSPDDKSSEAHSLAQREMVSGAEQASMKDDKRNKMVDVTFSSGEEQEIQRADVDLPTCPRYADCEGEKDHSPKTILAGSQSFCEASDKDVAPVKDDHTDPQSEVNVVDMNGANQDSAETEAMQIDGVSKGSSSDLPAALRSTDSNQPAEQDGLENSPSISACPKEHEKLEETSDEIGGGNSNRSRTDGDSHIMNLVGYSEDSDEDNSIQVADVGDVGSKETTHDGISAVPRGAEPGDGPCTEPTCETAVHVHEFNVDVAISEDGHGTMALGSVQASTTELKDLESGRCLEHGTGTPVALQEGTAVAAEPEAKKEVDEPKDVEPAAIKPEAVEHDGTEADPSKEASIPPQEETTAVALVTGPEQNEEADAPTQVKPVAVIPGTGPEEKKVEASTQEDNAEAVAAEPESARAQENAEASTQPSPMEIESVQETAMLGEAETRQQLPLPSAEGVVAEASEPPSIEVAAMKEPELLSTEPAPDGENAKLGEAEAEQLLQQPSSCEAMAVTGELPSAVGAKTDGTSDVAADESPAVVGEEVLNTETAPDGENPRPSEADTAQSPHLPEEGKAVAATEPANLEKAEANDGK

SEQ ID NO: 12 - DNA, 25747 bp, Triticum aestivum
  source 1..25747: mol_type = genomic DNA
  exon 1..268
  exon 4021..4134
  exon 4213..4274
  exon 6640..6845
  exon 6917..7639
  exon 7728..7930
  exon 8347..8546
  exon 8627..8691
  exon 8771..9600
  exon 9767..9864
  exon 9973..10158
  exon 10655..10835
  exon 10985..11149
  exon 11228..11271
  exon 11510..11566
  exon 11713..11809
  exon 11917..12089
  exon 12163..12376
  exon 12547..12672
  exon 12756..12845
  exon 16458..16574
  exon 16665..16745
  exon 16832..16939
  exon 17092..17261
  exon 17395..17473
  exon 17555..17629
  exon 19017..19114
  exon 19197..19304
  exon 19413..19470
  exon 19554..19775
  exon 19860..22044
  exon 22146..23309
  exon 23436..23510
  exon 23582..23647
  exon 23721..24515
  exon 24615..25747
agacagcggccagagaagaggaactgaaaagaaagaaaacggggaagaaaaaggaggcaagcagtgcacaggtctagtggaaaatggcggaggcggcgtgctcgacctcgggcacgtagctcacgcgcagctcaccgttccccgttccccgtcgcgctctccagagaccccgcgccgccgccggcgaccaccagctcccccgtgcggcggctccgcgtctccacccgtctcgttctcccgctagggtttcccccgatccccaatcactgtaagccgcgaagacttgtctcgctagtttccttctggttcaagctcacgggagcgtgcacgtggtccccgagtgggtggatttgggggtcgcggtctcggatcttgcgcgatcagtgtagcgctgttcccagctagggttagttcgtagaagcataagttgggaactggaattcgtggagctttatgtgatttgggtcagcgagctgcttctgtagcgagaagttataagctctgagcgcgccatgtggagtaattggcctattctgtgcaataatctcatctttaaacattttgtctttttcccggttccgatagggattttttgggtgtgacttgggtttattccttgtgtgcattgcctagccatgacctgattggttagcttttggttgcacttaattggtctgtgaattgtgttatagggtgggatgtcttgttagtgaagcttgatcagtatcacgcatctgattgcttttctcaaagagtggcactatttttttagaccaaatgagtggcgctatttcgttgttattcacagaatttgtatcatgtggagcggtcccacactatcatgaagcaagaaataccattttttaactttagctcagcatatagtgatatctctgctactttctccagagcagcttgaatgcatgccattgtgatgcctgctattaatttacatagcattacatgtggtgaacatgcaaattctatagcaacttttttggaagttctgttattggtagctatgtaactgtagagtatgcctgtttgcaattcactaaacctgctgctctgcattaacagtttgcatctacaaagattagctctgaaattcatgctgctgtatctgtactctctttcgaacttggatccataataattttcattccaaattttgaagacaaaatctctaaaaccctctataagcatccatgatttctcagactaaaaataggaggggcatggcagcgatctccataatctaaaaacaaaggagtatgatcagaaacctcgctagcaaaggcttgcgacatagacaaaggacaatgttcctcccatttagggcagaagaatactctatctagtttttcaaaggtagcatcctccaaattatttacccacatgaaatttctcccatttaaaggcttctctctcaactcggcgtgttaaaaatgatgtattaaacacaaaactctagtgatcagtatcattggatttgttttttcacagctctttccaattgtgttaaaatccccacctactaaacatggtagaggattatcatgatgtattctagccaactcatctaggaagttagcttttccttccaagtgcgcatcaccataaacagtaatgagatctgaattaaatttggcaatcttaccaaaaagtaatgttctaataaagtactctcccctctccacttggataatatcaaacacatttttactaatacccactaaaatcccactggacctccacctaggatgatttcaatgccactatttttttcctaccactcaaagagtttagttcattgttaggaaaaaatgttttgtggtttccaaaagaccaataaaatccaatctatgatcaattatcatttccctaacatatctcttttggagatcttgtcccaaacctctaacaattcaatccaaaagacctctcacgttacaacttggatggacctaaggcatgagtccgggagaaggtttcgaggagtcgcatcacaagcctgcgaccatccaccccatcccacgaggccttcctaacgcaagactccgtgctttgtcgagacgacgaaacctattattaaaatattgttttatttgtttttgtccatgtacgtatgcacccaagctaactatacttaaaaccgcgttacgaagaatacctctagttgggagttgttttcataacaacaagcctacaatcacaccttgttatatttcgttgagatggtcctagatttatgaaatggaatttgatcctgaatttttcgtttccacgtcaaaagtgtatgtgccaccttgaattggaatcctgattccactccgattccaacatttgcttttcgaaaacaagactctgacccagtttttcttttgttcgattctcctagaatcttgagaatcgggagaaagaactcggcctccggcatttgtttagggataacacaccatggccctggccatggccccaacgaagctgaaagcccagcccatcgggtacccacggcccttggccctcatgcctcagccctcacccatttccactagctaaatactggtaaacctccctcccctctcccccaccccaccacacacacaagacagcggccagagaagaggaactgaaaagaaaaaaagggggaagaaaaaggaggcaagcagtgcgcagatctagtggaaaatggcggaggcggcgtgctcgacctcaggcacgtagctcacgcgcagctcatcgttccccgtcgctctctccagagaccccgcgccgctgccggcgaccaccagcttccccatgcggcggctccgcgtctccacccgtctcgttctcccgttagggtttccaccgatccccaatcattgtaagccgcgaagacttgtctcgctagtttccttctggttcaagctcacgggagcgtgcgcgtggtacccaagtgggttggtttgggggtcgtggtctcccgttagggtttcccccgatccccgatcactgtaagccgcgaagacttgtctcgctagtttccttctggttcaagctcacgggagcgtgcacgtggtccccgagtgggtggatttgggggtcgtggtctcggatcttgcgcgatcagtgtagatctgttcccagctagggttagttcgtagaagcataagttgggaactggaattcgtggagccttatgtgatttgggtcagcgagctgcttctgtagcgagaagttataagctctgagcgcgccatgtggagtaattggcctattctgtgcaataatctcatctttaaacatttcgtctttttcccggttccgataggaatattttgggtgtgacttgggtttattccttgtgtgcattgcctagccatgacctgattggttagcttttggttgcacttaattgatctgtgaattgtgttatagggtgggatgtcttgttagtgaagcttgatcagtatcacgtatctgtttgcttttctcaaagagtggcactatttttttatatcaaatgagtggcgctatttcgttgttattcacagaatttgtagcatgtggagcggtcccacgctatcatgaagcaagaaataccattttttaacattagctcagcatatagtgatatctttgctactttctccagagcagcttgaatgcatgccattgtgatgcctgctattaatttacatagcattacatttggtgaacatgcaaattctatagcaacttttttggaagttctgttattggtagctatgtaactgtagagtatgcctgtttgcaatttactaaacctgctgctctgcattaacagtttgcatcttcaaaaattagctctgaaattcatgctgctgtatctgtactcaatgtactgtatttgattatcgaaatctatcaggtttgttttcctacattaactactggcgtactggtttgccttttataacttataatttataagtgttagttggattacgatttatttatcttctttttgattgatcttattttgatggcaagcagagtttgcgaatggcttcatcacagcatgttgaagtggaggctgcgaagctacttcaaaaactcattctggaatcaaaggatgagcccgctaaattagcaacaaaactttacgtggtatgcagcgcaacgaatatacaggacatgaaaagccttaactcaaccataaccttgtttctttgttcaatgttctagatatgtcaacatatgaagttaagtggaaaagagcagtctcttccctatcaggtcatatctaggtaaatatttcttctgttcttggctatcttttcagaagttttttttgccatcaattttactgtaaatgttagtcaaatattctgttagaaaaagattactccctccgatccatattaattgatgctggtttagttgtattaactttgtactaaacaagtgtcaactaatttggatcggggggagtagttaaagttctaccttgtgtcttacacatgttgtcttgttattcttgactttcagatttgataattgttgatgtgttgttcttatgttcgaaagttctgcttatttagatttcacacatcagttagtactcatcaaactagatttcacacatcagttctcactgtcaattgtggaatagtatacaaggagggggcctaaccatctaaatgctgttgcagcgaggttgtagcttggtactctccctaggtactaaatgttgctccaactagtttaggtgaagaaaataggaataagcagaaagtccagaggcccctggacacaggctcaatgagggagacaggaggatattgaagctcagtgatggacactttcctcatctatgtagtgaactgttaatacacacttacacagtagtatgatatccacaaccccaaaatgcatgggcaaattggagttcaacatcctccctctgagcagcctttctcatggagatggagattgagtagggagagaagtcgttggaggatggcaagagggagtggcagagaagtgcaagtaggagtaagatgggagtagcaagctgtcatttggaggcttaccactgataatatttttcttttggttgacttgttagcctgtagtaatagatcttgattcttgaaatcctctatccttgatgggagtagcgagctttttaagactatttgattgtgtttggctgggctgtggattttctgaaagcagatgcaagagatgtgccgtgggaaagctgctgtggactgtgtgttgtgagaaagctgtgaagccatttggcaaactagctgtctgaaatgcggctgcggggataaatgtctgaaatacccttgaaagctgagacattggatacatactgtttaatgataaaaacatcattacaggttgacctagttcgtaaatatagctattcaaatttgttttaatgcatattaacgaaaatgtatatagctctacatatcacaaaatagatgcactagtgccatacaaaatttacatatcaacagacacattaatctggttccagtctgaccataggctactactgccatacaacataaacatatcaccaaaaaatgcaatggtcgtacatctccagtagggaaaatctggagaaaggaacgacatgtacatgggcgagggaagcggcagaccggcagtagtacacctcgaatgggggatgtagcagaggaggtcaggcagccatggtcggcggcgaccttgctcgtctgagtaaccttggacactggtggaggtagatgagggggtgggggtggagcggggaagaggaggccaattgaccgaggtggatgaagggatggaagcatccactggcggtcttgcggtagcgtgccgtcagcgacatgggagcgagctggtgaccagcagctggccggcggtgctaatgaaccctagaatcgccagaggtgggggacgagaaaagggccttgctcgatgggctttgtagagctgtctctcgtggacgtaccggcaggattattttggcggcgaaggtgagtaatttgatctcaagtggatgtaggttcggggagccatgcagccaaagccagaaaagcacctcttcggccgctttcactcgtacatgtgttttgcgatggctttcaagggaatcgcgttcactcgttttgccgtttggttgcgatttcagctgcgaaggagagaaatccacagcgaaagccaaaccaaacgcagcctttgccttagacaatttaagagtgtagaaccttgagcgcaccttttgtctggaatcaatcatgagtgttgtcaactgaagctatcgttttccataaatttggggttggttttgcaccaaaagaattaagtatcttttgtttggtagagcttatactccattatgatattgagtgcgttatggtttatactctatagtaggtggtgtcagatgatttaccaaatgtactgtttgcaacgtgtagtataagtataataatacaaataatccagtttggttaggtctactttacctgagtgtttgtaatttcaaatgaaaggattctgcgtatgtcagaaagttctatcaaacttccaatttttctctagcttgacttctctcctctttctagtttctaagatgcctgtaacatccgtaatttttgcctgcagggccatggagactgtcgtaagtcaacatggaattgatatggatgcattgcgatcatcacgagttccatttgccggcggtccacaagcagtagattctagtggcgttatgtctaaggacaaggagatcattggtggtcagtcttccatggttggaagtgatgcatcccagagcagcggtcaagctgcattatggcatttgccaccaggtaaccaaccaacttgaaaaggaaactgcacactgttttggagatgtgatatgatttttttatattattaggttcagcagatatggcaaggcctggggtgtatattccaggcagggttccagcaggacaaaataggggcgatgtcgcaggatctgatattcatcaaggctccatgtcgcaaaagagtggcaggtcctctggagtcgaaagccctgcaagtctgcaaatggaggacactagatctatgaattcacatgattctttgaagtctgatgaaaaaacaagcaagaaagcttcctcttccaagagaaaaaggatggattcaaaagcagcaggggatatgcaatctgaagaaaactcaaaatcagatggtatctcaagtggacaaaatattagaaaaaggaaacaggttggcaaagctggtgcacaaggtcagccctccaggggagctgagcctgagcaatcacatatactgcaaggtgctactgctcaggtgccacccttacctggtggtgcatcatttttcagggctcaccaggaaggtccaccagcttctgctgggaggactattgacaatactaaaccatcaaacccattcgcaatgtcacaagtttcaaattttgctgaagggctggcttctggtagtatccccactgagttgcagaaaagtatactgggaggaacaaatatgtttaacactggttttggctggaatcagagttcacaaggttcagctattaagaatactcaaggttctgttgccaacttaatgcggccaggagttaatgttgaaggtacttccattaaaaaataatgacataacagcattgtgaaagacttgaattacaaatatttaccttaatgagcttgcttacactgcagggaaaattaatgtagggtcacaaggagcttttaaccctactcccacatcgcagatggattttcccaaaatccctccttacatgtcttcttcctttggaggtggctcacagtttctggacaagggcaaggactcggcttctggcaataccggcactgaacttcattctgctgctaaagttggagttaacatggggattgtgcatgtaaggcctgtagtttaatccttaaagacccggggtgttaacatgctattttggctacagtttggcccttctaaaaaaccttttaattgaaaagctaatattttttgctgtgttcgccaatggtaacttgttacggaaatgcctagtagtaatggtataatgcagggtattcatttgcataagattgtaatcgagcttcgaacacaagtgtattgcacgccggtttcgtgtatgtctatttgcgtgccttgatagactttctgctaggttttaggttgatcaaccgataaataagctgtttctgcctgcaagatttaagaattttgttgtctggtcatttagtgatattttaattgatttctgtatctcaagtagaggtgttttatttgatgcatctatgtaatacgactttgcagggcagtccaatgcaagaaaggcaaaatattaccagagcaccacagagggccgaatcatctttgcaagaagccagattgtcttcgctcccgaatagaaatgttgggccatatcaaacgtctcacatctctccgaacacacctttcaaagaacaacagttaaagcagctccgagcacagtgcttagtatttcttgcattcaggtacatgcttagagcactgtaggatgattggtatccgaagttcatctctgtagtactaatttagctactctttcttgtagaaataatatgcagcccagaaaggtgcaccttgaaattgccttaggtggaggccccactgcagagggtaagaactaagaacagaaaacattgtgtgagttgacagggtttctgtactcatgatgagcttataattaaataaacaggtggcggtgcaggtcagggaggtaacgagagcagagtggctgatggttctgtaagggaaaacggaaacagtcaggaaaactctgctattttcggcagccaaagtgatatgtctagactcccatccacatccgcaggcagcattgcagaggctgattcttcactgaaggactcggaaattaagaagaagatcaatatagctgaacatgagaagtcatcgatggaaatagaaaatatccagcaagctgttatgcagggaactggttcaagttctgaaatgcgctcccaagaaatagcatcccctgtgccatctggaccacagcagtcatactttcagggagataaaagaagaaatgcccctgagacctacaggacggatgcagaaaatttgaacaggaatttaggtttcggaggccagggaccatcttctttgggtggtaatagacaacatccaaattttgaagctgctgttttgaccaaagatcgattacaggatgaagcatctaaagaatcatatccaccttcgaggcttcatcacatgcctatcgatggttacagctccaatttaccaggaaaggatctaactccagatacagatagaaatgaagttgaacattgtacccagatgggggagatgtctgatcgatcagctgatgaaggagatgacgatctatttgagcatgatgattttgcatcaactcctccaaaatacacaatgactgaaaaatggatcatagattatcaaaagagaaaatatggagaaaatgaaaagaaggtattagagcagcagagcgcacataaaaggatgtcagcatcctatcagaagttaaaggtctctctctgccttcctcacatttattcttgaaatggggggagtgtcatttagaaatactgtgtacatatttatgagtttttgtgagttcctgtttcatatgttcagtttttcctcactgtagcagtgttggttgcaaaattttaagttcttgttcatcctacaggaaagtgttagttcatctgaagatcttactgcaaagacaaagagtgtcattgaattgaaaaagcttcaacttctctcacttcaacgtcgtgtgcgcaggtttgcttgccattggagaccatcagtcttcagtttctctccttgtgcttaccgcatgtttctatggctgtaacttccctattctaatttcttgcttatattgggcagtgaattcttgtcagactttttcaagcctaatacagctgatttggagcgtgtaaaagcagtaaagaaacaccggcatggacgccgtgtgaaacagcttgaaaaaattgaacagaaaatgaaggaggaaaggcaaaaaagaatacgcgagaggcaaaaagagttctttgctgatatagagtctcacaggttggatgactatatttgattattcattctgacccctttagtatggagatgttatttaatttttttcttacgcaatattctcaagtatttgtggcatctatgctccgtttgtacagtactgatgatttggggtctatttgccaatgcagtgactatcaagctttactttcattttggtattgtgtatagactaatatcatctgcattagagccacaacaaaagcagtttacattattattcttgcagctaaataaagtccatggtggagcacagcaaaaataagctggcccttaaataatcaaacataagtaagctaagctgaaataagtaaatggtggtttcttaagtaaacatattgctaaaagaactggattagaatagctgattcaacctagtcagtagtcacctttgtaaacgctgtctgtctgtgtttacaccccctcaacattttacccatgtcatttggtaataatgccttgcctttgtaacttgcagagagagactggaggatagtttcaaggctaaaagagagcgtctaaagggtttcaatcgatatataaaagagttccacaagaggaaagagcgaattcatcgggagaagctggataggatccagcgggagaaaattaacttgcttaagaacaatgacgtcgaagggtatcttaggatggtccaggtgagtcttatttgctttgtttctcatcatgttcttctatattagcttaacccttcacacgtcaaacaaagaaaagcttaatccttcattttagtttctcaatatttgttggactaagtcacatctgctaagtgtttgctgctttgcaggatgcaaaatctgaccgtgttaagcaactactacgagagactgagaaatatctacagaaacttggggccaaattacgaggtgacagctcaatggacggccgttcttatgtttctggtaagggcgtcactgcaaacgatgttgaagacgagagctaccagccacaggttttattatctctttgttttagtcaacgtctaggtgcatttttgttgaatatatacttaattttgttctctttccagaattatcttgagagcaacgagaagtactatcagttggcccacaggtactacatggattaaatagactttcatgcttcatttagtaaatccttatcaatgtctgcctagcgtaaattatgtactacctaactttctaatcctccatcttattcatacttctttttgaactttaccatcttattcatacttctttgccactgaactttctaattctttttttttgagattactgaacttactaattctgctttgtattcatacatatttgtttattttttctagtgtgaaggagattgtaaatgaccagcctacttatcttaatggtgggaagttgcgggagtaagttgtgctgctattttccctgcctttacctccttttcattttaagtgtatttttgacattattgttaccgacttgtgtgctgttacaatctgtttaaccatccagtacacatttccttgatctattacttgctgtattacaggtaccagatgaacggtttgcgttggctggtttcattgtacaataataatttgaatggaattttagctgacgagatggggcttggtaaaacagttcaagtaagatccagtacaacgccatctcagcatttattgttcggcttgtatgttatctgatctaaacaagtgtctgaattctgcttacactgcccttgctactttgtcaggtaatctctttgttgtgctaccttatggaaacaaaaaatgaccggggcccatttcttgtggttgtaccatcctctgttctttctggatgggtatctgaactcaacttctgggcacctagcataaataaaattgcttattttggtcctccagaagaaaggcgcagactgttcaagtaaattctgaatttatagttcgatactttgttgttcatgtgaacattttattaaccaagctaattttttcagagagatgattgttcaacagaagttcaatgtccttttgacaacatatgagtacttgatgaacaaacatgataggccaaaactaagcaaaatacagtggcactatataataatcgatgaagggcaccgtataaagaatgcgtcttgtaagctcaatgctgatctgaagctttatcggagttctcatcggctattgctgacaggaacacctctgcaggttctaaagcttgcacttatactttcacacttgatcctgtatttgttgcttttcaaggaatgtatgaacggcttgctcatatatttatttaatgttcttgggtctctgtatgaagtattctattatgcatatatgtcaagttgctaacttcacgtaacttcttcttgaagaataatcttgaggagctgtgggcacttttgaactttctgttgcctaatatatttaactcatccgaagatttctctcagtggtttaacaaaccatttgaaagcaatggtgataactcagctgatgaggtaaagctgccgtttttcatgatacagcattgttttcttggaaggaaactgtgtttgactccaatcatcttttttcttaaaaggccttactttcagaggaggaaaacttgctgatcataaaccgtcttcaccaagttcttcggccctttgtactccgaagacttaagcataaggtattgattttattcgctatctttatgcttgtgttgaaatcactggcactgtaggaattcaccatgcaatttatttgaaattccaagttccaacaggagatctatgctatgcttagctattcaacctcgttatctcaaactgagggagttccagccttccagaattgcatccgctgatcacattggcagaacccttgcttctaaccgaaacctagtaatagtagggagacagataagaaaataattgcttgatgtctttattgatgtgagggcctagccttatatagctggctacatagatatatggaaataaactaacaatcttggaagcttatctagttatttaaaagaaatctaataaccagtaaccaactagagatgaaatttgttacgtatttgcttaaggcagaccagggggttagactttaggcattggctgtatgcctgaccccacttgtcacacattataagctcatattatttgagcagtacacatgttccttaaatatgtgttacctatcaggagttactcacagcatgtaattcggctttcaatatgtcagctgattcagtagacattgcttgatgttccttacttctttttccatttgaagtctttatatgttgcatttgttgggatgattcatatttttgtattgtacgaatgctgagctgggcattgcagtggtgaagagctaaatattgtccataactaggttcaacagcacaacgcaacacaatatagcaacgtcaaactggttcttgttagctttgttgctctacatgatctgtaatttaaaaattctatggacaagatttctctatgtgcttgtacacatccatctagctgcgtgaatgccaaaaaatgttgcttattctgtttctcaatatatgccactttggcatatcagtacaagcacggtcacacttttcaagtttgacgaccaacatattaaaaacacctagattttcacatcagaaaaacactagtagctcttccactagagttgctctacaagttgtagatgcttttatgaatgtggattttctcaactagttgccgctgcaccctactctagcatccatcgcgaaaagttctaaaaagatgggaatttcgtagatgtacaatttgctataatatgtgcagctgataaatgaccatttgtgtattgtgcaactatgggcgtgtttggttccttgggttgcacctggctcgcacccaccatgcaattttctggatgtttggtaccctgcatgtccaactgggcctggcccgacagatgcaaaacgaggctcccagccaggctgaggggaaacgcaagtttcggccgtttccccgagcctgcatccgcgcatgcacccacccactcgagcaaagggggtcttctctcgcatcctcttctctcctgctactcgcgccgctctcctcgcttttctcttctctcctgtggctcgcatctcgccgccccgtcgcctttgtcgcatcgccgggcgcgtcctcatctccggcggagggagtactctcctcctcccttccctctcccatctgcctgcatccatctattctccctcccatctccagctctctgccgctcgcgctgttcttggcgctgctcgtggcggatgcgtgagcggaatggatcggcggcctcgtccgtccgtgaacgtgaacgaaggcaaggcggggctggaggttcgggaaggggcggtggctcatctgaccgatgcgtgctgatcccatctccccccctcttcttttttatttaatcttagacctgaccccaacctcattttcctctgtcgattagagatggttgggttgtttatatataaacgtggctattgattagcatgaattgggcagagatctgtccccaacctcattttccataggattatacatggctggtgattggtatttaggctgagatttgtgtgatctgtcccttcatgaaaaatgtctgcagattttttttatgtaaataggtgcagcaccattgttatgttcctttgttggagtgtaatggagtaatatggacaatatgtatttgtagctctatctaatatgtgaacactaagatgtactgtgtatctcatgcaacttcagatgcaacataccaaacaaaatctaagttgagcctggcccatatcatgtagtacaccaaacacgcatgtcaactcttttttgcataagctcaaccaggctagccccagccaagctccttcatgcaatgcatcccagatgcacccagggaaccaaacacgccctgtatgtgcacacatggtcacactcactcttaaagcaatctgtgcgagcattttgtatatctatgacttttttcgctttttgataaagaattacgtgctttccatcttcacatttttgtgaaatgcatgagatataattttgccaactactatacaaacatataatcattaagaccatgaacaggaaagcatctttcatttataaacggtgagtgctccatatttcttagtttatgattactagtaaaaggtactaactctgttcctaaatgtaagacgtttttagaactgcaaaaacgtcttacatttatgaacagaggatagagtatacgattcgaacagaaatcatggtatttggcaatgttcaaaaaatcattaactggtagctgcttggtcggctggtgataagggattgataggtgaatcggccagttaacggcaaatatatcagttaattggcctataagtcaattaatcggctactcggtgacccactgagtagggattaattggccagttaactgatttatcggccgatattctgacaatacttaattaggataattttcgaccatgtggtgtagacgtgcaactttgctttttagaggttggtgaaccaatcttgcaatcggttcattgatttttaaaatttgatatttgaagcaaatttgttacgccaaaagtcaaaattttgaatatgaaaactgaaatcttttgtgataaaattttcacaaaagaataaccgaaagtattgaaattatgcctgataattacgccaatagtcaaggaaactcgatcaaactacatattaattggttcttatgctaatgaccagctgaaaaattggttttggcaggagcactgtagatggtgtgtaaatcaagttcaaaactgctgtttacaagtactccctctgtaaataaatataagagcgtttagatcactactttagtgatccaaacgctcttatatttctttacgtagggagtagtagagattatgattactttacgttgcaacttagttaaaaaagcaactcatatggccatgcccctttttctcttggttttgaattgatttttgtttagactttagaaccgttgatgtcgaataaattcgaaagaagcaccaatcattggagctccaaccatttgtacttctttcaaacttattcgacatcaacggttctgaagtctaaacaaaaaactactattgtgatgctgtgtgggaaactagctcgtcaggttggggatttgatattgcttcccaactgtttctcatctttgtttgtatctggatcatctggatggtgcaatagtttcaattgcgttttactgtcttcaggttgaaagtgaattgccagggaagattgaaagacttgtaagatgcgaggcatcagcttatcagaaacttctgatgacaagggtggaagacaaccttggtggaattggagcagttaaggtgcgtagcgtgtgactgttctgagttgtttattttaatgtttcacttgtcagatatttcacaggttcttatgtgtcttaaattttttaggtccgctcggtgcacaattctgtcatggaattgaggaacatatgcaaccatccataccttagccagcttcatgttgaggaggtagagcatgattctgccctgtcgcgacattctggctatttttgtttcctcttgggcatcaccagccatatggattctctatgcagattgagggtcatctacctaggcactacctgccatctattgtgaggttgtgtgggaaacttgagatgttggacagattgctacccaaactcaaagctactggccatagggtaagtggattttactggtagtttggtaggtttgtaaagatctcctactcgtatgtcgcatgaattgtattttctcgaacaagtcacatatcaaacttgcattatctgagttgaagttgtcgttcgttccttgttccttccttggcatgcaggttctacttttttctacaatgacaagattgcttgatgtgatggaggattatctggtatggaaaaagtatcagtaccttcggttagatggacacacttctgggcatgagagaggagcacttattgatagatttaatgatcctgattctccagctttcatttttctgctaaggtaaaatattggttcagtatattgtggtgtaggaggtaatatataaatagaacatagtgaactcatgaatccttatcggccaatttaattaattaatatttgatacccaaggcctacttcactttttctgtagtatccgagcaggaggcgttggtgtcaatcttcaagcagctgatactgtcatcatatttgatactgattggaatcctcaggtagctaaagttccttaagtgttgtcactctatgttgtaagatttgttttacataaatatatcttttccttgattattcaggttgacttgcaagcacaggctagagcccacagaattggtcaaaagaaggaggttcttgttttacgtttagaaactgtaagtgcacactgacagttcgcttatcacctggagtaaatatgtagaaaccgaaatgaacaaggaacatttgtttgctaacaaggaaatggtagttaaaaaatagaacaagtcgccagttgagtccttagtgttgcatagggtttgtttgagcatcttagatcaatagttagatatgtggcttatgtggtattctaaatgaagaactggtccagatttactcaatggcactccaccatggggatgggcccccatgcatgaacagcaccctccttgcactttcttcctcacttcatgtaaaagggttaatttggaagtgcaatgttttgactcatcatgcatcatatgctactatgcccacactggaatctggattccaaacccactaaggtcaccactctaaacaggctggatgtttggagcctagatacatatctgtacgtcacagtattgtttttattggtgatgataaagtcatcctagtattgtttttatctaaattttgagtaattttcatgaccgcaacaacaaagcctttataattttcacgactacgtataaagaatcaagaaccagcaccattgctcgcacaagtttctggaacacgcagtaataaactgtagggccgtagctgactaattttgtcatataactcacatttttcttgaaagcttctcaattatatacctgaaagtgtcctttgttttatgtcatttcgtgtatttaggtatttttgtggtatttaatattgcttgttttcagatttattcaagaaattagtgatgtgcgtggtctatcttcattgtattatagcttgggttttcctctctttgcgccaatttgtggctgttgtgttgctgcgctgctttggaacctagctatagggatctttactgttttcttgtatattttggtgatataactccaaaagaagttactttcaactgctccctccgagaatacgcttctgaatatctgtccatggagaatttcacgagtgtagttattgctgtgtttccagtctctgttcttacttaaatgctttgtatctgtcaattagtaggggtgcgcatggtcatttctcatttactctctcagatttagtgctctctttgtctggtcgcttgatgaagtaactatccatatgtggaaaaaggtactgcactagctaccagatcgtgactgctctctacggagcctttgtcttcttggctgtttatttttctaagcttggacagaacccactagtgatttatgacactgccacaaatatgatacgaataaatgctgcctgttatgttctaaccagaaccaatgcattgtattacttcaactgaaaatttcaatacgcctgttcctgacttggatgtaccttgttgaatttaaggtccgaactgtagaagagcaagtcagggcttcggcagaacataaattaggcgttgctaatcagagtataactgctggatttttcgacaacaacacaaggtcaattcttctactcggttaagattttagcttttctagctctctttttcctttccttcatgctagatagtaacaattgcagtgctgaagatcggagggagtatcttgagtcacttctacgtgagtgtaaaaaggaagaatcagctccagtgttagatgatgatgctctgaataatattcttgcccgcaggtaagactgagtttgctgttagtattatttaagcattgttttaacaatctctgccactcctggtacttttaactaattacatgacatatcacatttctctccttgcagcgaagatgagatcgacatatttgaatctattgacaagcaaagactagatgatgaaatggtatactaaattcctttactttgtacatgtttatttctgctaatattttgtgcatcccaatttgattcttgtaccccttgtaggctgtatggctaaaggttgttcaggatggttcagttagtgggctagacccctcagtattgccaccccgccttgtgtctgatgatgatctgaagcccttctgtcatgctatgaagatttacgagtcttcaaatgtaaaaaatgtgaaggtaaatgtgaggaagaagggcgagcttggcggccttgatacaaagcattacggaaggggaaaacgtgctcgtgaggtcagttgcattatcatcttctgtatgtctctctattattggttgaagtatttgtttgctaatttcattatatatcctttgtaggtccggtcttatgaggatcaatggaccgaagaagaatttgaaaaactttgtcaggctgaatctcctgactcacctcaacctggtggtgtattgaaggatatagatatctctaaagagagtaagttggaggtacctgcagaaagttcaatagacccaaaagaaagttcaatagatccagtcgaagccaaaacggtgccagtcctggctgttccggactcctcaccaccagtcccgtctgttccagactcctcaccagctaagcggcgaagaggtagacctagaaggtcagacgtttcagtatctcctgttatgtccccagcaaaagctgtccaacaagaggcaggaactacacttggcagttctgcaccagcaagtaccatcgattctgcagcaccaactgctaccatccattctactggtccagatgttaccacccattctgctgcacctgttgctgccatcaaaccagatattggtacagaagttaaggctactgcttttgttgctgctgtaccaactgctaccatgaaacccgagattggtactgaagttacggaccatgttgttttggaagggtctatagcaaaggaagttggtccggcggtagagagcggtcatgacccagtagctgccagtgcagcccctcatccaccagctcctgctacatctagaggcagaaagacccaagcagttgaaacccctcgcagacgaggccgaaaaccaaaatctcttttctcatctagtgctggtgatattaatataaaccctgtggttgcaattggtagtggacctgcttctgtgggttctccatatcctcaaggggatatgcctgcaagtctcatgtcaagatttcagaaggatttggttacaggtaggcctgttacgtcattgccagagggagttaagggcatctccgcccctgaaagtacgacgcctgttgccgaagataaacacactggaactgcaataagctcggacaatgccaacttactaatgccaaagatcattcacaatgaaaatgttggatttgttcaagcgagctctgagcaagttttttctgcatcagtacctactttaactgctgtctcaggtggaatattgaaagcatcacatattctcttggcagataagcctgccgagaagcaaagtgcttcacgccgtcgcagaaagaaagcgcctggtggtgaggatactggagtaagcactaggcaaagagcagctatgaagaaatctgatggtattcctggtaccaatgacaatgttggtgcggacatgagcacagctgagaagctaggagcagtgaatgtaaaagatggcagttcacttcaagatactcccaaggaattaccaaatataaactctcctccatatgacaagtctgggtatgactctcaaccaagaacacctatagcagtccccattagtgaagctgcacttcctagtggttccggtaatgcccatgttgcttattctgatataactcctaggatacctaccaatcctgatggtcaagataaaccagtaaatctgcacataggagcacctctagccgcagcctcacaacctcaagtgccatgtaagacagggaacgaccatgttgcagtgtgttctgtggtcactaccacacattctgaaacggttactgaaaaaccattgctaaatcctgttagtgaactagcaaatgtccaggtcgaaccacctagttcttcacttaattcaggtaaaaacatcagtacagtgccttcagaggtcaatagtgtcgctcccagtaaggcatcaggtaggaggaggaaaggtcctgcctctgaaccacgcaccagaagtaaagccgcaacagctgcatgtgaacgtcgtgctcgactagctggaccaaagcagacaggtgatgcgagaaaattagaaatattggcaagcccaagcacggcggtttgtgtttcttcagttgagcaacaggaaaccgccctggcagagcctcccaccgcttctgtctgcgaaccgcagaagaatgctgagagtcatgtacgtggtggaatgtctactccgatggggatactagatgccccaaagcaaattgctacccagtcaattacagcatgtactgaagaaacaaatagcagtctaagcactcaaactcctgcacttcccatatccagagaaagtaatctttccatgggtgacaagcaaggttctctctctctctctctctctctctctctctgtgctgttattattcattgtttggtagtaacaatggctcatgctgatgcccatgatgccttttttcaggtgttggagtttataccatacatggacaaacaaagatggttttggctgcagaactggcatctgcaaatgatgaacataagctgcatgaagtacatgataagactgctgatggtaatatactccaacacagtgctgcaaatgacacactccaggataaaactgatagcattgctggtttggacctagcctctcgtcatagaattggtgatttggaaatggagaagggtgattctaatacagtgatgttaccagactgccaaaccccttttgatgcctcagttaaggatattaaggatactcttgcccccacagaagctgatgtcagtgatctgcaaagtgaggctgctgctattgatgtgactagtcctaagcaagatactatggtagttgaagcactgcacactaattccggaggttctgctagtcatctgcctgctgctttacaatcaacggactcaaaccagcatgcagaacggaaaggaagttcagagaacagtggctctaaattttttgcatctgggaagaaaacagaggaaatggaaggaactttggataagaatacggataacaatcttattcaggcaaatgccgatatagctttaggaagacattctccttcagaggacaaaagagaggacagttgtgcccatgtagttgatggtggcctgttgggaagcaaacaaactcttcttgaagtcgtttctgctgtaaacactgatggctctgaggaagcactcaatgcttcgtctacccattcgaataaagatgccacctcggtttgtgaagtaacaaaggatcctgagagccatgtaagagtgtctgtactggcctctgctgctatgaacgctcgtgatgactgtgaggaagttcacaatgttccatccacccattctgatagagggggcagcatggtagaagttgatgcgtctagagatgatgctacctctatttgcgaagtatgcaaggatcctgagagtaatgtatctggtgagttgtcgatgccagtagggttagcggagctcgagttagaactgccaaaccaatccaaatcttctagccagtcaagcgcagtaaatgctgatgaaacaaaggccagtatcaacattcagactacttcattggtagaatcaggagaacaaaaatcacccagaaatggtgcacatggtactccctatctctatcccctctttccccctccctctctcaccaaccatgatcctgtacacattccccggtgtatgctgattgttattcttatccagctagtgtatcttttttatgttttgccagagttgaaagaagggatggagttggccgggcctaagattgagtgcacaatactaatgccgagtcccgatgataagagtatgctctgttattactttctgttgtagtagagacggccagggggctcatgcacatctgcaccttttcaggttctgaggctcatagtttggcacaacgggagatggtttcgggtgcagaacaagcatctatgaaaggtacagttttaaatttctgaattaattaacgcatggtcaataattactcatgggttatctaacatatgtacagatgataaaagaaacaagatggttgatgttacattttcgtctggtgaggaacaagaaatacagcgagctgatgtagacttgcccacttgtccaagatatgcagattgtgagggtgaaaaggaccattcccctaaaactattttggcaggcagccaatctttttgtgaagcctcagataaggacgttgccccagtgaaagatgatcacactgatccgcaaagtgaagttaatgttgttgatatgaatggtgccaaccaagactcagctgaaaccgaagctatgcagattgatggtgtctccaaaggatcttcaagtgatttgcctgctgctttacgatcgaccgattcaaatcagccggcagaacaagatggattagagaatagtccctctatatctgcttgtccgaaagaacatgagaaattggaagaaacttctgatgaaattggtggtggcaattccaatcgtagtcggactgatggtgattctcatattatgaatctagttggttattcggaagactcagatgaggacaattctatccaggtagctgatgttggtgatgtgggaagtaaagaaactactcatgatggcatctcagctgtccctagaggagcagaaccaggagatggaccctgcacagagcctacttgtgaaactgctgttcatgtgcacgaattcaatgtggacgttgctatttctgaggatggtcatggcacaatggcccttggcagcgtccaagcgtctacgacggaactaaaggatttggagagtggaagatgtctagaacatggaacaggtacttctttatctgcttgcaatgttcatcaaagcccactgaaagaacttagttatggtatttcagtaatccctgaccctgttgagcatgatggcacaggaacccctgtggctcttcaggagggaactgctgtcgctgcagaaccagaagcaaagaaagaggtcgacgaacctaaagatgttgagccggctgccataaagccagaggcggtggagcatgatggtacagaagccgatccaagtaaagaagcatctatacctcctcaagaggaaaccactgctgtagccttggttacaggaccggaacaaaatgaagaagcagatgcacctactcaagtcaaaccagttgctgttatacctggtacgggaccagaagagaagaaagtagaggcatccacccaagaggataatgctgaagcagttgccgcagagccagaatctgctagagcccaggaaaatgcggaagcttctactcagcctagtcctatggagatagagtcagttcaggaaacagctatgctgggagaagctgaaaccaggcagcaactgccacttccgtctgccgagggtgtggtggccgaggctagtgaacctccaagcatagaggtggctgctatgaaggaaccagagttgctgagcactgaaccagcacctgacggtgaaaatgcgaagcttggagaagccgaagctgaacagctgttgcagcaaccttcatcctgcgaggctatggcagtcacaggagagcttcctagcgcagtcggagcgaaaacggatggaacttcagacgtggcagctgatgagtctcctgctgtcgtgggagaggaggtgctcaacactgaaactgcacctgatggtgaaaatccaaggccgagcgaggctgatacggcgcagtcgccacatttgcccgaggagggcaaggccgttgcagctaccgagcctgccaaccttgagaaggcggaggccaatgatggaaagtagttagtgcgcaaaaatggaagcagatgttgcgttgaagaacatctgccgttagatcagagagagcatgtttgggctgatgaaactgagaagtaccttagactttatgcaagtgttgtatgtagaacataattaagaaacctgttgtattcagaggagttgttggtacataagttataactaccttgtcgctttgcaatactagtaccttgttggacctgatgcaattggttgagatcctctacggcagtactgccg

SEQ ID NO: 13 - RNA, 20 nt, synthetic construct
  source 1..20: mol_type = other RNA
tgcatccgggaagaaaacag

SEQ ID NO: 14 - RNA, 20 nt, synthetic construct
  source 1..20: mol_type = other RNA
tgctgctatgaaggaaccag

SEQ ID NO: 15 - RNA, 20 nt, synthetic construct
  source 1..20: mol_type = other RNA
accagaagagaagaaggtag

SEQ ID NO: 16 - RNA, 21 nt, synthetic construct
  source 1..21: mol_type = other RNA
agcattgcacactaattctgg

SEQ ID NO: 17 - RNA, 20 nt, synthetic construct
  source 1..20: mol_type = other RNA
agaaacgatttcgggaagag

SEQ ID NO: 18 - RNA, 20 nt, synthetic construct
  source 1..20: mol_type = other RNA
cgctcaagaggatattgctg

SEQ ID NO: 19 - RNA, 20 nt, synthetic construct
  source 1..20: mol_type = other RNA
tcacatgatgaaggttgctg

SEQ ID NO: 20 - RNA, 20 nt, synthetic construct
  source 1..20: mol_type = other RNA
actcaagtcgaaccagttgc

SEQ ID NO: 21 - RNA, 20 nt, synthetic construct
  source 1..20: mol_type = other RNA
tcacatgatgaaggttgctg